European Patent Application EP 4 636 088 A1, published October 22, 2025. Title: POLYNUCLEOTIDE, PROTEIN, BIOLOGICAL MATERIAL, AND USE THEREOF IN IMPROVING QUALITY OF PLANT FRUIT. Applicant: Agricultural Genomics Institute, Chinese Academy of Agricultural Sciences. Application EP. The sequence listing filed with the application follows.

SEQUENCE LISTING (196 sequences)

SEQ ID NO: 1 - DNA, 1602 bp, Solanum lycopersicum
  source 1..1602: mol_type = other DNA
atggggaattgctgtgggacacctggtaattcttctgagaataagaagaagaagaacaaaccaaacccttttgctcttgattatggtgcaactcaagcatctggaggtgatggaaacaagcttgttgtgttgaaagatccaacaggacacaatattcaagaaaaatatgatcttggttgtgagctaggaagaggagaatttggggttacatatttatgtactgatgttgatacaggggacaaatatgcttgcaaatcgatatcaaagaagaaacttaggactgctgtagatatagatgatgttaggagagaagttgagatcatgaagcatttgcctaaacatcctaatattgtgaccttgaaggacacttatgaggatgataatgcagtgcatattgtgatggaactttgtgaggggggtgagttgtttgataggattgttgccaggggacattatacagagagagcagctgcggttattatgaagactatagtagaagttgttcagatgtgtcatatgcatggagtaatgcatcgtgatctcaaacctgagaactttctgtttggtaacaagaaagaaactgctcctttgaaggctattgactttggattatcagtgttctttaaacccggggaacgctttaatgagattgtgggaagtccttattacatggctccagaggtcctaaaacgcaattatggcccggaggttgatgtctggagtgctggagttatcctttatattcttctttgtggtgttccacctttctgggcagagactgaacaaggagtagcccaagcaattattcggtctgtggttgatttcaagagagatccatggcctaaggtttctgataatgcaaaggatcttgtaaagaagatgcttgacccggatccaactcgacgactcacagctcagcaggttcttgagcacacctggttacaaaatataaagaaagcaccaaatgtctcattgggtgagactgtgaaagcaaggcttaaacaattttcagtaatgaacaagctcaagaaaagagctctaacgattatggccgagtttttatcagcggaagaagtggctggaatgaaggacgcatttgatatgatggatacaggaaagaaaggcaagattaaccttggagaacttaaaaatggtctgcaaaagcttggccatcagatccctgatgttgatcttcagattcttatggaagctgcggatgttgatggagatggaagcttaaattatggggagtttgttgctgtatctgttcatctcagaaaaatggcaaatgatgagcacctgcacaaagcattttcagtttttgacagagatcagagtggttacatagaaatcgaggagctgcgcagtgccttgagtgatgaggatggtggcaacagtgaggaagtcatcaatgccattatgcatgatgttgacactgacaaggatggccgcattagttacgaggaatttgctgcaatgatgaaggctggcacagattggagaaaagcatcgagacagtattctcgtgaaagattcaacagtctcagcttaaaattgatgagagatggctcgatacaagtcggaaaggaagaaggtagatga

SEQ ID NO: 2 - protein, 533 aa, Solanum lycopersicum
MGNCCGTPGNSSENKKKKNKPNPFALDYGATQASGGDGNKLVVLKDPTGHNIQEKYDLGCELGRGEFGVTYLCTDVDTGDKYACKSISKKKLRTAVDIDDVRREVEIMKHLPKHPNIVTLKDTYEDDNAVHIVMELCEGGELFDRIVARGHYTERAAAVIMKTIVEVVQMCHMHGVMHRDLKPENFLFGNKKETAPLKAIDFGLSVFFKPGERFNEIVGSPYYMAPEVLKRNYGPEVDVWSAGVILYILLCGVPPFWAETEQGVAQAIIRSVVDFKRDPWPKVSDNAKDLVKKMLDPDPTRRLTAQQVLEHTWLQNIKKAPNVSLGETVKARLKQFSVMNKLKKRALTIMAEFLSAEEVAGMKDAFDMMDTGKKGKINLGELKNGLQKLGHQIPDVDLQILMEAADVDGDGSLNYGEFVAVSVHLRKMANDEHLHKAFSVFDRDQSGYIEIEELRSALSDEDGGNSEEVINAIMHDVDTDKDGRISYEEFAAMMKAGTDWRKASRQYSRERFNSLSLKLMRDGSIQVGKEEGR

SEQ ID NO: 3 - DNA, 4914 bp, Solanum lycopersicum
  source 1..4914: mol_type = genomic DNA
atggggaattgctgtgggacacctggtaattcttctgagaataagaagaagaagaacaaaccaaacccttttgctcttgattatggtgcaactcaagcatctggaggtgatggaaacaagcttgttgtgttgaaagatccaacaggacacaatattcaagaaaaatatgatcttggttgtgagctaggaagaggagaatttggggttacatatttatgtactgatgttgatacaggggacaaatatgcttgcaaatcgatatcaaagaagaaacttaggactgctgtagatatagatgatgttaggagagaagttgagatcatgaagcatttgcctaaacatcctaatattgtgaccttgaaggacacttatgaggatgataatgcagtgcatattgtgatggaactttgtgaggggggtgagttgtttgataggattgttgccaggggacattatacagagagagcagctgcggttattatgaagactatagtagaagttgttcaggtacagttttactaattaatgcttgtctttgcttttcatctataattgttacttgtttgtttatttcatgtaatttaggggttgctaatttaggattatgttaatgaagtttgaattgacaatgccaactgaaagtgtcaatttagactagaaaggaatgttgagattgaagtttcatgtttgtaagcagaatgaatgttcttgtcgaagaatctcttttaagaatatctttcccacttcttcagtaaattttcctactttcttatgtcgataactgccactccttttctgagtttgcctgcactctcttggtagataggacactccctttcttagctcaggatctactttgcttgtgtaaatgagtgcttaatgtttttatttgattcattttacacgttgagatcctatagcatttaattagactagattttatcttccaatatcactaaacctagatgtcaaatatagtaaaaagttatgttgctcgaactcttcaaagatatcgacatgtgtgtgtcagatcctccaaaagtagtgcatttttggaggatccgacgggggtggggcaacaattttggagagttcgagcaacttaggtaaaaagtgtattcatgctctaaatgttgttaggttttctatctttcttatcttgtcttgtgaattttgctttcttggcaactgtttcattgtcctatatttttctcatgcaaatacctttaaaattatatactttcgtgccaaccatttaaatgaaacttaaggaagctaatcacacaggatttcaccatccaaatgtcgaaaatgaatcgcaatttgtgatagttttagacagagagcttatttttatagatgcaattagaataatagaaatgtaaaataactatcagtaaccagtaagatgccggtctttatggtctattttcagagggggagatctattgtagcttgctttcagcatcagttagtatagcataggactgttgctaacagggttcaattttaaactgtatttggtgaacataatgacatgagagctcaacttacataactacagattagagagagacattcattttatggaatggatttaagaagttcatgtttctacatttagttgttataagaacagggtggtaactggtaaccgacgcaaacatgatggctaattatcccaagtttatacaatttaatctatgtggttgctcatacatctttggtcaatgttcactttacagttgcattatgtttcctcaagaaatggctgttcttctttcaattttcaacttacggagtttcaattgacattgcagatgtgtcatatgcatggagtaatgcatcgtgatctcaaacctgagaactttctgtttggtaacaagaaagaaactgctcctttgaaggctattgactttggattatcagtgttctttaaacccggtaatgcaataagtaatgatagtgtgttgtaactttttttcatgctaaaaaagattaatgttggaatcatcttttaatatgtttaacaggggaacgctttaatgagattgtgggaagtccttattacatggctccagaggtcctaaaacgcaattatggcccggaggttgatgtctggagtgctggagttatcctttatattcttctttgtggtgttccacctttctgggcaggtccgtttcttttatttgccttctttaggtaacaagtaatacctcggttcaccgacaaataacaaagtaaatcaaccttggtgcatactattcatttcttagaacttggtaatttattaatgagtgtcaaaatgaaatggaatttgaaacatattgatgcgttgttaacatcgtcgatgactaggtgagggtggctgcaagagtgaatcccacctcttcctggaccaattcaaaatcaaagttcctttttttccttttggcctgtgatagtcagtactttgtgcttccattaatttactcacagctttctcagtaattgcctaaaattctactgaatatgtgcagagactgaacaaggagtagcccaagcaattattcggtctgtggttgatttcaagagagatccatggcctaaggtttctgataatgcaaaggatcttgtaaagaagatgcttgacccggatccaactcgacgactcacagctcagcaggttcttggtaatgtttgttaatccttgagatgctatactttcatttgcttgctgtttgttctctcttagtttcataagttcaattttgtgacttttttggggctttcgtgcatatacatgaatgcagagcacacctggttacaaaatataaagaaagcaccaaatgtctcattgggtgagactgtgaaagcaaggcttaaacaattttcagtaatgaacaagctcaagaaaagagctctaacggtaaaatattcccttttcatttgcagttacatatcattagcgttctgcaccttctcagaaggatatcttcatatgcctaattcttaaagcccaaaataaggacaaaagattttctgccttctcacaaaagtttcgggtgttatattctttcttcattgcttgcacagattatggccgagtttttatcagcggaagaagtggctggaatgaaggacgcatttgatatgatggatacaggaaagaaaggcaagattaaccttggagaacttaaaaatggtctgcaaaagcttggccatcagatccctgatgttgatcttcagattcttatggaagctgtaagcattctcatgctcttcatttcacttgattggattttctttcaactttacgaagactaaatatatatatttataagtcaagcgtctaatattattataattgttcccttttttatcttctgcttcacttttataggcggatgttgatggagatggaagcttaaattatggggagtttgttgctgtatctgttcatctcagaaaaatggcaaatgatgagcacctgcacaaagcattttcagtttttgacagagatcagagtggttacatagaaatcgaggagctgcgcagtgccttgagtgatgaggatggtggcaacagtgaggaagtcatcaatgccattatgcatgatgttgacactgacaaggttagaattttttttgtgtccattcatgtatatctactggatttcatactagtgcatatacttcttttataaatgtctctttaattgcttgtggaaccataaataccccccttatcttgttccgcagctccaactacacacgaaactatgttgaagacgtattacccccttgtacttgtaaaatgtgtatcttccgtcatcctgagaggcatatatgatgtaaccaaatgtgaacatttaagtatatgcatgtgctgcctcatgtcatttacccctttttcccttttcacttctcttccatctccgcaacatgttaatgtcctctagcaaatctgaaaaaagatggagtgagcttctcaacggaaaaaatcggattcaccctagttttagttttctggcaacataaacagctcaagtcgatacaaaaaaacaaatgttcctatcaaaaaactcaaattagtagaaaggaaaagaagggtcataggtaagggaagaacaaaaaggaatagaaagacccttcggggtggcccagttatttgggcttggggcttggggcttgggacttccatgttggaggtctcaagttcaaaaccccttgccaatgaaagcaacgggttttccttctacgttgactgtcgagctcgtcgcaccgggcttacctagtgcggtttacctctcctttgcgtgctataggaataggggttttaccctgtgtgcactcaaagggtagcgactgcggatttcccaaaagaaaaaggaagagaaaggtaaagaaaacattttaaaaaagagtaggatggttataatagaagaaatgctacaatattttttcacctcaggcgctttaagagagtaaatactctacgttacatggcgtcccaatgttgtcgtagttacattttggacaagaacagggagtaataggcctcccgcaaagttaaaatgtagtggggaatgggggaataattgaggaaggtatttatatattttctcctttctaaatcatattttcttttccattcactgctcttctgttcaaccttatcattcatttggactaaatgttgaattgattttgagcttttagtttgttaccacagcttcaaagttcatcagttacattgtctataaccatgcaggatggccgcattagttacgaggaatttgctgcaatgatgaaggctggcacagattggagaaaagcatcgagacagtattctcgtgaaagattcaacagtctcagcttaaaattgatgagagatggctcgatacaagtcggaaaggaagaaggtagatga

SEQ ID NO: 4 - DNA, 19 bp, Solanum lycopersicum
  source 1..19: mol_type = other DNA
ttggttgtgagctaggaag

SEQ ID NO: 5 - RNA, 76 nt, synthetic construct
  source 1..76: mol_type = other RNA
gttttagagctagaaatagcaagttaaaataaggctagtccgttatcaacttgaaaaagtggcaccgagtcggtgc

SEQ ID NO: 6 - DNA, 76 bp, synthetic construct
  source 1..76: mol_type = other DNA
gttttagagctagaaatagcaagttaaaataaggctagtccgttatcaacttgaaaaagtggcaccgagtcggtgc

SEQ ID NO: 7 - DNA, 20 bp, synthetic construct
  source 1..20: mol_type = other DNA
atggggaattgctgtgggac

SEQ ID NO: 8 - DNA, 27 bp, synthetic construct
  source 1..27: mol_type = other DNA
ttcataataaccgcagctgctctctct

SEQ ID NO: 9 - DNA, 1602 bp, Solanum lycopersicum
  source 1..1602: mol_type = other DNA
atgggtaattgctgtgtgaaaccgggtaaatctgccgaaaaaaagaataaaaagaacaacagcaaacctaaccctttttcaattgattatggggggactaaacatgcctctgggagtggaaacaagctagttgtattaaaagaaccaacagggcaaaatatacatgataagtatgatttggggcatgagctcggaagaggagaatttggggttacttatctatgtactgacttggaaggaggagaaaaatatgcttgcaaatcgatatctaaaaagaagctaaggactgcagtggatattgatgatgttaggagagaggttgagatcatgaaacatttgcctgtgcatccgaatattgtgaccttgaaggatacttatgaggatgataatgcagtgcacattgtgatggaattgtgtgagggtggggagttgtttgatcgaatcgttgctagaggccactatacagagagagcagctgctggaattttgaagactgtcgtggaagtcgttcagatgtgtcacaggcaaggggtaatgcatcgtgatctcaaacctgagaattttctttttggtaacaagaaagaaacagctccactgaaggctattgactttgggttgtctgttttctttaaacctggggaacgctttaatgagatagtgggaagtccttattacatggctcctgaggtcctaaagcgcaattatggaccagaggtcgatgtctggagtgctggagttatactttacattcttctatgcggtgttccacctttctgggcagagactgaacaaggagtagcccaagcgattattcgttctgtgattgatttcaagagggatccatggcctaaagtttctgataatgcaaaggatcttgtaaagaaaatgcttgatccagatccaactcgacggctcacagctcatcaagttcttgagcatccctggttacataatataaagaaagcaccaaacgtctcattgggtgagactgttaaagcaagactcaagcagttttcagtaatgaacaagctcaagaaaaaagctctgacggttatagctgagtttttgtctgcggaggaagtcgctggaatgaaggaagcatttgaaatgatggataccggaaagaagggcaagataaacctgaatgaacttaaagatggcttgcagaagcttggccatcaaatccctgatgctgatcttcatattctcatggaagcggctgacgttgatggagatggaagtttaaattatccagagtttgttgctgtatctattcatcttagaaagatggccaatgatgaacacctgcacaaagcattttcatttttcgacaaaaatcagagtggtttcatagaaatcgaagagcttcgtagtgctttgagggatgaagacgacagcaacagcgaggaagtcaccaatgccattatgcatgacgttgatacagacaaggatggtcggattagttatgaggaatttgctgcgatgatgaaggctggtacggactggagaaaagcatcgagacagtattctcgtgaacgttttaacagtctaagcttaaagttgatgagggaaggctcattacaagttgaaaacaaagtctag

SEQ ID NO: 10 - protein, 533 aa, Solanum lycopersicum
MGNCCVKPGKSAEKKNKKNNSKPNPFSIDYGGTKHASGSGNKLVVLKEPTGQNIHDKYDLGHELGRGEFGVTYLCTDLEGGEKYACKSISKKKLRTAVDIDDVRREVEIMKHLPVHPNIVTLKDTYEDDNAVHIVMELCEGGELFDRIVARGHYTERAAAGILKTVVEVVQMCHRQGVMHRDLKPENFLFGNKKETAPLKAIDFGLSVFFKPGERFNEIVGSPYYMAPEVLKRNYGPEVDVWSAGVILYILLCGVPPFWAETEQGVAQAIIRSVIDFKRDPWPKVSDNAKDLVKKMLDPDPTRRLTAHQVLEHPWLHNIKKAPNVSLGETVKARLKQFSVMNKLKKKALTVIAEFLSAEEVAGMKEAFEMMDTGKKGKINLNELKDGLQKLGHQIPDADLHILMEAADVDGDGSLNYPEFVAVSIHLRKMANDEHLHKAFSFFDKNQSGFIEIEELRSALRDEDDSNSEEVTNAIMHDVDTDKDGRISYEEFAAMMKAGTDWRKASRQYSRERFNSLSLKLMREGSLQVENKV

SEQ ID NO: 11 - DNA, 5526 bp, Solanum lycopersicum
  source 1..5526: mol_type = genomic DNA
atgggtaattgctgtgtgaaaccgggtaaatctgccgaaaaaaagaataaaaagaacaacagcaaacctaaccctttttcaattgattatggggggactaaacatgcctctgggagtggaaacaagctagttgtattaaaagaaccaacagggcaaaatatacatgataagtatgatttggggcatgagctcggaagaggagaatttggggttacttatctatgtactgacttggaaggaggagaaaaatatgcttgcaaatcgatatctaaaaagaagctaaggactgcagtggatattgatgatgttaggagagaggttgagatcatgaaacatttgcctgtgcatccgaatattgtgaccttgaaggatacttatgaggatgataatgcagtgcacattgtgatggaattgtgtgagggtggggagttgtttgatcgaatcgttgctagaggccactatacagagagagcagctgctggaattttgaagactgtcgtggaagtcgttcaggtatagtttttatcaacttcttagttctcagttacctactgcttttattaccttttgcttaggttatcttattatatccattattttcagcatagcttcttcattactgtatttccttttcatattgtttttatatatgtcttacttaggctgagggtccattggaaatagcctctctaccttcacaaggtaggagtaaggctgcgtacacactacccttcccacaccccacttgtgggactatactaagtatgttgttgttttagttctcaattgatgctttttggtttttatgtagtaacttgtggtgtttcttttactgagttcttcaaagcttttgtatgggttttatatcatgacggatgtatcctgtattgttgtttcgggtttttattaaagaagtctggcaatttcaagttaaaaagaaaatcatatcttaaaagagaagcctaatcttgagcaaatcttgagcagatagcaatttcagggtgaaatgtgaatattcttggtgaagttgcatatgaactggtaaccattattcaattcatttctagtgttgatctttgcaatcaatggtttcattctagtgtacgttcatgctgtagcatttaccttgatatcctcatggaatttcctttactgccaaaattataatgagaagtggttatcttttttaataatggtaaagtatgagaagaggttttcttatgttctcagtctttgctagttctatttctttactcgttttacttaacttttttagtttcttgtgaactgtagtattgctctatatcttctcactcaaattcatgttctaaatcttaaccattctagtgatataaatgaagttaattggtgatataggatatccccctccaaaatctaacaatctttcaactcatcatagtcttgggcagatagctagttagaaccgtaacaaatatttaggaaagtagatcattcgaaatagttatccttgtgaaatattattctttatcttcattattgaccattggttttcaaactctagtactcttaagtggaagactcacttcttgtttctgtggagtattagctatagcggcctacaacagaatttgattgttgcactcaaagttaaacagagttctacagtttagggaaatgataatggaatttaaatttagtttgtatactgaagtaaatatggttgacactatcagaaacaagtgctttttacttcaaatattgatctttatcctcattgcgaaccattgatgtccaaactgttttagatggaagagcaatttgttgttcatttgagtggaatagtcaccaacaacagctaattaactacgtatagcttagagagatgcgaaccaatggtaaatttaagttgtctcctgaagtagttactgattgttcatgataaaggtcattaaagttgaattctctatttagtcagtgtccttttctgcatcgactatatagtggcctgaatgacattacaaaatatttatgagttggtaggaatctttttttcatatgtgaatcatgaatgtgttcacaaatgatcaatcagagagtgattattgtattatgtggtgttgataacttttgaacttttcttcatttggtttgtgtttaactgttatctgaaaggcttggttggtggtactaaagctattggattagcagaaaactttatacatgtttatggtcatgtttcgctctccagtccccgtttttatttgtcaaaggtcagttcatatatttccaatggttttgcagatgtgtcacaggcaaggggtaatgcatcgtgatctcaaacctgagaattttctttttggtaacaagaaagaaacagctccactgaaggctattgactttgggttgtctgttttctttaaacctggtaatggaattggaaaaaaaacagtgagtttaagacttttatcatgctaaacaaaggtttaacatgttgattattttaacaggggaacgctttaatgagatagtgggaagtccttattacatggctcctgaggtcctaaagcgcaattatggaccagaggtcgatgtctggagtgctggagttatactttacattcttctatgcggtgttccacctttctgggcaggtctgcttattttatttcttcgttttttataaccatggaacgaacctcaatgcagatattttcatgtgcaatttttggaacttgataattgattaactaagattgtgaatatgaagtagaacttgattcatgttagaatatgttgttgaaatattagatgatgaggcaagtgaggtgaaagactgtccctgctttaatcaatgtagatcatgttcaattattttggtttctcttaatggttcttatgggttggactttgctaaataacttgcataaatatgttaacatattcttgatacttcccttaagttcctctgaatatttgcagagactgaacaaggagtagcccaagcgattattcgttctgtgattgatttcaagagggatccatggcctaaagtttctgataatgcaaaggatcttgtaaagaaaatgcttgatccagatccaactcgacggctcacagctcatcaagttcttggtaatgtttgtggaatattgagatattgtactttattcattcgttgttttactctctctctctctctctctctctctctatctatctctgataagtatttttttccggggctttgactcttgtggtgcagagcatccctggttacataatataaagaaagcaccaaacgtctcattgggtgagactgttaaagcaagactcaagcagttttcagtaatgaacaagctcaagaaaaaagctctgacggtaagcacacacttagtctgcaatcatatttataagctctggattcttcactgtccactaaagatgaattcatatgcttttcctcatagatcgaaatgaaggagagaaggttgtgtcttaattatttactgcactgccttgtgctatttaataaaaacttaattctcatcgtaaaaaatgagaggcggttctcaaaattttgatcaagtttcgtttttttatcttgatatatgtactttcttgtattccaaacaggttatagctgagtttttgtctgcggaggaagtcgctggaatgaaggaagcatttgaaatgatggataccggaaagaagggcaagataaacctgaatgaacttaaagatggcttgcagaagcttggccatcaaatccctgatgctgatcttcatattctcatggaagcggtaagcggtctcatgccctgcttcttggctcgatcagatttcttatagctctaccgggggtaacataatatttgaaagttagctgctaaacttttctgcctcaaagagaaaacaggtgcctgagatgatatggccatgtcttacgtagaactgtaaattacatcaatggacattattttaaaatgaccgaaaactacatggaatccatgtgaacttagtaaagaaaatattcaatggaagtaaaggataccaagtagttggattaaggctagattgttggtggtacactgacattagtgtctcaatgtttactaagagtctcagtttgattagagatttgcacgtagatgcagggataaccgtgagattaagaaaattttaagaaattcacggagatgaaaaagatctgtaatactcatatagcttagggccaagcccaactagtttgggatcaaatcgtagttgttgttgataagaatttagcattagacttttgtctgtcaccctactgtcaaaaaattgattgattacaaaatatattttgtcaatataagttgtaacatttttctaccatttcaatgtagaaaaaaggaaaatctgtagcaaaattagcttgacatttcgcttgtcttagcatccctggttcaatgcttattattatccagaaaggaaaaaaaaaacatttctcttgatccttttgcatcttcgacctgaaggatgcttatcttttttattattttatttccttgaacttttgttttatgtttttcttattctgtatcggttttacaggctgacgttgatggagatggaagtttaaattatccagagtttgttgctgtatctattcatcttagaaagatggccaatgatgaacacctgcacaaagcattttcatttttcgacaaaaatcagagtggtttcatagaaatcgaagagcttcgtagtgctttgagggatgaagacgacagcaacagcgaggaagtcaccaatgccattatgcatgacgttgatacagacaaggtcagtatgtccatttatgtgcacgtacaccatttagtaacttttcgttctttggttcatacttcatagtgcaaatattatgcattgttgctaatgtttacatcttaatgagttctcattttgaagttctcttctgaaccctcgtttgagtttagagctcaaatactccacctagttgtgacttattgtatctctaaagtccgtcatattatataaacgtattatactttgatggcatgcacactttctagcacatatgtgttgctaacgaaactctagtgctgtgacaaatgaaatacatgtatacattgatggcatctgttcttcccatcacatatgtactaccggtcattactctctagtgctgtgacattatgctctccctgttcgcttcatgagttacacggttggttaacctgctgctcgttacatgtctgctacagaattcaagttttgttagctgttttccatctcatctctaacaacatccccactcatttgtattagcttcttatctggagttttgtgagctcagtcttgtatcgtcttgtgtcaaaacgtgtgcaggatggtcggattagttatgaggaatttgctgcgatgatgaaggctggtacggactggagaaaagcatcgagacagtattctcgtgaacgttttaacagtctaagcttaaagttgatgagggaaggctcattacaagttgaaaacaaagtctag

SEQ ID NO: 12 - DNA, 19 bp, Solanum lycopersicum
  source 1..19: mol_type = other DNA
tggggcatgagctcggaag

SEQ ID NO: 13 - RNA, 76 nt, synthetic construct; identical to SEQ ID NO: 5
  source 1..76: mol_type = other RNA

SEQ ID NO: 14 - DNA, 76 bp, synthetic construct; identical to SEQ ID NO: 6
  source 1..76: mol_type = other DNA

SEQ ID NO: 15 - DNA, 22 bp, synthetic construct
  source 1..22: mol_type = other DNA
agaacaacagcaaacctaaccc

SEQ ID NO: 16 - DNA, 20 bp, synthetic construct
  source 1..20: mol_type = other DNA
tccagcagctgctctctctg

SEQ ID NO: 17 - DNA, 2418 bp, Solanum lycopersicum
  source 1..2418: mol_type = other DNA
atggctcaacgtgttctaactcgtgttcacagtcttcgtgaacgtcttgatgctactttggatgctcatcgcaatgaaattttgctctttctttcaaggatcgaaagccacgggaaagggatcttgaaacctcaccagctactggctgagtttgaatcaattcagaaagaagacaaagacaaactgaatgatcatgcctttgaagaagtcctgaaatccactcaggaagcaattgttttgcccccatgggttgcacttgctattcgtttgaggcccggtgtgtgggaatatgtccgtgtgaatgttaatgctcttagtgttgaggagctgactgtgcctgagtttttgcaattcaaggaagaacttgttaacggaacttccagtgataactttgttcttgaattggattttgagcccttcactgcatcatttccaaaaccaaccctcacgaaatcaattggaaatggagttgaattcctcaacaggcacctctctgctaaaatgttccatgacaaggaaagcatgacccctcttctcgagtttcttcgagttcaccactacaatggaaagtcaatgatgctgaatgatagaattcagaatttgtatactctccaaaaagtcctgaggaaggccgaggaatacctcaccaccctttcgccagaaacttcatactcctcatttgagcacaagttccaagaaattggcttggagagaggttggggtgacaccgcagagcgtgttctagagatgatctgcatgctcctggatctccttgaggctcctgactcatgtactcttgagaagttccttagtagaattcctatggttttcaatgtagttatactttcacctcatggatatttcgcccaggaaaatgtcttgggttaccccgacactggtggtcaggttgtctatattttggatcaagttcctgccttggagcgtgagatgctcaagcgcataaaggagcaaggacttgatatcaaaccgcgtattcttattgttactcggcttctccctgatgcagttggtaccacttgtggtcagcgactcgagaaggtatttggaactgagcattcacatattcttagggtcccctttaggactgaaaagggcattgttcgcaaatggatctctcgttttgaagtctggccatacatggagactttcattgaggatgtggggaaagaaataaccgcagaactgcaagctaagccagatcttattattggaaactatagtgagggaaaccttgcagcctccttgttggctcacaagttaggtgtaacacagtgcaccattgctcatgcattggagaaaaccaaatatcctgattctgacatttacttgaacaaatttgacgagaaataccacttctcagctcagttcacagctgatcttatagcaatgaatcatactgatttcattatcaccagcaccttccaggagatagcaggaagcaaggacactgttggacagtatgagagccacatggccttcacaatgcctggattgtatagagttgttcatggcattgatgtgttcgaccccaaattcaacattgtgtcaccaggagctgatgtgaatctctatttcccatactccgaaaaggaaaagagattgacaacttttcaccctgaaattgaagacttgctgtttagcgatgttgagaacgaagaacacctgtgtgtgttgaaggacaggaataagcccatcatattcaccatggcaagattggaccgagtgaagaacttaactggacttgtcgagtggtatgctaagaatccacgactaagggagttggttaaccttgtagtggttggtggagaccgaagaaaggaatccaaagacttggaagagcaggcagagatgaagaagatgtatgaacttataaagactcacaatttgaatggccagttccgatggatttcttcccagatgaaccgcgtgaggaatggggaactctacaggtacattgctgacacaaggggagctttcgtgcagcctgcattctacgaggctttcggtctgactgttgttgaggccatgagctgcggtttgcctacatttgcaactaatcaaggtggtccagctgagatcatcgttcatggaaagtctggtttccaaattgatccataccatggcgagcaggctgctgatctcctcgctgagttcttcgagaaatgtaaggtagacccttcacattgggaagccatttccaagggtggccttaagcgtatacaggagaagtacacatggcaaatctactccgaccggctgttgacactagctgctgtttacgggttctggaagcacgtttccaagcttgatcgtcttgaaattcgtcgttatcttgagatgttttacgctctcaaattccgcaagctggctgaacttgtcccattggctgttgagtaa

SEQ ID NO: 18 - protein, 805 aa, Solanum lycopersicum
MAQRVLTRVHSLRERLDATLDAHRNEILLFLSRIESHGKGILKPHQLLAEFESIQKEDKDKLNDHAFEEVLKSTQEAIVLPPWVALAIRLRPGVWEYVRVNVNALSVEELTVPEFLQFKEELVNGTSSDNFVLELDFEPFTASFPKPTLTKSIGNGVEFLNRHLSAKMFHDKESMTPLLEFLRVHHYNGKSMMLNDRIQNLYTLQKVLRKAEEYLTTLSPETSYSSFEHKFQEIGLERGWGDTAERVLEMICMLLDLLEAPDSCTLEKFLSRIPMVFNVVILSPHGYFAQENVLGYPDTGGQVVYILDQVPALEREMLKRIKEQGLDIKPRILIVTRLLPDAVGTTCGQRLEKVFGTEHSHILRVPFRTEKGIVRKWISRFEVWPYMETFIEDVGKEITAELQAKPDLIIGNYSEGNLAASLLAHKLGVTQCTIAHALEKTKYPDSDIYLNKFDEKYHFSAQFTADLIAMNHTDFIITSTFQEIAGSKDTVGQYESHMAFTMPGLYRVVHGIDVFDPKFNIVSPGADVNLYFPYSEKEKRLTTFHPEIEDLLFSDVENEEHLCVLKDRNKPIIFTMARLDRVKNLTGLVEWYAKNPRLRELVNLVVVGGDRRKESKDLEEQAEMKKMYELIKTHNLNGQFRWISSQMNRVRNGELYRYIADTRGAFVQPAFYEAFGLTVVEAMSCGLPTFATNQGGPAEIIVHGKSGFQIDPYHGEQAADLLAEFFEKCKVDPSHWEAISKGGLKRIQEKYTWQIYSDRLLTLAAVYGFWKHVSKLDRLEIRRYLEMFYALKFRKLAELVPLAVE

SEQ ID NO: 19 - DNA, 3869 bp, Solanum lycopersicum
  source 1..3869: mol_type = genomic DNA
atggctcaacgtgttctaactcgtgttcacagtcttcgtgaacgtcttgatgctactttggatgctcatcgcaatgaaattttgctctttctttcaaggtatggtcttacagccatgttttcgctttttgtaattttcgtttggtatgtttcgcaagcctaaatagttttggggatacaaacttagtactgccttattcctttgtttggttattgatctcggaataagttatatcagaattagtaattagtacctcgataagttatctctgatggaataatagtactgttaactagtaatcctggaacaatacaatgaaaatgacaaaaatcccccagaggtcccttagatccttttttacttaataaggtggaaggtattctcgtaaacaaataactttcgttcttaaaaattatgcaatgaatgtttgtcctagtaaaacttgtcttcaaaccaaacgacccctaattgacggacaaatatatggttccatcaagtacatcatgagttattcttgctgtttttggctgtatcaggatcgaaagccacgggaaagggatcttgaaacctcaccagctactggctgagtttgaatcaattcagaaagaagacaaagacaaactgaatgatcatgcctttgaagaagtcctgaaatccactcaggtaacttggttttgttgttaggttgattatatttaattttcttactaagctaacatgtgtatctgtttgtacttgcatttgaaattttcttttgcgttgttcgtcatactaggaagcaattgttttgcccccatgggttgcacttgctattcgtttgaggcccggtgtgtgggaatatgtccgtgtgaatgttaatgctcttagtgttgaggagctgactgtgcctgagtttttgcaattcaaggaagaacttgttaacggaacgtaagttttacgtttgaatttgatgatgagttatctaatcaacatgttcttagaatctttttgattaatgttgtgattttccctgatgcagttccagtgataactttgttcttgaattggattttgagcccttcactgcatcatttccaaaaccaaccctcacgaaatcaattggaaatggagttgaattcctcaacaggcacctctctgctaaaatgttccatgacaaggaaagcatgacccctcttctcgagtttcttcgagttcaccactacaatggaaaggtaaatttagtgttatggtggtttttctccgataaatttcgagtatggagttactgatttttgcatccaacaaatgattaacatgttcgaacaatcattttctgtgcagtcaatgatgctgaatgatagaattcagaatttgtatactctccaaaaagtcctgaggaaggccgaggaatacctcaccaccctttcgccagaaacttcatactcctcatttgagcacaagttccaagaaattggcttggagagaggttggggtgacaccgcagagcgtgttctagagatgatctgcatgctcctggatctccttgaggctcctgactcatgtactcttgagaagttccttagtagaattcctatggttttcaatgtagttatactttcacctcatggatatttcgcccaggaaaatgtcttgggttaccccgacactggtggtcaggtgcattgcttatttgtgatcactttgtcttactccttagaaacctattggggcaagtgctgagttcccgttcctttaatttgcaggttgtctatattttggatcaagttcctgccttggagcgtgagatgctcaagcgcataaaggagcaaggacttgatatcaaaccgcgtattcttattgttagtattctcagagattgtgcttatagattatgattatgcaggattttgatttgttctaatgcaacatctgatctttgtttaaattctcaggttactcggcttctccctgatgcagttggtaccacttgtggtcagcgactcgagaaggtatttggaactgagcattcacatattcttagggtcccctttaggactgaaaagggcattgttcgcaaatggatctctcgttttgaagtctggccatacatggagactttcattgaggtgaagcaacttttctgtattcatttttcagtcttctagttgatttttgcagcaattttctacttacactaaaactgtgactttaatacattaggatgtggggaaagaaataaccgcagaactgcaagctaagccagatcttattattggaaactatagtgagggaaaccttgcagcctccttgttggctcacaagttaggtgtaacacaggtctgtaacattggtcacatgtataagattgactttgcatttcctttcatttggaactcggagttattaagaattctcttttgcgttgatctgcagtgcaccattgctcatgcattggagaaaaccaaatatcctgattctgacatttacttgaacaaatttgacgagaaataccacttctcagctcagttcacagctgatcttatagcaatgaatcatactgatttcattatcaccagcaccttccaggagatagcaggaaggtatgacatcaattcgctctatgattaaattgttcttcttcctgtttcattgtgtttgatcctaaaacatttttcaattttctttagcaaggacactgttggacagtatgagagccacatggccttcacaatgcctggattgtatagagttgttcatggcattgatgtgttcgaccccaaattcaacattgtgtcaccaggagctgatgtgaatctctatttcccatactccgaaaaggaaaagagattgacaacttttcaccctgaaattgaagacttgctgtttagcgatgttgagaacgaagaacacctgtatgtttctataatagtgcaacattgtgtttactgatataaacaagcttgtactgaaatagatttgtgttcctatatcaggtgtgtgttgaaggacaggaataagcccatcatattcaccatggcaagattggaccgagtgaagaacttaactggacttgtcgagtggtatgctaagaatccacgactaagggagttggttaaccttgtagtggttggtggagaccgaagaaaggaatccaaagacttggaagagcaggcagagatgaagaagatgtatgaacttataaagactcacaatttgaatggccagttccgatggatttcttcccagatgaaccgcgtgaggaatggggaactctacaggtacattgctgacacaaggggagctttcgtgcagcctgcattctacgaggctttcggtctgactgttgttgaggccatgagctgcggtttgcctacatttgcaactaatcaaggtggtccagctgagatcatcgttcatggaaagtctggtttccaaattgatccataccatggcgagcaggctgctgatctcctcgctgagttcttcgagaaatgtaaggtagacccttcacattgggaagccatttccaagggtggccttaagcgtatacaggagaagtaagctgctcatcttttcgtcctatcacgtgatcactattgagtgcattaattcaaagtgattctaatctcctgttgctgtaggtacacatggcaaatctactccgaccggctgttgacactagctgctgtttacgggttctggaagcacgtttccaagcttgatcgtcttgaaattcgtcgttatcttgagatgttttacgctctcaaattccgcaagctggtatgtctctctgctttctgcacttgtccaatagtctaaagcaactgttaatggagcttctgtattttgttttgattcaggctgaacttgtcccattggctgttgagtaa

SEQ ID NO: 20 - DNA, 21 bp, synthetic construct
  source 1..21: mol_type = other DNA
atggcatcctcatattgagat

SEQ ID NO: 21 - DNA, 20 bp, synthetic construct
  source 1..20: mol_type = other DNA
tattcctcggccttcctcag

SEQ ID NO: 22 - DNA, 12 bp, synthetic construct
  source 1..12: mol_type = other DNA
ttgttgttgttg

SEQ ID NO: 23 - DNA, 4897 bp, Solanum lycopersicum
  source 1..4897: mol_type = genomic DNA
atggggaattgctgtgggacacctggtaattcttctgagaataagaagaagaacaaaccaaacccgtttgctcttgattatggtgcaactcaagcatctggaggtgatggaaacaagcttgttgtgttgaaagatccaacaggacacaatattcaagaaaaatatgatcttggttgtgagctaggaagaggagaatttggggttacatatttatgtactgatgttgatacaggggacaaatatgcttgcaaatcgatatcgaagaagaaacttaggactgctgtagatatagatgatgttaggagagaagttgagatcatgaagcatttgcctaaacatcctaatattgtgaccttgaaggacacttatgaggatgataatgcagtgcatattgtgatggaactttgtgaggggggtgagttgtttgataggattgttgccaggggacattatacagagagagcagctgcggttgttatgaagactatagtagaagttgttcaggtacagttttactaattgatgcttgtctttgcttttcatctataattgttacttgtttgtttatttcatgtaatttaggggttgctaatttaggattatgttaatgaagtttgaattgacaatgccaactgaaagtatcaatttagactagaaaggaatgttgagattgaagtttcatgtttgtaagcagaatgaatgttcttgtcgaagaatctcttttaagaatatctttcccacttcttcagtaaattttcctactttcttatgtcgataactgccactccttttctgagtttgcctgcactctcttggtagataggacactccctttcttagctcaggatttactttgcttgtgtaaatgagtgcttaatgtttttatttgattcattttacacgttgagatcctatagcatttaattagactagattttatcttccaatatcactaaacctagatgtcaaatatagtaaaaagctatgttgctcgaactcttcaaagatatcgacatgtgtgtgtcagatcctccaaaagtagtgcatttttggaggatccgacgggggtggggcaacaattttggagagttcgagcaacttaggtaaaaagtgtattcatgctctaaatgttgttaggttttctatctttcttatcttgtcttgtgaattttgctttcttggcaactgtttcattgtcctatatttttctcatgcaaatacctttaaaattatatactttcgtgccaaccatttaaatgaaacttaaggaagctaatcacacaggatttcaccatccaaatgtcgaaaatgaatcgcaatttgtgatagttttagacagagagcttatttttatagatgcaattagaataatagaaatgtaaaataactatcagtaaccagtaagatgccggtctttatggtctattttcagagggggagatctattgtagcttgctttcagcatcagttagtatagcataggactgttgctaacagggttcaattttaaactgtatttggtgaacataatgacatgagagctcaacttacataactacagattagagagagacattcattttatggaatggatttaagaagttcatgtttctacatttagttgttataagaacagggtggtaactggtaaccgacgcaaacatgatggctaattatcccaagtttatacaatttaatctatgtggttgctcatacatctttggtcaatgttcactttacagttgcattatgtttcctcaagaaatggctgttcttctttcaattttcaacttacggagtttcaattgacattgcagatgtgtcatatgcatggagtaatgcatcgtgatctcaaacctgagaactttctgtttggtaacaagaaagaaattgctcctttgaaggctattgactttggattatcagtgttctttaaacccggtaatgcaataagtaatgatagtgtgttgtaactttttttcatgctaaaaaagattaatgttggaatcatcttttaatatgtttaacaggggaacggtttaatgagattgtgggaagtccttattacatggctccagaggtcctaaaacgcaattatggcccggaggttgatgtctggagtgctggagttatcctttatattcttctttgtggtgttccacctttctgggcaggtccgtttcttttatttgccttctttaggtaacaagtaatacctcggttcaccgacaaataacaaattaaatcaaccttggtgcatactattcatttcttagaacttggtaatttattaatgagtgtcaaaatgaaatggaatttgaaacatattgatgcgttgttaacatcgtcgatgactaggtgagggtggctgcaagagtgaatcccacctcttcctggaccaattcaaaatcaaagttcctttttttccttttggcctgtgatagtcagtactttgtgcttccattaatttactcacagctttctcagtaattgcctaaaattctactgaatatgtgcagagactgaacaaggagtagcccaagcaattattcggtctgtggttgatttcaagagagatccatggcctaaggtttctgataatgcaaaggatcttgtaaagaagatgcttgacccggatccaactcgacgactcacagctcagcaggttcttggtaatgtttgttaatccttgagatgctatactttcatttgcttgctgtttgttctctcttagtttcataagttcaattttgtgacttttttggggctttcgtgcatatacatgaatgcagagcacacctggttacaaaatataaagaaagcaccaaatgtctcattgggtgagactgtgaaagcaaggcttaaacaattttcagtaatgaacaagctcaagaaaagagctctaacggtaaaatattcccttttcatttgcagttacatatcattagcgttctgcaccttctcagaaggatatcttcatatgcctaattcttaaagcccaaaataaggacaaaagattttctgccttctcacaaaagtttcgggtgttatattctttcttcattgcttgcacagattatggccgagtttttatcagcggaagaagtggctggaatgaaggacgcatttgatatgatggatacaggaaagaaaggcaagattaaccttggagaacttaaaaatggtctgcaaaagcttggccatcagatccctgatgttgatcttcagattcttatggaagctgtaagcattctcatgctcttcatttcacttgattggattttctttcaactttacgaagactaaatatatatatttataagtcaagcgtctaatattattataattgttccctttttgatcttctgcttcacttttataggcggatgttgatggagatggaagcttaaattatggggagtttgttgctgtatctgttcatctcagaaaaatggcaaatgatgagcacctgcacaaagcattttcagttttcgacagagatcagagtggttacatagaaatcgaggagctgcgcagtgccttgagtgatgaggatggtggcaacagtgaggaagtcatcaatgccattatgcatgatgttgacactgacaaggttagaattttttttgtgtccattcatgtatatctactggatttcatactagtgcatatacttctcttataaatgtctctttaattgcttgtggaaccataaataccccccttatcttgttccgcagttccaactacacacgaaactatgttgaagacgtattacccccttgtacttgtaaaatgtgtatcttccgtcatcctgagaggcatatatgatgtaaccaaatgtgaacatttaagtatatgcatgtgctgcctcatgtcatttacccctttttcccttttcacttctcttccatctccgcaacatgttaatgtcctctagcaaatctgaaaaaagatggagtgagcttctcaacggaaaaaatcggattcaccctagttttagttttctggcaacataaacagctcaagtcgatacaaaaaaacaaatgttcctatcaaaaaactcaaattagtagaaaggaaaagaagggtcataggtaagggaagaacaaaaaggaatagaaagacccttcggggtggcccagttatttgggcttggggcttccatgttggaggtctcaagttcaaaaccccttgccaatgaaagcaacgggttttccttctacgttgactgtcgagctcgtcgcaccgggcttacctagtgcggtttacctctcctttgcgtgctataggaataggggttttaccctgtgtgcactcaaagggtagcgactgcggatttcccaaaagaaaaaggaagagaaaggtaaagaaaacattttaaaaaagagtaggatggttataatagaagaaatgctataatattttttcacctcaggcgctttaagagagtaaatactctacgttacatggcgtcccaatgttgtcgtagttacattttggacaagaacagggagtaataggcctcccgcaaagttaaaatgtagtagggaatgggggaataattgaggaaggtatttatatattttctcctttctaaatcatattttcttttccattcactgctcttctgttcaaccttatcattcatttggactaaatgttgaattgattttgagcttttagtttgttaccacagcttcaaagttcatcagttacattgtctataaccatgcaggatggccgcattagttacgaggaatttgctgcaatgatgaaggctggcacagattggagaaaagcatcgagacagtattctcgtgaaagattcaacagtctcagcttaaaattgatgagagatggctcgatacaagtcggaaaggaagaaggtagatga

SEQ ID NO: 24 - DNA, 4914 bp, Solanum lycopersicum
  source 1..4914: mol_type = genomic DNA
atggggaattgctgtgggacacctggtaattcttctgagaataagaagaagaagaacaaaccaaacccttttgctcttgattatggtgcaactcaagcatctggaggtgatggaaacaagcttgttgtgttgaaagatccaacaggacacaatattcaagaaaaatatgatcttggttgtgagctaggaagaggagaatttggggttacatatttatgtactgatgttgatacaggggacaaatatgcttgcaaatcgatatcaaagaagaaacttaggactgctgtagatatagatgatgttaggagagaagttgagatcatgaagcatttgcctaaacatcctaatattgtgaccttgaaggacacttatgaggatgataatgcagtgcatattgtgatggaactttgtgaggggggtgagttgtttgataggattgttgccaggggacattatacagagagagcagctgcggttattatgaagactatagtagaagttgttcaggtacagttttactaattaatgcttgtctttgcttttcatctataattgttacttgtttgtttatttcatgtaatttaggggttgctaatttaggattatgttaatgaagtttgaattgacaatgccaactgaaagtgtcaatttagactagaaaggaatgttgagattgaagtttcatgtttgtaagcagaatgaatgttcttgtcgaagaatctcttttaagaatatctttcccacttcttcagtaaattttcctactttcttatgtcgataactgccactccttttctgagtttgcctgcactctcttggtagataggacactccctttcttagctcaggatctactttgcttgtgtaaatgagtgcttaatgtttttatttgattcattttacacgttgagatcctatagcatttaattagactagattttatcttccaatatcactaaacctagatgtcaaatatagtaaaaagttatgttgctcgaactcttcaaagatatcgacatgtgtgtgtcagatcctccaaaagtagtgcatttttggaggatccgacgggggtggggcaacaattttggagagttcgagcaacttaggtaaaaagtgtattcatgctctaaatgttgttaggttttctatctttcttatcttgtcttgtgaattttgctttcttggcaactgtttcattgtcctatatttttctcatgcaaatacctttaaaattatatactttcgtgccaaccatttaaatgaaacttaaggaagctaatcacacaggatttcaccatccaaatgtcgaaaatgaatcgcaatttgtgatagttttagacagagagcttatttttatagatgcaattagaataatagaaatgtaaaataactatcagtaaccagtaagttgccggtctttatggtctattttcagagggggagatctattgtagcttgctttcagcatcagttagtatagcataggactgttgctaacagggttcaattttaaactgtatttggtgaacataatgacatgagagctcaacttacacaactacagattagagagagacattcattttatggaatggatttaagaagttcatgtttctacatttagttgttataagaacagggtggtaactggtaaccgacgcaaacatgatggctaattatcccaagtttatacaatttaatctatgtggttgctcatacatctttggtcaatgttcactttacagttgcattatgtttcctcaagaaatggctgttcttctttcaattttcaacttacggagtttcaattgacattgcagatgtgtcatatgcatggagtaatgcatcgtgatctcaaacctgagaactttctgtttggtaacaagaaagaaactgctcctttgaaggctattgactttggattatcagtgttctttaaacccggtaatgcaataagtaatgatagtgtgttgtaactttttttcatgctaaaaaagattaatgttggaatcatcttttaatatgtttaacaggggaacgctttaatgagattgtgggaagtccttattacatggctccagaggtcctaaaacgcaattatggcccggaggttgatgtctggagtgctggagttatcctttatattcttctttgtggtgttccacctttctgggcaggtccgtttcttttatttgccttctttaggtaacaagtaatacctcggttcaccgacaaataacaaagtaaatcaaccttggtgcatactattcatttcttagaacttggtaatttattaatgagtgtcaaaatgaaatggaatttgaaacatattgatgcgttgttaacatcgtcgatgactaggtgagggtggctgcaagagtgaatcccacctcttcctggaccaattcaaaatcaaagttcctttttttccttttggcctgtgatagtcagtactttgtgcttccattaatttactcacagctttctcagtaattgcctaaaattctactgaatatgtgcagagactgaacaaggagtagcccaagcaattattcggtctgtggttgatttcaagagagatccatggcctaaggtttctgataatgcaaaggatcttgtaaagaagatgcttgacccggatccaactcgacgactcacagctcagcaggttcttggtaatgtttgttaatccttgagatgctatactttcatttgcttgctgtttgttctctcttagtttcataagttcaattttgtgacttttttggggctttcgtgcatatacatgaatgcagagcacacctggttacaaaatataaagaaagcaccaaatgtctcattgggtgagactgtgaaagcaaggcttaaacaattttcagtaatgaacaagctcaagaaaagagctctaacggtaaaatattcccttttcatttgcagttacatatcattagcgttctgcaccttctcagaaggatatcttcatatgcctaattcttaaagcccaaaataaggacaaaagattttctgccttctcacaaaagtttcgggtgttatattctttcttcattgcttgcacagattatggccgagtttttatcagcggaagaagtggctggaatgaaggacgcatttgatatgatggatacaggaaagaaaggcaagattaaccttggagaacttaaaaatggtctgcaaaagcttggccatcagatccctgatgttgatcttcagattcttatggaagctgtaagcattctcatgctcttcatttcacttgattggattttctttcaactttacgaagactaaatatatatatttataagtcaagcgtctaatattattataattgttcccttttttatcttctgcttcacttttataggcggatgttgatggagatggaagcttaaattatggggagtttgttgctgtatctgttcatctcagaaaaatggcaaatgatgagcacctgcacaaagcattttcagtttttgacagagatcagagtggttacatagaaatcgaggagctgcgcagtgccttgagtgatgaggatggtggcaacagtgaggaagtcatcaatgccattatgcatgatgttgacactgacaaggttagaattttttttgtgtccattcatgtatatctactggatttcatactagtgcatatacttctcttataaatgtctctttaattgcttgtggaaccataaataccccccttatcttgttccgcagctccaactacacacgaaactatgttgaagacgtattacccccttgtacttgtaaaatgtgtatcttccgtcatcctgagaggcatatatgatgtaaccaaatgtgaacatttaagtatatgcatgtgctgcctcatgtcatttacccctttttcccttttcacttctcttccatctccgcaacatgttaatgtcctctagcaaatctgaaaaaagatggagtgagcttctcaacggaaaaaatcggattcaccctagttttagttttctggcaacataaacagctcaagtcgatacaaaaaaacaaatgttcctatcaaaaaattcaaattagtagaaaggaaaagaagggtcataggtaagggaagaacaaaaaggaatagaaagacccttcggggtggcccagttatttgggcttggggcttggggcttgggacttccatgttggaggtctcaagttcaaaaccccttgccaatgaaagcaacgggttttccttctacgttgactgtcgagctcgtcgcaccgggcttacctagtgcggtttacctctcctttgcgtgctataggaataggggttttaccctgtgtgcactcaaagggtagcgactgcggatttcccaaaagaaaaaggaagagaaaggtaaagaaaacattttaaaaaagagtaggatggttataatagaagaaatgctacaatattttttcacctcaggcgctttaagagagtaaatactctacgttacatggcgtcccaatgttgtcgtagttacattttggacaagaacagggagtaataggcctcccgcaaagttaaaatgtagtggggaatgggggaataattgaggaaggtatttatatattttctcctttctaaatcatattttcttttccattcactgctcttctgttcaaccttatcattcatttggactaaatgttgaattgattttgagcttttagtttgttaccacagcttcaaagttcatcagttacattgtctataaccatgcaggatggccgcattagttacgaggaatttgctgcaatgatgaaggctggcacagattggagaaaagcatcgagacagtattctcgtgaaagattcaacagtctcagcttaaaattgatgagagatggctcgatacaagtcggaaaggaagaaggtagatga

SEQ ID NO: 25 - DNA, 4897 bp, Solanum lycopersicum
  source 1..4897: mol_type = genomic DNA
atggggaattgctgtgggacacctggtaattcttctgagaataagaagaagaacaaaccaaacccgtttgctcttgattatggtgcaactcaagcatctggaggtgatggaaacaagcttgttgtgttgaaagatccaacaggacacaatattcaagaaaaatatgatcttggttgtgagctaggaagaggagaatttggggttacatatttatgtactgatgttgatacaggggacaaatatgcttgcaaatcgatatcgaagaagaaacttaggactgctgtagatatagatgatgttaggagagaagttgagatcatgaagcatttgcctaaacatcctaatattgtgaccttgaaggacacttatgaggatgataatgcagtgcatattgtgatggaactttgtgaggggggtgagttgtttgataggattgttgccaggggacattatacagagagagcagctgcggttattatgaagactatagtagaagttgttcaggtacagttttactaattgatgcttgtctttgcttttcatctataattgttacttgtttgtttatttcatgtaatttaggggttgctaatttaggattatgttaatgaagtttgaattgacaatgccaactgaaagtatcaatttagactagaaaggaatgttgagattgaagtttcatgtttgtaagcagaatgaatgttcttgtcgaagaatctcttttaagaatatctttcccacttcttcagtaaattttcctactttcttatgtcgataactgccactccttttctgagtttgcctgcactctcttggtagataggacactccctttcttagctcaggatttactttgcttgtgtaaatgagtgcttaatgtttttatttgattcattttacacgttgagatcctatagcatttaattagactagattttatcttccaatatcactaaacctagatgtcaaatatagtaaaaagctatgttgctcgaactcttcaaagatatcgacatgtgtgtgtcagatcctccaaaagtagtgcatttttggaggatccgacgggggtggggcaacaattttggagagttcgagcaacttaggtaaaaagtgtattcatgctctaaatgttgttaggttttctatctttcttatcttgtcttgtgaattttgctttcttggcaactgtttcattgtcctatatttttctcatgcaaatacctttaaaattatatactttcgtgccaaccatttaaatgaaacttaaggaagctaatcacacaggatttcaccatccaaatgtcgaaaatgaatcgcaatttgtgatagttttagacagagagcttatttttatagatgcaattagaataatagaaatgtaaaataactatcagtaaccagtaagatgccggtctttatggtctattttcagagggggagatctattgtagcttgctttcagcatcagttagtatagcataggactgttgctaacagggttcaattttaaactgtatttggtgaacataatgacatgagagctcaacttacataactacagattagagagagacattcattttatggaatggatttaagaagttcatgtttctacatttagttgttataagaacagggtggtaactggtaaccgacgcaaacatgatggctaattatcccaagtttatacaatttaatctatgtggttgctcatacatctttggtcaatgttcactttacagttgcattatgtttcctcaagaaatggctgttcttctttcaattttcaacttacggagtttcaattgacattgcagatgtgtcatatgcatggagtaatgcatcgtgatctcaaacctgagaactttctgtttggtaacaagaaagaaattgctcctttgaaggctattgactttggattatcagtgttctttaaacccggtaatgcaataagtaatgatagtgtgttgtaactttttttcatgctaaaaaagattaatgttggaatcatcttttaatatgtttaacaggggaacggtttaatgagattgtgggaagtccttattacatggctccagaggtcctaaaacgcaattatggcccggaggttgatgtctggagtgctggagttatcctttatattcttctttgtggtgttccacctttctgggcaggtccgtttcttttatttgccttctttaggtaacaagtaatacctcggttcaccgacaaataacaaattaaatcaaccttggtgcatactattcatttcttagaacttggtaatttattaatgagtgtcaaaatgaaatggaatttgaaacatattgatgcgttgttaacatcgtcgatgactaggtgagggtggctgcaagagtgaatcccacctcttcctggaccaattcaaaatcaaagttcctttttttccttttggcctgtgatagtcagtactttgtgcttccattaatttactcacagctttctcagtaattgcctaaaattctactgaatatgtgcagagactgaacaaggagtagcccaagcaattattcggtctgtggttgatttcaagagagatccatggcctaaggtttctgataatgcaaaggatcttgtaaagaagatgcttgacccggatccaactcgacgactcacagctcagcaggttcttggtaatgtttgttaatccttgagatgctatactttcatttgcttgctgtttgttctctcttagtttcataagttcaattttgtgacttttttggggctttcgtgcatatacatgaatgcagagcacacctggttacaaaatataaagaaagcaccaaatgtctcattgggtgagactgtgaaagcaaggcttaaacaattttcagtaatgaacaagctcaagaaaagagctctaacggtaaaatattcccttttcatttgcagttacatatcattagcgttctgcaccttctcagaaggatatcttcatatgcctaattcttaaagcccaaaataaggacaaaagattttctgccttctcacaaaagtttcgggtgttatattctttcttcattgcttgcacagattatggccgagtttttatcagcggaagaagtggctggaatgaaggacgcatttgatatgatggatacaggaaagaaaggcaagattaaccttggagaacttaaaaatggtctgcaaaagcttggccatcagatccctgatgttgatcttcagattcttatggaagctgtaagcattctcatgctcttcatttcacttgattggattttctttcaactttacgaagactaaatatatatatttataagtcaagcgtctaatattattataattgttccctttttgatcttctgcttcacttttataggcggatgttgatggagatggaagcttaaattatggggagtttgttgctgtatctgttcatctcagaaaaatggcaaatgatgagcacctgcacaaagcattttcagttttcgacagagatcagagtggttacatagaaatcgaggagctgcgcagtgccttgagtgatgaggatggtggcaacagtgaggaagtcatcaatgccattatgcatgatgttgacactgacaaggttagaattttttttgtgtccattcatgtatatctactggatttcatactagtgcatatacttctcttataaatgtctctttaattgcttgtggaaccataaataccccccttatcttgttccgcagttccaactacacacgaaactatgttgaagacgtattacccccttgtacttgtaaaatgtgtatcttccgtcatcctgagaggcatatatgatgtaaccaaatgtgaacatttaagtatatgcatgtgctgcctcatgtcatttacccctttttcccttttcacttctcttccatctccgcaacatgttaatgtcctctagcaaatctgaaaaaagatggagtgagcttctcaacggaaaaaatcggattcaccctagttttagttttctggcaacataaacagctcaagtcgatacaaaaaaacaaatgttcctatcaaaaaactcaaattagtagaaaggaaaagaagggtcataggtaagggaagaacaaaaaggaatagaaagacccttcggggtggcccagttatttgggcttggggcttccatgttggaggtctcaagttcaaaaccccttgccaatgaaagcaacgggttttccttctacgttgactgtcgagctcgtcgcaccgggcttacctagtgcggtttacctctcctttgcgtgctataggaataggggttttaccctgtgtgcactcaaagggtagcgactgcggatttcccaaaagaaaaaggaagagaaaggtaaagaaaacattttaaaaaagagtaggatggttataatagaagaaatgctataatattttttcacctcaggcgctttaagagagtaaatactctacgttacatggcgtcccaatgttgtcgtagttacattttggacaagaacagggagtaataggcctcccgcaaagttaaaatgtagtagggaatgggggaataattgaggaaggtatttatatattttctcctttctaaatcatattttcttttccattcactgctcttctgttcaaccttatcattcatttggactaaatgttgaattgattttgagcttttagtttgttaccacagcttcaaagttcatcagttacattgtctataaccatgcaggatggccgcattagttacgaggaatttgctgcaatgatgaaggctggcacagattggagaaaagcatcgagacagtattctcgtgaaagattcaacagtctcagcttaaaattgatgagagatggctcgatacaagtcggaaaggaagaaggtagatga

SEQ ID NO: 26 - DNA, 4913 bp, Solanum lycopersicum
  source 1..4913: mol_type = genomic DNA
atggggaattgctgtgggacacctggtaattcttctgagaataagaagaagaagaacaaaccaaacccttttgctcttgattatggtgcaactcaagcatctggaggtgatggaaacaagcttgttgtgttgaaagatccaacaggacacaatattcaagaaaaatatgatcttggttgtgagctaggaagaggagaatttggggttacatatttatgtactgatgttgatacaggggacaaatatgcttgcaaatcgatatcaaagaagaaacttaggactgctgtagatatagatgatgttaggagagaagttgagatcatgaagcatttgcctaaacatcctaatattgtgaccttgaaggacacttatgaggatgataatgcagtgcatattgtgatggaactttgtgaggggggtgagttgtttgataggattgttgccaggggacattatacagagagagcagctgcggttattatgaagactatagtagaagttgttcaggtacagttttactaattaatgcttgtctttgcttttcatctataattgttacttgtttgtttatttcatgtaatttaggggttgctaatttaggattatgttaatgaagtttgaattgacaatgccaactgaaagtgtcaatttagactagaaaggaatgttgagattgaagtttcatgtttgtaagcagaatgaatgttcttgtcgaagaatctcttttaagaatatctttcccacttcttcagtaaattttcctactttcttatgtcgataactgccactccttttctgagtttgcctgcactctcttggtagataggacactccctttcttagctcaggatctactttgcttgtgtaaatgagtgcttaatgtttttatttgattcattttacacgttgagatcctatagcatttaattagactagattttatcttccaatatcactaaacctagatgtcaaatatagtaaaaagttatgttgctcgaactcttcaaagatatcgacatgtgtgtgtcagatcctccaaaagtagtgcatttttggaggatccgacgggggtggggcaacaattttggagagttcgagcaacttaggtaaaaagtgtattcatgctctaaatgttgttaggttttctatctttcttatcttgtcttgtgaattttgctttcttggcaactgtttcattgtcctatatttttctcatgcaaatacctttaaaattatatactttcgtgccaaccatttaaatgaaacttaaggaagctaatcacacaggatttcaccatccaaatgtcgaaaatgaatcgcaatttgtgatagttttagacagagagcttatttttatagatgcaattagaataatagaaatgtaaaataactatcagtaaccagtaagttgccggtctttatggtctattttcagagggggagatctattgtagcttgctttcagcatcagttagtatagcataggactgttgctaacagggttcaattttaaactgtatttggtgaacataatgacatgagagctcaacttacacaactacagattagagagagacattcattttatggaatggatttaagaagttcatgtttctacatttagttgttataagaacagggtggtaactggtaaccgacgcaaacatgatggctaattatcccaagtttatacaatttaatctatgtggttgctcatacatctttggtcaatgttcactttacagttgcattatgtttcctcaagaaatggctgttcttctttcaattttcaacttacggagtttcaattgacattgcagatgtgtcatatgcatggagtaatgcatcgtgatctcaaacctgagaactttctgtttggtaacaagaaagaaactgctcctttgaaggctattgactttggattatcagtgttctttaaacccggtaatgcaataagtaatgatagtgtgttgtaactttttttcatgctaaaaaagattaatgttggaatcatcttttaatatgtttaacaggggaacgctttaatgagattgtgggaagtccttattacatggctccagaggtcctaaaacgcaattatggcccggaggttgatgtctggagtgctggagttatcctttatattcttctttgtggtgttccacctttctgggcaggtccgtttcttttatttgccttctttaggtaacaagtaatacctcggttcaccgacaaataacaaagtaaatcaaccttggtgcatactattcatttcttagaacttggtaatttattaatgagtgtcaaaatgaaatggaatttgaaacatattgatgcgttgttaacatcgtcgatgactaggtgagggtggctgcaagagtgaatcccacctcttcctggaccaattcaaaatcaaagttcctttttttccttttggcctgtgatagtcagtacattgtgcttccattaatttactcacagctttctcagtaattgcctaaaattctactgaatatgtgcagagactgaacaaggagtagcccaagcaattattcggtctgtggttgatttcaagagagatccatggcctaaggtttctgataatgcaaaggatcttgtaaagaagatgcttgacccggatccaactcgacgactcacagctcagcaggttcttggtaatgtttgttaatccttgagatgctatactttcatttgcttgctgtttgttctctcttagtttcataagttcaattttgtgacttttttggggctttcgtgcatatacatgaatgcagagcacacctggttacaaaatataaagaaagcaccaaatgtctcattgggtgagactgtgaaagcaaggcttaaacaattttcagtaatgaacaagctcaagaaaagagctctaacggtaaaatattcccttttcatttgcagttacatatcattagcgttctgcaccttctcagaaggatatcttcatatgcctaattcttaaagcccaaaataaggacaaaagattttctgccttctcacaaaagtttcgggtgttatattctttcttcattgcttgcacagattatggccgagtttttatcagcggaagaagtggctggaatgaaggacgcatttgatatgatggatacaggaaagaaaggcaagattaaccttggagaacttaaaaatggtctgcaaaagcttggccatcagatccctgatgttgatcttcagattcttatggaagctgtaagcattctcatgctcttcatttcacttgattggattttctttcaactttacgaagactaaatatatatatttataagtcaagcgtctaatattattataattgttcccttttttatcttctgcttcacttttataggcggatgttgatggagatggaagcttaaattatggggagtttgttgctgtatctgttcatctcagaaaaatggcaaatgatgagcacctgcacaaagcattttcagtttttgacagagatcagagtggttacatagaaatcgaggagctgcgcagtgccttgagtgatgaggatggtggcaacagtgaggaagtcatcaatgccattatgcatgatgttgacactgacaaggttagaattttttttgtgtccattcatgtatatctactggatttcatactagtgcatatacttctcttataaatgtctctttaattgcttgtggaaccataaataccccccttatcttgttccgcagctccaactacacacgaaactatgttgaagacgtattacccccttgtacttgtaaaatgtgtatcttccgtcatcctgagaggcatatatgatgtaaccaaatgtgaacatttaagtatatgcatgtgctgcctcatgtcatttacccctttttcccttttcacttctcttccatctccgcaacatgttaatgtcctctagcaaatctgaaaaaagatggagtgagcttctcaacggaaaaaatcggattcaccctagttttagttttctggcaacataaacagctcaagtcgatacaaaaaaacaaatgttcctatcaaaaaattcaaattagtagaaaggaaaagaagggtcataggtaagggaagaacaaaaaggaatagaaagacccttcggggtggcccagttatttgggcttggggcttggggcttgggacttccatgttggaggtctcaagttcaaaaccccttgccaatgaaagcaacgggttttccttctacgttgactgtcgagctcgtcgcaccgggcttacctagtgcggtttacctctcctttgcgtgctataggaataggggttttaccctgtgtacactcaaagggtagcgactgcggatttcccaaaagaaaaaggaagagaaaggtaaagaaaacattttaaaaaagagtaggatggttataatagaagaaatgctacaatattttttcacctcaggcgctttaagagagtaaatactctacgttacatggcgtcccaatgttgtcgtagttacattttggacaagaacagggagtaataggcctcccgcaaagttaaaatgtagtggggaatgggggaataattgaggaaggtatttatatattttctccttctaaatcatattttcttttccattcactgctcttctgttcaaccttatcattcatttggactaaatgttgaattgattttgagcttttagtttgttaccacagcttcaaagttcatcagttacattgtctataaccatgcaggatggccgcattagttacgaggaatttgctgcaatgatgaaggctggcacagattggagaaaagcatcgagacagtattctcgtgaaagattcaacagtctcagcttaaaattgatgagagatggctcgatacaagtcggaaaggaagaaggtagatga

SEQ ID NO: 27 - DNA, 4914 bp, Solanum lycopersicum
  source 1..4914: mol_type = genomic DNA
atggggaattgctgtgggacacctggtaattcttctgagaataagaagaagaagaacaaaccaaacccttttgctcttgattatggtgcaactcaagcatctggaggtgatggaaacaagcttgttgtgttgaaagatccaacaggacacaatattcaagaaaaatatgatcttggttgtgagctaggaagaggagaatttggggttacatatttatgtactgatgttgatacaggggacaaatatgcttgcaaatcgatatcaaagaagaaacttaggactgctgtagatatagatgatgttaggagagaagttgagatcatgaagcatttgcctaaacatcctaatattgtgaccttgaaggacacttatgaggatgataatgcagtgcatattgtgatggaactttgtgaggggggtgagttgtttgataggattgttgccaggggacattatacagagagagcagctgcggttattatgaagactatagtagaagttgttcaggtacagttttactaattaatgcttgtctttgcttttcatctataattgttacttgtttgtttatttcatgtaatttaggggttgctaatttaggattatgttaatgaagtttgaattgacaatgccaactgaaagtgtcaatttagactagaaaggaatgttgagattgaagtttcatgtttgtaagcagaatgaatgttcttgtcgaagaatctcttttaagaatatctttcccacttcttcagtaaattttcctactttcttatgtcgataactgccactccttttctgagtttgcctgcactctcttggtagataggacactccctttcttagctcaggatctactttgcttgtgtaaatgagtgcttaatgtttttatttgattcattttacacgttgagatcctatagcatttaattagactagattttatcttccaatatcactaaacctagatgtcaaatatagtaaaaagttatgttgctcgaactcttcaaagatatcgacatgtgtgtgtcagatcctccaaaagtagtgcatttttggaggatccgacgggggtggggcaacaattttggagagttcgagcaacttaggtaaaaagtgtattcatgctctaaatgttgttaggttttctatctttcttatcttgtcttgtgaattttgctttcttggcaactgtttcattgtcctatatttttctcatgcaaatacctttaaaattatatactttcgtgccaaccatttaaatgaaacttaaggaagctaatcacacaggatttcaccatccaaatgtcgaaaatgaatcgcaatttgtgatagttttagacagagagcttatttttatagatgcaattagaataatagaaatgtaaaataactatcagtaaccagtaagatgccggtctttatggtctattttcagagggggagatctattgtagcttgctttcagcatcagttagtatagcataggactgttgctaacagggttcaattttaaactgtatttggtgaacataatgacatgagagctcaacttacataactacagattagagagagacattcattttatggaatggatttaagaagttcatgtttctacatttagttgttataagaacagggtggtaactggtaaccgacgcaaacatgatggctaattatcccaagtttatacaatttaatctatgtggttgctcatacatctttggtcaatgttcactttacagttgcattatgtttcctcaagaaatggctgttcttctttcaattttcaacttacggagtttcaattgacattgcagatgtgtcatatgcatggagtaatgcatcgtgatctcaaacctgagaactttctgtttggtaacaagaaagaaactgctcctttgaaggctattgactttggattatcagtgttctttaaacccggtaatgcaataagtaatgatagtgtgttgtaactttttttcatgctaaaaaagattaatgttggaatcatcttttaatatgtttaacaggggaacgctttaatgagattgtgggaagtccttattacatggctccagaggtcctaaaacgcaattatggcccggaggttgatgtctggagtgctggagttatcctttatattcttctttgtggtgttccacctttctgggcaggtccgtttcttttatttgccttctttaggtaacaagtaatacctcggttcaccgacaaataacaaagtaaatcaaccttggtgcatactattcatttcttagaacttggtaatttattaatgagtgtcaaaatgaaatggaatttgaaacatattgatgcgttgttaacatcgtcgatgactaggtgagggtggctgcaagagtgaatcccacctcttcctggaccaattcaaaatcaaagttcctttttttccttttggcctgtgatagtcagtactttgtgcttccattaatttactcacagctttctcagtaattgcctaaaattctactgaatatgtgcagagactgaacaaggagtagcccaagcaattattcggtctgtggttgatttcaagagagatccatggcctaaggtttctgataatgcaaaggatcttgtaaagaagatgcttgacccggatccaactcgacgactcacagctcagcaggttcttggtaatgtttgttaatccttgagatgctatactttcatttgcttgctgtttgttctctcttagtttcataagttcaattttgtgacttttttggggctttcgtgcatatacatgaatgcagagcacacctggttacaaaatataaagaaagcaccaaatgtctcattgggtgagactgtgaaagcaaggcttaaacaattttcagtaatgaacaagctcaagaaaagagctctaacggtaaaatattcccttttcatttgcagttacatatcattagcgttctgcaccttctcagaaggatatcttcatatgcctaattcttaaagcccaaaataaggacaaaagattttctgccttctcacaaaagtttcgggtgttatattctttcttcattgcttgcacagattatggccgagtttttatcagcggaagaagtggctggaatgaaggacgcatttgatatgatggatacaggaaagaaaggcaagattaaccttggagaacttaaaaatggtctgcaaaagcttggccatcagatccctgatgttgatcttcagattcttatggaagctgtaagcattctcatgctcttcatttcacttgattggattttctttcaactttacgaagactaaatatatatatttataagtcaagcgtctaatattattataattgttcccttttttatcttctgcttcacttttataggcggatgttgatggagatggaagcttaaattatggggagtttgttgctgtatctgttcatctcagaaaaatggcaaatgatgagcacctgcacaaagcattttcagtttttgacagagatcagagtggttacatagaaatcgaggagctgcgcagtgccttgagtgatgaggatggtggcaacagtgaggaagtcatcaatgccattatgcatgatgttgacactgacaaggttagaattttttttgtgtccattcatgtatatctactggatttcatactagtgcatatacttcttttataaatgtctctttaattgcttgtggaaccataaataccccccttatcttgttccgcagctccaactacacacgaaactatgttgaagacgtattacccccttgtacttgtaaaatgtgtatcttccgtcatcctgagaggcatatatgatgtaaccaaatgtgaacatttaagtatatgcatgtgctgcctcatgtcatttacccctttttcccttttcacttctcttccatctccacaacatgttaatgtcctctagcaaatctgaaaaaagatggagtgagcttctcaacggaaaaaatcggattcaccctagttttagttttctggcaacataaacagctcaagtcgatacaaaaaaacaaatgttcctatcaaaaaactcaaattagtagaaaggaaaagaagggtcataggtaagggaagaacaaaaaggaatagaaagacccttcggggtggcccagttatttgggcttggggcttggggcttgggacttccatgttggaggtctcaagttcaaaaccccttgccaatgaaagcaacgggttttccttctacgttgactgtcgagctcgtcgcaccgggcttacctagtgcggtttacctctcctttgcgtgctataggaataggggttttaccctgtgtgcactcaaagggtagcgactgcggatttcccaaaagaaaaaggaagagaaaggtaaagaaaacattttaaaaaagagtaggatggttataatagaagaaatgctacaatattttttcacctcaggcgctttaagagagtaaatactctacgttacatggcgtcccaatgttgtcgtagttacattttggacaagaacagggagtaataggcctcccgcaaagttaaaatgtagtggggaatgggggaataattgaggaaggtatttatatattttctcctttctaaatcatattttcttttccattcactgctcttctgttcaaccttatcattcatttggactaaatgttgaattgattttgagcttttagtttgttaccacagcttcaaagttcatcagttacattgtctataaccatgcaggatggccgcattagttacgaggaatttgctgcaatgatgaaggctggcacagattggagaaaagcatcgagacagtattctcgtgaaagattcaacagtctcagcttaaaattgatgagagatggctcgatacaagtcggaaaggaagaaggtagatga

SEQ ID NO: 28 - DNA, 4897 bp, Solanum lycopersicum
  source 1..4897: mol_type = genomic DNA
atggggaattgctgtgggacacctggtaattcttctgagaataagaagaagaacaaaccaaacccgtttgctcttgattatggtgcaactcaagcatctggaggtgatggaaacaagcttgttgtgttgaaagatccaacaggacacaatattcaagaaaaatatgatcttggttgtgagctaggaagaggagaatttggggttacatatttatgtactgatgttgatacaggggacaaatatgcttgcaaatcgatatcgaagaagaaacttaggactgctgtagatatagatgatgttaggagagaagttgagatcatgaagcatttgcctaaacatcctaatattgtgaccttgaaggacacttatgaggatgataatgcagtgcatattgtgatggaactttgtgaggggggtgagttgtttgataggattgttgccaggggacattatacagagagagcagctgcggttattatgaagactatagtagaagttgttcaggtacagttttactaattgatgcttgtctttgcttttcatctataattgttacttgtttgtttatttcatgtaatttaggggttgctaatttaggattatgttaatgaagtttgaattgacaatgccaactgaaagtatcaatttagactagaaaggaatgttgagattgaagtttcatgtttgtaagcagaatgaatgttcttgtcgaagaatctcttttaagaatatctttcccacttcttcagtaaattttcctactttcttatgtcgataactgccactccttttctgagtttgcctgcactctcttggtagataggacactccctttcttagctcaggatttactttgcttgtgtaaatgagtgcttaatgtttttatttgattcattttacacgttgagatcctatagcatttaattagactagattttatcttccaatatcactaaacctagatgtcaaatatagtaaaaagttatgttgctcgaactcttcaaagatatcgacatgtgtgtgtcagatcctccaaaagtagtgcatttttggaggatccgacgggggtggggcaacaattttggagagttcgagcaacttaggtaaaaagtgtattcatgctctaaatgttgttaggttttctatctttcttatcttgtcttgtgaattttgctttcttggcaactgtttcattgtcctatatttttctcatgcaaatacctttaaaattatatactttcgtgccaaccatttaaatgaaacttaaggaagctaatcacacaggatttcaccatccaaatgtcgaaaatgaatcgcaatttgtgatagttttagacagagagcttatttttatagatgcaattagaataatagaaatgtaaaataactatcagtaaccagtaagatgccggtctttatggtctattttcagagggggagatctattgtagcttgctttcagcattagttagtatagcataggactgttgctaacagggttcaattttaaactgtatttggtgaacataatgacatgagagctcaacttacataactacagattagagagagacattcattttatggaatggatttaagaagttcatgtttctacatttagttgttataagaacagggtggtaactggtaaccgacgcaaacatgatggctaattatcccaagtttatacaatttaatctatgtggttgctcatacatctttggtcaatgttcactttacagttgcattatgtttcctcaagaaatggctgttcttctttcaattttcaacttacggagtttcaattgacattgcagatgtgtcatatgcatggagtaatgcatcgtgatctcaaacctgagaactttctgtttggtaacaagaaagaaattgctcctttgaaggctattgactttggattatcagtgttctttaaacccggtaatgcaataagtaatgatagtgtgttgtaactttttttcatgctaaaaaagattaatgttggaatcatcttttaatatgtttaacaggggaacggtttaatgagattgtgggaagtccttattacatggctccagaggtcctaaaacgcaattatggcccggaggttgatgtctggagtgctggagttatcctttatattcttctttgtggtgttccacctttctgggcaggtccgtttcttttatttgccttctttaggtaacaagtaatacctcggttcaccgacaaataacaaattaaatcaaccttggtgcatactattcatttcttagaacttggtaatttattaatgagtgtcaaaatgaaatggaatttgaaacatattgatgcgttgttaacatcgtcgatgactaggtgagggtggctgcaagagtgaatcccacctcttcctggaccaattcaaaatcaaagttcctttttttccttttggcctgtgatagtcagtactttgtgcttccattaatttactcacagctttctcagtaattgcctaaaattctactgaatatgtgcagagactgaacaaggagtagcccaagcaattattcggtctgtggttgatttcaagagagatccatggcctaaggtttctgataatgcaaaggatcttgtaaagaagatgcttgacccggatccaactcgacgactcacagctcagcaggttcttggtaatgtttgttaatccttgagatgctatactttcatttgcttgctgtttgttctctcttagtttcataagttcaattttgtgactcttttggggctttcgtgcatatacatgaatgcagagcacacctggttacaaaatataaagaaagcaccaaatgtctcattgggtgagactgtgaaagcaaggcttaaacaattttcagtaatgaacaagctcaagaaaagagctctaacggtaaaatattcccttttcatttgcagttacatatcattagcgttctgcaccttctcagaaggatatcttcatatgcctaattcttaaagcccaaaataaggacaaaagattttctgccttctcacaaaagtttcgggtgttatattctttcttcattgcttgcacagattatggccgagtttttatcagcggaagaagtggctggaatgaaggacgcatttgatatgatggatacaggaaagaaaggcaagattaaccttggagaacttaaaaatggtctgcaaaagcttggccatcagatccctgatgttgatcttcagattcttatggaagctgtaagcattctcatgctcttcatttcacttgattggattctctttcaactttacgaagactaaatatatatatttataagtcaagcgtctaatattattataattgttccctttttgatcttctgcttcacttttataggcggatgttgatggagatggaagcttaaattatggggagtttgttgctgtatctgttcatctcagaaaaatggcaaatgatgagcacctgcacaaagcattttcagttttcgacagagatcagagtggttacatagaaatcgaggagctgcgcagtgccttgagtgatgaggatggtggcaacagtgaggaagtcatcaatgccattatgcatgatgttgacactgacaaggttagaattttttttgtgtccattcatgtatatctactggatttcatactagtgcatatacttctcttataaatgtctctttaattgcttgtggaaccataaataccccccttatcttgttccgcagttccaactacacacgaaactatgttgaagacgtattacccccttgtacttgtaaaatgtgtatcttccgtcatcctgagaggcatatatgatgtaaccaaatgtgaacatttaagtatatgcatgtgctgcctcatgtcatttacccctttttcccttttcacttctcttccatctccgcaacatgttaatgtcctctagcaaatctgaaaaaagatggagtgagcttctcaacggaaaaaatcggattcaccctagttttagttttctggcaacataaacagctcaagtcgatacaaaaaaacaaatgttcctatcaaaaaactcaaattagtagaaaggaaaagaagggtcataggtaagggaagaacaaaaaggaatagaaagacccttcggggtggcccagttatttgggcttggggcttccatgttggaggtctcaagttcaaaaccccttgccaatgaaagcaacgggttttccttctacgttgactgtcgagctcgtcgcaccgggcttacctagtgcggtttacctctcctttgcgtgctataggaataggggttttaccctgtgtgcactcaaagggtagcgactgcggatttcccaaaagaaaaaggaagagaaaggtaaagaaaacattttaaaaaagagtaggatggttataatagaagaaatgctataatattttttcacctcaggcgctttaagagagtaaatactctacgttacatggcgtcccaatgttgtcgtagttacattttggacaagaacagggagtaataggcctcccgcaaagttaaaatgtagtagggaatgggggaataattgaggaaggtatttatatattttctcctttctaaatcatattttcttttccattcactgctcttctgttcaaccttatcattcatttggactaaatgttgaattgattttgagcttttagtttgttaccacagcttcaaagttcatcagttacattgtctataaccatgcaggatggccgcattagttacgaggaatttgctgcaatgatgaaggctggcacagattggagaaaagcatcgagacagtattctcgtgaaagattcaacagtctcagcttaaaattgatgagagatggctcgatacaagtcggaaaggaagaaggtagatga

SEQ ID NO: 29 - DNA, 4897 bp, Solanum lycopersicum
  source 1..4897: mol_type = genomic DNA
atggggaattgctgtgggacacctggtaattcttctgagaataagaagaagaacaaaccaaacccgtttgctcttgattatggtgcaactcaagcatctggaggtgatggaaacaagcttgttgtgttgaaagatccaacaggacacaatattcaagaaaaatatgatcttggttgtgagctaggaagaggagaatttggggttacatatttatgtactgatgttgatacaggggacaaatatgcttgcaaatcgatatcgaagaagaaacttaggactgctgtagatatagatgatgttaggagagaagttgagatcatgaagcatttgcctaaacatcctaatattgtgaccttgaaggacacttatgaggatgataatgcagtgcatattgtgatggaactttgtgaggggggtgagttgtttgataggattgttgccaggggacattatacagagagagcagctgcggttattatgaagactatagtagaagttgttcaggtacagttttactaattgatgcttgtctttgcttttcatctataattgttacttgtttgtttatttcatgtaatttaggggttgctaatttaggattatgttaatgaagtttgaattgacaatgccaactgaaagtatcaatttagactagaaaggaatgttgagattgaagtttcatgtttgtaagcagaatgaatgttcttgtcgaagaatctcttttaagaatatctttcccacttcttcagtaaattttcctactttcttatgtcgataactgccactccttttctgagtttgcctgcactctcttggtagataggacactccctttcttagctcaggatttactttgcttgtgtaaatgagtgcttaatgtttttatttgattcattttacacgttgagatcctatagcatttaattagactagattttatcttccaatatcactaaacctagatgtcaaatatagtaaaaagttatgttgctcgaactcttcaaagatatcgacatgtgtgtgtcagatcctccaaaagtagtgcatttttggaggatccgacgggggtggggcaacaattttggagagttcgagcaacttaggtaaaaagtgtattcatgctctaaatgttgttaggttttctatctttcttatcttgtcttgtgaattttgctttcttggcaactgtttcattgtcctatatttttctcatgcaaatacctttaaaattatatactttcgtgccaaccatttaaatgaaacttaaggaagctaatcacacaggatttcaccatccaaatgtcgaaaatgaatcgcaatttgtgatagttttagacagagagcttatttttatagatgcaattagaataatagaaatgtaaaataactatcagtaaccagtaagatgccggtctttatggtctattttcagagggggagatctattgtagcttgctttcagcatcagttagtatagcataggactgttgctaacagggttcaattttaaactgtatttggtgaacataatgacatgagagctcaacttacataactacagattagagagagacattcattttatggaatggatttaagaagttcatgtttctacatttagttgttataagaacagggtggtaactggtaaccgacgcaaacatgatggctaattatcccaagtttatacaatttaatctatgtggttgctcatacatctttggtcaatgttcactttacagttgcattatgtttcctcaagaaatggctgttcttctttcaattttcaacttacggagtttcaattgacattgcagatgtgtcatatgcatggagtaatgcatcgtgatctcaaacctgagaactttctgtttggtaacaagaaagaaattgctcctttgaaggctattgactttggattatcagtgttctttaaacccggtaatgcaataagtaatgatagtgtgttgtaactttttttcatgctaaaaaagattaatgttggaatcatcttttaatatgtttaacaggggaacggtttaatgagattgtgggaagtccttattacatggctccagaggtcctaaaacgcaattatggcccggaggttgatgtctggagtgctggagttatcctttatattcttctttgtggtgttccacctttctgggcaggtccgtttcttttatttgccttctttaggtaacaagtaatacctcggttcaccgacaaataacaaattaaatcaaccttggtgcatactattcatttcttagaacttggtaatttattaatgagtgtcaaaatgaaatggaatttgaaacatattgatgcgttgttaacatcgtcgatgactaggtgagggtggctgcaagagtgaatcccacctcttcctggaccaattcaaaatcaaagttcctttttttccttttggcctgtgatagtcagtactttgtgcttccattaatttactcacagctttctcagtaattgcctaaaattctactgaatatgtgcagagactgaacaaggagtagcccaagcaattattcggtctgtggttgatttcaagagagatccatggcctaaggtttctgataatgcaaaggatcttgtaaagaagatgcttgacccagatccaactcgacgactcacagctcagcaggttcttggtaatgtttgttaatccttgagatgctatactttcatttgcttgctgtttgttctctcttagtttcataagttcaattttgtgacttttttggggctttcgtgcatatacatgaatgcagagcacacctggttacaaaatataaagaaagcaccaaatgtctcattgggtgagactgtgaaagcaaggcttaaacaattttcagtaatgaacaagctcaagaaaagagctctaacggtaaaatattcccttttcatttgcagttacatatcattagcgttctgcaccttctcagaaggatatcttcatatgcctaattcttaaagcccaaaataaggacaaaagattttctgccttctcacaaaagtttcgggtgttatattctttcttcattgcttgcacagattatggccgagtttttatcagcggaagaagtggctggaatgaaggacgcatttgatatgatggatacaggaaagaaaggcaagattaaccttggagaacttaaaaatggtctgcaaaagcttggccatcagatccctgatgttgatcttcagattcttatggaagctgtaagcattctcatgctcttcatttcacttgattggattttctttcaactttacgaagactaaatatatatatttataagtcaagcgtctaatattattataattgttccctttttgatcttctgcttcacttttataggcggatgttgatggagatggaagcttaaattatggggagtttgttgctgtatctgttcatctcagaaaaatggcaaatgatgagcacctgcacaaagcattttcagttttcgacagagatcagagtggttacatagaaatcgaggagctgcgcagtgccttgagtgatgaggatggtggcaacagtgaggaagtcatcaatgccattatgcatgatgttgacactgacaaggttagaattttttttgtgtccattcatgtatatctactggatttcatactagtgcatatacttctcttataaatgtctctttaattgcttgtggaaccataaataccccccttatcttgttccgcagttccaactacacacgaaactatgttgaagacgtattacccccttgtacttgtaaaatgtgtatcttccgtcatcctgagaggcatatatgatgtaaccaaatgtgaacatttaagtatatgcatgtgctgcctcatgtcatttacccctttttcccttttcacttctcttccatctccgcaacatgttaatgtcctctagcaaatctgaaaaaagatggagtgagcttctcaacggaaaaaatcggattcaccctagttttagttttctggcaacataaacagctcaagtcgatacaaaaaaacaaatgttcctatcaaaaaactcaaattagtagaaaggaaaagaagggtcataggtaagggaagaacaaaaaggaatagaaagacccttcggggtggcccagttatttgggcttggggcttccatgttggaggtctcaagttcaaaaccccttgccaatgaaagcaacgggttttccttctacgttgactgtcgagctcgtcgcaccgggcttacctagtgcggtttacctctcctttgcgtgctataggaataggggttttaccctgtgtgcactcaaagggtagcgactgcggatttcccaaaagaaaaaggaagagaaaggtaaagaaaacattttaaaaaagagtaggatggttataatagaagaaatgctataatattttttcacctcaggcgctttaagagagtaaatactctacgttacatggcgtcccaatgttgtcgtagttacattttggacaagaacagggagtaataggcctcccgcaaagttaaaatgtagtagggaatgggggaataattgaggaaggtatttatatattttctcctttctaaatcatattttcttttccattcactgctcttctgttcaaccttatcattcatttggactaaatgttgaattgattttgagcttttagtttgttaccacagcttcaaagttcatcagttacattgtctataaccatgcaggatggccgcattagttacgaggaatttgctgcaatgatgaaggctggcacagattggagaaaagcatcgagacagtattctcgtgaaagattcaacagtctcagcttaaaattgatgagagatggctcgatacaagtcggaaaggaagaaggtagatga

SEQ ID NO: 30 - DNA, 4897 bp, Solanum lycopersicum
  source 1..4897: mol_type = genomic DNA
atggggaattgctgtgggacacctggtaattcttctgagaataagaagaagaacaaaccaaacccgtttgctcttgattatggtgcaactcaagcatctggaggtgatggaaacaagcttgttgtgttgaaagatccaacaggacacaatattcaagaaaaatatgatcttggttgtgagctaggaagaggagaatttggggttacatatttatgtactgatgttgatacaggggacaaatatgcttgcaaatcgatatcgaagaagaaacttaggactgctgtagatatagatgatgttaggagagaagttgagatcatgaagcatttgcctaaacatcctaatattgtgaccttgaaggacacttatgaggatgataatgcagtgcatattgtgatggaactttgtgaggggggtgagttgtttgataggattgttgccaggggacattatacagagagagcagctgcggttattatgaagactatagtagaagttgttcaggtacagttttactaattgatgcttgtctttgcttttcatctataattgttacttgtttgtttatttcatgtaatttaggggttgctaatttaggattatgttaatgaagtttgaattgacaatgccaactgaaagtatcaatttagactagaaaggaatgttgagattgaagtttcatgtttgtaagcagaatgaatgttcttgtcgaagaatctcttttaagaatatctttcccacttcttcagtaaattttcctactttcttatgtcgataactgccactccttttctgagtttgcctgcactctcttggtagataggacactccctttcttagctcaggatttactttgcttgtgtaaatgagtgcttaatgtttttatttgattcattttacacgttgagatcctatagcatttaattagactagattttatcttccaatatcactaaacctagatgtcaaatatagtaaaaagttatgttgctcgaactcttcaaagatatcgacatgtgtgtgtcagatcctccaaaagtagtgcatttttggaggatccgacgggggtggggcaacaattttggagagttcgagcaacttaggtaaaaagtgtattcatgctctaaatgttgttaggttttctatctttcttatcttgtcttgtgaattttgctttcttggcaactgtttcattgtcctatatttttctcatgcaaatacctttaaaattatatactttcgtgccaaccatttaaatgaaacttaaggaagctaatcacacaggatttcaccatccaaatgtcgaaaatgaatcgcaatttgtgatagttttagacagagagcttatttttatagatgcaattagaataatagaaatgtaaaataactatcagtaaccagtaagatgccggtctttatggtctattttcagagggggagatctattgtagcttgctttcagcatcagttagtatagcataggactgttgctaacagggttcaattttaaactgtatttggtgaacataatgacatgagagctcaacttacataactacagattagagagagacattcattttatggaatggatttaagaagttcatgtttctacatttagttgttataagaacagggtggtaactggtaaccgacgcaaacatgatggctaattatcccaagtttatacaatttaatctatgtggttgctcatacatctttggtcaatgttcactttacagttgcattatgtttcctcaagaaatggctgttcttctttcaattttcaacttacggagtttcaattgacattgcagatgtgtcatatgcatggagtaatgcatcgtgatctcaaacctgagaactttctgtttggtaacaagaaagaaattgctcctttgaaggctattgactttggattatcagtgttctttaaacccggtaatgcaataagtaatgatagtgtgttgtaactttttttcatgctaaaaaagattaatgttggaatcatcttttaatatgtttaacaggggaacggtttaatgagattgtgggaagtccttattacatggctccagaggtcctaaaacgcaattatggcccggaggttgatgtctggagtgctggagttatcctttatattcttctttgtggtgttccacctttctgggcaggtccgtttcttttatttgccttctttaggtaacaagtaatacctcggttcaccgacaaataacaaattaaatcaaccttggtgcatactattcatttcttagaacttggtaatttattaatgagtgtcaaaatgaaatggaatttgaaacatattgatgcgttgttaacatcgtcgatgactaggtgagggtggctgcaagagtgaatcccacctcttcctggaccaattcaaaatcaaagttcctttttttccttttggcctgtgatagtcagtactttgtgcttccattaatttactcacagctttctcagtaattgcctaaaattctactgaatatgtgcagagactgaacaaggagtagcccaagcaattattcggtctgtggttgatttcaagagagatccatggcctaaggtttctgataatgcaaaggatcttgtaaagaagatgcttgacccggatccaactcgacgactcacagctcagcaggttcttggtaatgtttgttaatccttgagatgctatactttcatttgcttgctgtttgttctctcttagtttcataagttcaattttgtgacttttttggggctttcgtgcatatacatgaatgcagagcacacctggttacaaaatataaagaaagcaccaaatgtctcattgggtgagactgtgaaagcaaggcttaaacaattttcagtaatgaacaagctcaagaaaagagctctaacggtaaaatattcccttttcatttgcagttacatatcattagcgttctgcaccttctcagaaggatatcttcatatgcctaattcttaaagcccaaaataaggacaaaagattttctgccttctcacaaaagtttcgggtgttatattctttcttcattgcttgcacagattatggccgagtttttatcagcggaagaagtggctggaatgaaggacgcatttgatatgatggatacaggaaagaaaggcaagattaaccttggagaacttaaaaatggtctgcaaaagcttggccatcagatccctgatgttgatcttcagattcttatggaagctgtaagcattctcatgctcttcatttcacttgattggattttctttcaactttacgaagactaaatatatatatttataagtcaagcgtctaatattattataattgttccctttttgatcttctgcttcacttttataggcggatgttgatggagatggaagcttaaattatggggagtttgttgctgtatctgttcatctcagaaaaatggcaaatgatgagcacctgcacaaagcattttcagttttcgacagagatcagagtggttacatagaaatcgaggagctgcgcagtgccttgagtgatgaggatggtggcaacagtgaggaagtcatcaatgccattatgcatgatgttgacactgacaaggttagaattttttttgtgtccattcatgtatatctactggatttcatactagtgcatatacttctcttataaatgtctctttaattgcttgtggaaccataaataccccccttatcttgttccgcagttccaactacacacgaaactatgttgaagacgtattacccccttgtacttgtaaaatgtgtatcttccgtcatcctgagaggcatatatgatgtaaccaaatgtgaacatttaagtatatgcatgtgctgcctcatgtcatttacccctttttcccttttcacttctcttccatctccgcaacatgttaatgtcctctagcaaatctgaaaaaagatggagtgagcttctcaacggaaaaaatcggattcaccctagttttagttttctggcaacataaacagctcaagtcgatacaaaaaaacaaatgttcctatcaaaaaactcaaattagtagaaaggaaaagaagggtcataggtaagggaagaacaaaaaggaatagaaagacccttcggggtggcccagttatttgggcttggggcttccatgttggaggtctcaagttcaaaaccccttgccaatgaaagcaacgggttttccttctacgttgactgtcgagctcgtcgcaccgggcttacctagtgcggtttacctctcctttgcgtgctataggaataggggttttaccctgtgtgcactcaaagggtagcgactgcggatttcccaaaagaaaaaggaagagaaaggtaaagaaaacattttaaaaaagagtaggatggttataatagaagaaatgctataatattttttcacctcaggcgctttaagagagtaaatactctacgttacatggcgtcccaatgttgtcgtagttacattttggacaagaacagggagtaataggcctcccgcaaagttaaaatgtagtagggaatgggggaataattgaggaaggtatttatatattttctcctttctaaatcatattttcttttccattcactgctcttctgttcaaccttatcattcatttggactaaatgttgaattgattttgagcttttagtttgttaccacagcttcaaagttcatcagttacattgtctataaccatgcaggatggccgcattagttacgaggaatttgctgcaatgatgaaggctggcacagattggagaaaagcatcgagacagtattctcgtgaaagattcaacagtctcagcttaaaattgatgagagatggctcgatacaagtcggaaaggaagaaggtagatga

SEQ ID NO: 31 - DNA, 4914 bp, Solanum lycopersicum; identical to SEQ ID NO: 3
  source 1..4914: mol_type = genomic DNA

SEQ ID NO: 32 - DNA, 4914 bp, Solanum lycopersicum
  source 1..4914: mol_type = genomic DNA
atggggaattgctgtgggacacctggtaattcttctgagaataagaagaagaagaacaaaccaaacccttttgctcttgattatggtgcaactcaagcatctggaggtgatggaaacaagcttgttgtgttgaaagatccaacaggacacaatattcaagaaaaatatgatcttggttgtgagctaggaagaggagaatttggggttacatatttatgtactgatgttgatacaggggacaaatatgcttgcaaatcgatatcaaagaagaaacttaggactgctgtagatatagatgatgttaggagagaagttgagatcatgaagcatttgcctaaacatcctaatattgtgaccttgaaggacacttatgaggatgataatgcagtgcatattgtgatggaactttgtgaggggggtgagttgtttgataggattgttgccaggggacattatacagagagagcagctgcggttattatgaagactatagtagaagttgttcaggtacagttttactaattaatgcttgtctttgcttttcatctataattgttacttgtttgtttatttcatgtaatttaggggttgctaatttaggattatgttaatgaagtttgaattgacaatgccaactgaaagtgtcaatttagactagaaaggaatgttgagattgaagtttcatgtttgtaagcagaatgaatgttcttgtcgaagaatctcttttaagaatatctttcccacttcttcagtaaattttcctactttcttatgtcgataactgccactccttttctgagtttgcctgcactctcttggtagataggacactccctttcttagctcaggatctactttgcttgtgtaaatgagtgcttaatgtttttatttgattcattttacacgttgagatcctatagcatttaattagactagattttatcttccaatatcactaaacctagatgtcaaatatagtaaaaagttatgttgctcgaactcttcaaagatatcgacatgtgtgtgtcagatcctccaaaagtagtgcatttttggaggatccgacgggggtggggcaacaattttggagagttcgagcaacttaggtaaaaagtgtattcatgctctaaatgttgttaggttttctatctttcttatcttgtcttgtgaattttgctttcttggcaactgtttcattgtcctatatttttctcatgcaaatacctttaaaattatatactttcgtgccaaccatttaaatgaaacttaaggaagctaatcacacaggatttcaccatccaaatgtcgaaaatgaatcgcaatttgtgatagttttagacagagagcttatttttatagatgcaattagaataatagaaatgtaaaataactatcagtaaccagtaagatgccggtctttatggtctattttcagagggggagatctattgtagcttgctttcagcatcagttagtatagcataggactgttgctaacagggttcaattttaaactgtatttggtgaacataatgacatgagagctcaacttacataactacagattagagagagacattcattttatggaatggatttaagaagttcatgtttctacatttagttgttataagaacagggtggtaactggtaaccgacgcaaacatgatggctaattatcccaagtttatacaatttaatctatgtggttgctcatacatctttggtcaatgttcactttacagttgcattatgtttcctcaagaaatggctgttcttctttcaattttcaacttacggagtttcaattgacattgcagatgtgtcatatgcatggagtaatgcatcgtgatctcaaacctgagaactttctgtttggtaacaagaaagaaactgctcctttgaaggctattgactttggattatcagtgttctttaaacccggtaatgcaataagtaatgatagtgtgttgtaactttttttcatgctaaaaaagattaatgttggaatcatcttttaatatgtttaacaggggaacgctttaatgagattgtgggaagtccttattacatggctccagaggtcctaaaacgcaattatggcccggaggttgatgtctggagtgctggagttatcctttatattcttctttgtggtgttccacctttctgggcaggtccgtttcttttatttgccttctttaggtaacaagtaatacctcggttcaccgacaaataacaaagtaaatcaaccttggtgcatactattcatttcttagaacttggtaatttattaatgagtgtcaaaatgaaatggaatttgaaacatattgatgcgttgttaacatcgtcgatgactaggtgagggtggctgcaagagtgaatcccacctcttcctggaccaattcaaaatcaaagttcctttttttccttttggcctgtgatagtcagtactttgtgcttccattaatttactcacagctttctcagtaattgcctaaagttctactgaatatgtgcagagactgaacaaggagtagcccaagcaattattcggtctgtggttgatttcaagagagatccatggcctaaggtttctgataatgcaaaggatcttgtaaagaagatgcttgacccggatccaactcgacgactcacagctcagcaggttcttggtaatgtttgttaatccttgagatgctatactttcatttgcttgctgtttgttctctcttagtttcataagttcaattttgtgacttttttggggctttcgtgcatatacatgaatgcagagcacacctggttacaaaatataaagaaagcaccaaatgtctcattgggtgagactgtgaaagcaaggcttaaacaattttcagtaatgaacaagctcaagaaaagagctctaacggtaaaatattcccttttcatttgcagttacatatcattagcgttctgcaccttctcagaaggatatcttcatatgcctaattcttaaagcccaaaataaggacaaaagattttctgccttctcacaaaagtttcgggtgttatattctttcttcattgcttgcacagattatggccgagtttttatcagcggaagaagtggctggaatgaaggacgcatttgatatgatggatacaggaaagaaaggcaagattaaccttggagaacttaaaaatggtctgcaaaagcttggccatcagatccctgatgttgatcttcagattcttatggaagctgtaagcattctcatgctcttcatttcacttgattggattttctttcaactttacgaagactaaatatatatatttataagtcaagcgtctaatattattataattgttcccttttttatcttctgcttcacttttataggcggatgttgatggagatggaagcttaaattatggggagtttgttgctgtatctgttcatctcagaaaaatggcaaatgatgagcacctgcacaaagcattttcagtttttgacagagatcagagtggttacatagaaatcgaggagctgcgcagtgccttgagtgatgaggatggtggcaacagtgcggaagtcatcaatgccattatgcatgatgttgacactgacaaggttagaattttttttgtgtccattcatgtatatctactggatttcatactagtgcatatacttctcttataaatgtctctttaattgcttgtggaaccataaataccccccttatcttgttccgcagctccaactacacacgaaactatgttgaagacgtattacccccttgtacttgtaaaatgtgtatcttccgtcatcctgagaggcatatatgatgtaaccaaatgtgaacatttaagtatatgcatgtgctgcctcatgtcatttacccctttttcccttttcacttctcttccatctccgcaacatgttaatgtcctctagcaaatctgaaaaaagatggagtgagcttctcaacggaaaaaatcggattcaccctagttttagttttctggcaacataaacagctcaagtcgatacaaaaaaacaaatgttcctatcaaaaaactcaaattagtagaaaggaaaagaagggtcataagtaagggaagaacaaaaaggaatagaaagacccttcggggtggcccagttatttgggcttggggcttggggcttgggacttccatgttggaggtctcaagttcaaaaccccttgccaatgaaagcaacgggttttccttctacgttgactgtcgagctcgtcgcaccgggcttacctagtgcggtttacctctcctttgcgtgctataggaataggggttttaccctgtgtgcactcaaagggtagcgactgcggatttcccaaaagaaaaaggaagagaaaggtaaagaaaacattttaaaaaagagtaggatggttataatagaagaaatgctacaatattttttcacctcaggcgctttaagagagtaaatactctacgttacatggcgtcccaatgttgtcgtagttacattttggacaagaacagggagtaataggcctcccgcaaagttaaaatgtagtggggaatgggggaataattgaggaaggtatttatatattttctcctttctaaatcatattttcttttccattcactgctcttctgttcaaccttatcattcatttggactaaatgttgaattgattttgagcttttagtttgttaccacagcttcaaagttcatcagttacattgtctataaccatgcaggatggccgcattagttacgaggaatttgctgcaatgatgaaggctggcacagattggagaaaagcatcgagacagtattctcgtgaaagattcaacagtctcagcttaaaattgatgagagatggctcgatacaagtcggaaaggaagaaggtagatga

SEQ ID NO: 33 - DNA, 4914 bp, Solanum lycopersicum; identical to SEQ ID NO: 3
  source 1..4914: mol_type = genomic DNA

SEQ ID NO: 34 - DNA, 4897 bp, Solanum lycopersicum
  source 1..4897: mol_type = genomic DNA
atggggaattgctgtgggacacctggtaattcttctgagaataagaagaagaacaaaccaaacccgtttgctcttgattatggtgcaactcaagcatctggaggtgatggaaacaagcttgttgtgttgaaagatccaacaggacacaatattcaagaaaaatatgatcttggttgtgagctaggaagaggagaatttggggttacatatttatgtactgatgttgatacaggggacaaatatgcttgcaaatcgatatcgaagaagaaacttaggactgctgtagatatagatgatgttaggagagaagttgagatcatgaagcatttgcctaaacatcctaatattgtgaccttgaaggacacttatgaggatgataatgcagtgcatattgtgatggaactttgtgaggggggtgagttgtttgataggattgttgccaggggacattatacagagagagcagctgcggttattatgaagactatagtagaagttgttcaggtacagttttactaattgatgcttgtctttgcttttcatctataattgttacttgtttgtttatttcatgtaatttaggggttgctaatttaggattatgttaatgaagtttgaattgacaatgccaactgaaagtatcaatttagactagaaaggaatgttgagattgaagtttcatgtttgtaagcagaatgaatgttcttgtcgaagaatctcttttaagaatatctttcccacttcttcagtaaattttcctactttcttatgtcgataactgccactccttttctgagtttgcctgcactctcttggtagataggacactccctttcttagctcaggatttactttgcttgtgtaaatgagtgcttaatgtttttatttgattcattttacacgttgagatcctatagcatttaattagactagattttatcttccaatatcactaaacctagatgtcaaatatagtaaaaagttatgttgctcgaactcttcaaagatatcgacatgtgtgtgtcagatcctccaaaagtagtgcatttttggaggatccgacgggggtggggcaacaattttggagagttcgagcaacttaggtaaaaagtgtattcatgctctaaatgttgttaggttttctatctttcttatcttgtcttgtgaattttgctttcttggcaactgtttcattgtcctatatttttctcatgcaaatacctttaaaattatattctttcgtgccaaccatttaaatgaaacttaaggaagctaatcacacaggatttcaccatccaaatgtcgaaaatgaatcgcaatttgtgatagttttagacagagagcttatttttatagatgcaattagaataatagaaatgtaaaataactatcagtaaccagtaagatgccggtctttatggtctattttcagagggggagatctattgtagcttgctttcagcatcagttagtatagcataggactgttgctaacagggttcaattttaaactgtatttggtgaacataatgacatgagagctcaacttacataactacagattagagagagacattcattttatggaatggatttaagaagttcatgtttctacatttagttgttataagaacagggtggtaactggtaaccgacgcaaacatgatggctaattatcccaagtttatacaatttaatctatgtggttgctcatacatctttggtcaatgttcactttacagttgcattatgtttcctcaagaaatggctgttcttctttcaattttcaacttacggagtttcaattgacattgcagatgtgtcatatgcatggagtaatgcatcgtgatctcaaacctgagaactttctgtttggtaacaagaaagaaattgctcctttgaaggctattgactttggattatcagtgttctttaaacccggtaatgcaataagtaatgatagtgtgttgtaactttttttcatgctaaaaaagattaatgttggaatcatcttttaatatgtttaacaggggaacggtttaatgagattgtgggaagtccttattacatggctccagaggtcctaaaacgcaattatggcccggaggttgatgtctggagtgctggagttatcctttatattcttctttgtggtgttccacctttctgggcaggtccgtttcttttatttgccttctttaggtaacaagtaatacctcggttcaccgacaaataacaaattaaatcaaccttggtgcatactattcatttcttagaacttggtaatttattaatgagtgtcaaaatgaaatggaatttgaaacatattgatgcgttgttaacatcgtcgatgactaggtgagggtggctgcaagagtgaatcccacctcttcctggaccaattcaaaatcaaagttcctttttttccttttggcctgtgatagtcagtactttgtgcttccattaatttactcacagctttctcagtaattgcctaaaattctactgaatatgtgcagagactgaacaaggagtagcccaagcaattattcggtctgtggttgatttcaagagagatccatggcctaaggtttctgataatgcaaaggatcttgtaaagaagatgcttgacccggatccaactcgacgactcacagctcagcaggttcttggtaatgtttgttaatccttgagatgctatactttcatttgcttgctgtttgttctctcttagtttcataagttcaattttgtgacttttttggggctttcgtgcatatacatgaatgcagagcacacctggttacaaaatataaagaaagcaccaaatgtctcattgggtgagactgtgaaagcaaggcttaaacaattttcagtaatgaacaagctcaagaaaagagctctaacggtaaaatattcccttttcatttgcagttacatatcattagcgttctgcaccttctcagaaggatatcttcatatgcctaattcttaaagcccaaaataaggacaaaagattttctgccttctcacaaaagtttcgggtgttatattctttcttcattgcttgcacagattatggccgagtttttatcagcggaagaagtggctggaatgaaggacgcatttgatatgatggatacaggaaagaaaggcaagattaaccttggagaacttaaaaatggtctgcaaaagcttggccatcagatccctgatgttgatcttcagattcttatggaagctgtaagcattctcatgctcttcatttcacttgattggattttctttcaactttacgaagactaaatatatatatttataagtcaagcgtctaatattattataattgttccctttttgatcttctgcttcacttttataggcggatgttgatggagatggaagcttaaattatggggagtttgttgctgtatctgttcatctcagaaaaatggcaaatgatgagcacctgcacaaagcattttcagttttcgacagagatcagagtggttacatagaaatcgaggagctgcgcagtgccttgagtgatgaggatggtggcaacagtgaggaagtcatcaatgccattatgcatgatgttgacactgacaaggttagaattttttttgtgtccattcatgtatatctactggatttcatactagtgcatatacttctcttataaatgtctctttaattgcttgtggaaccataaataccccccttatcttgttccgcagttccaactacacacgaaactatgttgaagacgtattacccccttgtacttgtaaaatgtgtatcttccgtcatcctgagaggcatatatgatgtaaccaaatgtgaacatttaagtatatgcatgtgctgcctcatgtcatttacccctttttcccttttcacttctcttccatctccgcaacatgttaatgtcctctagcaaatctgaaaaaagatggagtgagcttctcaacggaaaaaatcggattcaccctagttttagttttctggcaacataaacagctcaagtcgatacaaaaaaacaaatgttcctatcaaaaaactcaaattagtagaaaggaaaagaagggtcataggtaagggaagaacaaaaaggaatagaaagacccttcggggtggcccagttatttgggcttggggcttccatgttggaggtctcaagttcaaaaccccttgccaatgaaagcaacgggttttccttctacgttgactgtcgagctcgtcgcaccgggcttacctagtgcggtttacctctcctttgcgtgctataggaataggggttttaccctgtgtgcactcaaagggtagcgactgcggatttcccaaaagaaaaaggaagagaaaggtaaagaaaacattttaaaaaagagtaggatggttataatagaagaaatgctataatattttttcacctcaggcgctttaagagagtaaatactctacgttacatggcgtcccaatgttgtcgtagttacattttggacaagaacagggagtaataggcctcccgcaaagttaaaatgtagtagggaatgggggaataattgaggaaggtatttatatattttctcctttctaaatcatattttcttttccattcactgctcttctgttcaaccttatcattcatttggactaaatgttgaattgattttgagcttttagtttgttaccacagcttcaaagttcatcagttacattgtctataaccatgcaggatggccgcattagttacgaggaatttgctgcaatgatgaaggctggcacagattggagaaaagcatcgagacagtattctcgtgaaagattcaacagtctcagcttaaaattgatgagagatggctcgatacaagtcggaaaggaagaaggtagatga

SEQ ID NO: 35 - DNA, 4897 bp, Solanum lycopersicum; identical to SEQ ID NO: 34
  source 1..4897: mol_type = genomic DNA

SEQ ID NO: 36 - DNA, 4914 bp, Solanum lycopersicum; identical to SEQ ID NO: 3
  source 1..4914: mol_type = genomic DNA

SEQ ID NO: 37 - DNA, 1602 bp, Solanum lycopersicum; identical to SEQ ID NO: 1
  source 1..1602: mol_type = other DNA

SEQ ID NO: 38 - DNA, 1638 bp, Solanum lycopersicum
  source 1..1638: mol_type = other DNA
atggggaattgctgtgggacacctggtaattcttctgagaataagaagaagaacaaaccaaacccgtttgctcttgattatggtgcaactcaagcatctggaggtgatggaaacaagcttgttgtgttgaaagatccaacaggacacaatattcaagaaaaatatgatcttggttgtgagctaggaagaggagaatttggggttacatatttatgtactgatgttgatacaggggacaaatatgcttgcaaatcgatatcgaagaagaaacttaggactgctgtagatatagatgatgttaggagagaagttgagatcatgaagcatttgcctaaacatcctaatattgtgaccttgaaggacacttatgaggatgataatgcagtgcatattgtgatggaactttgtgaggggggtgagttgtttgataggattgttgccaggggacattatacagagagagcagctgcggttgttatgaagactatagtagaagttgttcagatgtgtcatatgcatggagtaatgcatcgtgatctcaaacctgagaactttctgtttggtaacaagaaagaaattgctcctttgaaggctattgactttggattatcagtgttctttaaacccggggaacggtttaatgagattgtgggaagtccttattacatggctccagaggtcctaaaacgcaattatggcccggaggttgatgtctggagtgctggagttatcctttatattcttctttgtggtgttccacctttctgggcagagactgaacaaggagtagcccaagcaattattcggtctgtggttgatttcaagagagatccatggcctaaggtttctgataatgcaaaggatcttgtaaagaagatgcttgacccggatccaactcgacgactcacagctcagcaggttcttgagcacacctggttacaaaatataaagaaagcaccaaatgtctcattgggtgagactgtgaaagcaaggcttaaacaattttcagtaatgaacaagctcaagaaaagagctctaacgattatggccgagtttttatcagcggaagaagtggctggaatgaaggacgcatttgatatgatggatacaggaaagaaaggcaagattaaccttggagaacttaaaaatggtctgcaaaagcttggccatcagatccctgatgttgatcttcagattcttatggaagctgcggatgttgatggagatggaagcttaaattatggggagtttgttgctgtatctgttcatctcagaaaaatggcaaatgatgagcacctgcacaaagcattttcagttttcgacagagatcagagtggttacatagaaatcgaggagctgcgcagtgccttgagtgatgaggatggtggcaacagtgaggaagtcatcaatgccattatgcatgatgttgacactgacaagcttcaaagttcatcagttacattgtctataaccatgcaggatggccgcattagttacgaggaatttgctgcaatgatgaaggctggcacagattggagaaaagcatcgagacagtattctcgtgaaagattcaacagtctcagcttaaaattgatgagagatggctcgatacaagtcggaaaggaagaaggtagatga

SEQ ID NO: 39 - DNA, 1641 bp, Solanum lycopersicum
  source 1..1641: mol_type = other DNA
atggggaattgctgtgggacacctggtaattcttctgagaataagaagaagaagaacaaaccaaacccttttgctcttgattatggtgcaactcaagcatctggaggtgatggaaacaagcttgttgtgttgaaagatccaacaggacacaatattcaagaaaaatatgatcttggttgtgagctaggaagaggagaatttggggttacatatttatgtactgatgttgatacaggggacaaatatgcttgcaaatcgatatcaaagaagaaacttaggactgctgtagatatagatgatgttaggagagaagttgagatcatgaagcatttgcctaaacatcctaatattgtgaccttgaaggacacttatgaggatgataatgcagtgcatattgtgatggaactttgtgaggggggtgagttgtttgataggattgttgccaggggacattatacagagagagcagctgcggttattatgaagactatagtagaagttgttcagatgtgtcatatgcatggagtaatgcatcgtgatctcaaacctgagaactttctgtttggtaacaagaaagaaactgctcctttgaaggctattgactttggattatcagtgttctttaaacccggggaacgctttaatgagattgtgggaagtccttattacatggctccagaggtcctaaaacgcaattatggcccggaggttgatgtctggagtgctggagttatcctttatattcttctttgtggtgttccacctttctgggcagagactgaacaaggagtagcccaagcaattattcggtctgtggttgatttcaagagagatccatggcctaaggtttctgataatgcaaaggatcttgtaaagaagatgcttgacccggatccaactcgacgactcacagctcagcaggttcttgagcacacctggttacaaaatataaagaaagcaccaaatgtctcattgggtgagactgtgaaagcaaggcttaaacaattttcagtaatgaacaagctcaagaaaagagctctaacgattatggccgagtttttatcagcggaagaagtggctggaatgaaggacgcatttgatatgatggatacaggaaagaaaggcaagattaaccttggagaacttaaaaatggtctgcaaaagcttggccatcagatccctgatgttgatcttcagattcttatggaagctgcggatgttgatggagatggaagcttaaattatggggagtttgttgctgtatctgttcatctcagaaaaatggcaaatgatgagcacctgcacaaagcattttcagtttttgacagagatcagagtggttacatagaaatcgaggagctgcgcagtgccttgagtgatgaggatggtggcaacagtgaggaagtcatcaatgccattatgcatgatgttgacactgacaagcttcaaagttcatcagttacattgtctataaccatgcaggatggccgcattagttacgaggaatttgctgcaatgatgaaggctggcacagattggagaaaagcatcgagacagtattctcgtgaaagattcaacagtctcagcttaaaattgatgagagatggctcgatacaagtcggaaaggaagaaggtagatga

SEQ ID NO: 40 - DNA, 1641 bp, Solanum lycopersicum; identical to SEQ ID NO: 39
  source 1..1641: mol_type = other DNA

SEQ ID NO: 41 - DNA, 1602 bp, Solanum lycopersicum; identical to SEQ ID NO: 1
  source 1..1602: mol_type = other DNA

SEQ ID NO: 42 - DNA, 1713 bp, Solanum lycopersicum
  source 1..1713: mol_type = other DNA
atggggaattgctgtgggacacctggtaattcttctgagaataagaagaagaacaaaccaaacccgtttgctcttgattatggtgcaactcaagcatctggaggtgatggaaacaagcttgttgtgttgaaagatccaacaggacacaatattcaagaaaaatatgatcttggttgtgagctaggaagaggagaatttggggttacatatttatgtactgatgttgatacaggggacaaatatgcttgcaaatcgatatcgaagaagaaacttaggactgctgtagatatagatgatgttaggagagaagttgagatcatgaagcatttgcctaaacatcctaatattgtgaccttgaaggacacttatgaggatgataatgcagtgcatattgtgatggaactttgtgaggggggtgagttgtttgataggattgttgccaggggacattatacagagagagcagctgcggttattatgaagactatagtagaagttgttcagttgcattatgtttcctcaagaaatggctgttcttctttcaattttcaacttacggagtttcaattgacattgcagatgtgtcatatgcatggagtaatgcatcgtgatctcaaacctgagaactttctgtttggtaacaagaaagaaattgctcctttgaaggctattgactttggattatcagtgttctttaaacccggggaacggtttaatgagattgtgggaagtccttattacatggctccagaggtcctaaaacgcaattatggcccggaggttgatgtctggagtgctggagttatcctttatattcttctttgtggtgttccacctttctgggcagagactgaacaaggagtagcccaagcaattattcggtctgtggttgatttcaagagagatccatggcctaaggtttctgataatgcaaaggatcttgtaaagaagatgcttgacccggatccaactcgacgactcacagctcagcaggttcttgagcacacctggttacaaaatataaagaaagcaccaaatgtctcattgggtgagactgtgaaagcaaggcttaaacaattttcagtaatgaacaagctcaagaaaagagctctaacgattatggccgagtttttatcagcggaagaagtggctggaatgaaggacgcatttgatatgatggatacaggaaagaaaggcaagattaaccttggagaacttaaaaatggtctgcaaaagcttggccatcagatccctgatgttgatcttcagattcttatggaagctgcggatgttgatggagatggaagcttaaattatggggagtttgttgctgtatctgttcatctcagaaaaatggcaaatgatgagcacctgcacaaagcattttcagttttcgacagagatcagagtggttacatagaaatcgaggagctgcgcagtgccttgagtgatgaggatggtggcaacagtgaggaagtcatcaatgccattatgcatgatgttgacactgacaagcttcaaagttcatcagttacattgtctataaccatgcaggatggccgcattagttacgaggaatttgctgcaatgatgaaggctggcacagattggagaaaagcatcgagacagtattctcgtgaaagattcaacagtctcagcttaaaattgatgagagatggctcgatacaagtcggaaaggaagaaggtagatga

SEQ ID NO: 43 - DNA, 1641 bp, Solanum lycopersicum
  source 1..1641: mol_type = other DNA
atggggaattgctgtgggacacctggtaattcttctgagaataagaagaagaagaacaaaccaaacccttttgctcttgattatggtgcaactcaagcatctggaggtgatggaaacaagcttgttgtgttgaaagatccaacaggacacaatattcaagaaaaatatgatcttggttgtgagctaggaagaggagaatttggggttacatatttatgtactgatgttgatacaggggacaaatatgcttgcaaatcgatatcaaagaagaaacttaggactgctgtagatatagatgatgttaggagagaagttgagatcatgaagcatttgcctaaacatcctaatattgtgaccttgaaggacacttatgaggatgataatgcagtgcatattgtgatggaactttgtgaggggggtgagttgtttgataggattgttgccaggggacattatacagagagagcagctgcggttattatgaagactatagtagaagttgttcagatgtgtcatatgcatggagtaatgcatcgtgatctcaaacctgagaactttctgtttggtaacaagaaagaaactgctcctttgaaggctattgactttggattatcagtgttctttaaacccggggaacgctttaatgagattgtgggaagtccttattacatggctccagaggtcctaaaacgcaattatggcccggaggttgatgtctggagtgctggagttatcctttatattcttctttgtggtgttccacctttctgggcagagactgaacaaggagtagcccaagcaattattcggtctgtggttgatttcaagagagatccatggcctaaggtttctgataatgcaaaggatcttgtaaagaagatgcttgacccggatccaactcgacgactcacagctcagcaggttcttgagcacacctggttacaaaatataaagaaagcaccaaatgtctcattgggtgagactgtgaaagcaaggcttaaacaattttcagtaatgaacaagctcaagaaaagagctctaacgattatggccgagtttttatcagcggaagaagtggctggaatgaaggacgcatttgatatgatggatacaggaaagaaaggcaagattaaccttggagaacttaaaaatggtctgcaaaagcttggccatcagatacctgatgttgatcttcagattcttatggaagctgcggatgttgatggagatggaagcttaaattatggggagtttgttgctgtatctgttcatctcagaaaaatggcaaatgatgagcacctgcacaaagcattttcagtttttgacagagatcagagtggttacatagaaatcgaggagctgcgcagtgccttgagtgatgaggatggtggcaacagtgaggaagtcatcaatgccattatgcatgatgttgacactgacaagcttcaaagttcatcagttacattgtctataaccatgcaggatggccgcattagttacgaggaatttgctgcaatgatgaaggctggcacagattggagaaaagcatcgagacagtattctcgtgaaagattcaacagtctcagcttaaaattgatgagagatggctcgatacaagtcggaaaggaagaaggtagatga

SEQ ID NO: 44 - DNA, 1602 bp, Solanum lycopersicum; identical to SEQ ID NO: 1
  source 1..1602: mol_type = other DNA

SEQ ID NO: 45 - DNA, 1602 bp, Solanum lycopersicum; identical to SEQ ID NO: 1
  source 1..1602: mol_type = other DNA

SEQ ID NO: 46 - DNA, 1599 bp, Solanum lycopersicum
  source 1..1599: mol_type = other DNA
atggggaattgctgtgggacacctggtaattcttctgagaataagaagaagaacaaaccaaacccgtttgctcttgattatggtgcaactcaagcatctggaggtgatggaaacaagcttgttgtgttgaaagatccaacaggacacaatattcaagaaaaatatgatcttggttgtgagctaggaagaggagaatttggggttacatatttatgtactgatgttgatacaggggacaaatatgcttgcaaatcgatatcgaagaagaaacttaggactgctgtagatatagatgatgttaggagagaagttgagatcatgaagcatttgcctaaacatcctaatattgtgaccttgaaggacacttatgaggatgataatgcagtgcatattgtgatggaactttgtgaggggggtgagttgtttgataggattgttgccaggggacattatacagagagagcagctgcggttattatgaagactatagtagaagttgttcagatgtgtcatatgcatggagtaatgcatcgtgatctcaaacctgagaactttctgtttggtaacaagaaagaaattgctcctttgaaggctattgactttggattatcagtgttctttaaacccggggaacggtttaatgagattgtgggaagtccttattacatggctccagaggtcctaaaacgcaattatggcccggaggttgatgtctggagtgctggagttatcctttatattcttctttgtggtgttccacctttctgggcagagactgaacaaggagtagcccaagcaattattcggtctgtggttgatttcaagagagatccatggcctaaggtttctgataatgcaaaggatcttgtaaagaagatgcttgacccggatccaactcgacgactcacagctcagcaggttcttgagcacacctggttacaaaatataaagaaagcaccaaatgtctcattgggtgagactgtgaaagcaaggcttaaacaattttcagtaatgaacaagctcaagaaaagagctctaacgattatggccgagtttttatcagcggaagaagtggctggaatgaaggacgcatttgatatgatggatacaggaaagaaaggcaagattaaccttggagaacttaaaaatggtctgcaaaagcttggccatcagatccctgatgttgatcttcagattcttatggaagctgcggatgttgatggagatggaagcttaaattatggggagtttgttgctgtatctgttcatctcagaaaaatggcaaatgatgagcacctgcacaaagcattttcagttttcgacagagatcagagtggttacatagaaatcgaggagctgcgcagtgccttgagtgatgaggatggtggcaacagtgaggaagtcatcaatgccattatgcatgatgttgacactgacaaggatggccgcattagttacgaggaatttgctgcaatgatgaaggctggcacagattggagaaaagcatcgagacagtattctcgtgaaagattcaacagtctcagcttaaaattgatgagagatggctcgatacaagtcggaaaggaagaaggtagatga

SEQ ID NO: 47 - DNA, 1599 bp, Solanum lycopersicum
  source 1..1599: mol_type = other DNA
atggggaattgctgtgggacacctggtaattcttctgagaataagaagaagaacaaaccaaacccgtttgctcttgattatggtgcaactcaagcatctggaggtgatggaaacaagcttgttgtgttgaaagatccaacaggacacaatattcaagaaaaatatgatcttggttgtgagctaggaagaggagaatttggggttacatatttatgtactgatgttgatacaggggacaaatatgcttgcaaatcgatatcgaagaagaaacttaggactgctgtagatatagatgatgttaggagagaagttgagatcatgaagcatttgcctaaacatcctaatattgtgaccttgaaggacacttatgaggatgataatgcagtgcatattgtgatggaactttgtgaggggggtgagttgtttgataggattgttgccaggggacattatacagagagagcagctgcggttattatgaagactatagtagaagttgttcagatgtgtcatatgcatggagtaatgcatcgtgatctcaaacctgagaactttctgtttggtaacaagaaagaaattgctcctttgaaggctattgactttggattatcagtgttctttaaacccggggaacggtttaatgagattgtgggaagtccttattacatggctccagaggtcctaaaacgcaattatggcccggaggttgatgtctggagtgctggagttatcctttatattcttctttgtggtgttccacctttctgggcagagactgaacaaggagtagcccaagcaattattcggtctgtggttgatttcaagagagatccatggcctaaggtttctgataatgcaaaggatcttgtaaagaagatgcttgacccagatccaactcgacgactcacagctcagcaggttcttgagcacacctggttacaaaatataaagaaagcaccaaatgtctcattgggtgagactgtgaaagcaaggcttaaacaattttcagtaatgaacaagctcaagaaaagagctctaacgattatggccgagtttttatcagcggaagaagtggctggaatgaaggacgcatttgatatgatggatacaggaaagaaaggcaagattaaccttggagaacttaaaaatggtctgcaaaagcttggccatcagatccctgatgttgatcttcagattcttatggaagctgcggatgttgatggagatggaagcttaaattatggggagtttgttgctgtatctgttcatctcagaaaaatggcaaatgatgagcacctgcacaaagcattttcagttttcgacagagatcagagtggttacatagaaatcgaggagctgcgcagtgccttgagtgatgaggatggtggcaacagtgaggaagtcatcaatgccattatgcatgatgttgacactgacaaggatggccgcattagttacgaggaatttgctgcaatgatgaaggctggcacagattggagaaaagcatcgagacagtattctcgtgaaagattcaacagtctcagcttaaaattgatgagagatggctcgatacaagtcggaaaggaagaaggtagatga

SEQ ID NO: 48 - DNA, 1713 bp, Solanum lycopersicum; identical to SEQ ID NO: 42
  source 1..1713: mol_type = other DNA

SEQ ID NO: 49 - DNA, 1677 bp, Solanum lycopersicum
  source 1..1677: mol_type = other DNA
atggggaattgctgtgggacacctggtaattcttctgagaataagaagaagaagaacaaaccaaacccttttgctcttgattatggtgcaactcaagcatctggaggtgatggaaacaagcttgttgtgttgaaagatccaacaggacacaatattcaagaaaaatatgatcttggttgtgagctaggaagaggagaatttggggttacatatttatgtactgatgttgatacaggggacaaatatgcttgcaaatcgatatcaaagaagaaacttaggactgctgtagatatagatgatgttaggagagaagttgagatcatgaagcatttgcctaaacatcctaatattgtgaccttgaaggacacttatgaggatgataatgcagtgcatattgtgatggaactttgtgaggggggtgagttgtttgataggattgttgccaggggacattatacagagagagcagctgcggttattatgaagactatagtagaagttgttcagttgcattatgtttcctcaagaaatggctgttcttctttcaattttcaacttacggagtttcaattgacattgcagatgtgtcatatgcatggagtaatgcatcgtgatctcaaacctgagaactttctgtttggtaacaagaaagaaactgctcctttgaaggctattgactttggattatcagtgttctttaaacccggggaacgctttaatgagattgtgggaagtccttattacatggctccagaggtcctaaaacgcaattatggcccggaggttgatgtctggagtgctggagttatcctttatattcttctttgtggtgttccacctttctgggcagagactgaacaaggagtagcccaagcaattattcggtctgtggttgatttcaagagagatccatggcctaaggtttctgataatgcaaaggatcttgtaaagaagatgcttgacccggatccaactcgacgactcacagctcagcaggttcttgagcacacctggttacaaaatataaagaaagcaccaaatgtctcattgggtgagactgtgaaagcaaggcttaaacaattttcagtaatgaacaagctcaagaaaagagctctaacgattatggccgagtttttatcagcggaagaagtggctggaatgaaggacgcatttgatatgatggatacaggaaagaaaggcaagattaaccttggagaacttaaaaatggtctgcaaaagcttggccatcagatccctgatgttgatcttcagattcttatggaagctgcggatgttgatggagatggaagcttaaattatggggagtttgttgctgtatctgttcatctcagaaaaatggcaaatgatgagcacctgcacaaagcattttcagtttttgacagagatcagagtggttacatagaaatcgaggagctgcgcagtgccttgagtgatgaggatggtggcaacagtgcggaagtcatcaatgccattatgcatgatgttgacactgacaaggatggccgcattagttacgaggaatttgctgcaatgatgaaggctggcacagattggagaaaagcatcgagacagtattctcgtgaaagattcaacagtctcagcttaaaattgatgagagatggctcgatacaagtcggaaaggaagaaggtagatga

SEQ ID NO: 50 - DNA, 1716 bp, Solanum lycopersicum
  source 1..1716: mol_type = other DNA
atggggaattgctgtgggacacctggtaattcttctgagaataagaagaagaagaacaaaccaaacccttttgctcttgattatggtgcaactcaagcatctggaggtgatggaaacaagcttgttgtgttgaaagatccaacaggacacaatattcaagaaaaatatgatcttggttgtgagctaggaagaggagaatttggggttacatatttatgtactgatgttgatacaggggacaaatatgcttgcaaatcgatatcaaagaagaaacttaggactgctgtagatatagatgatgttaggagagaagttgagatcatgaagcatttgcctaaacatcctaatattgtgaccttgaaggacacttatgaggatgataatgcagtgcatattgtgatggaactttgtgaggggggtgagttgtttgataggattgttgccaggggacattatacagagagagcagctgcggttattatgaagactatagtagaagttgttcagttgcattatgtttcctcaagaaatggctgttcttctttcaattttcaacttacggagtttcaattgacattgcagatgtgtcatatgcatggagtaatgcatcgtgatctcaaacctgagaactttctgtttggtaacaagaaagaaactgctcctttgaaggctattgactttggattatcagtgttctttaaacccggggaacgctttaatgagattgtgggaagtccttattacatggctccagaggtcctaaaacgcaattatggcccggaggttgatgtctggagtgctggagttatcctttatattcttctttgtggtgttccacctttctgggcagagactgaacaaggagtagcccaagcaattattcggtctgtggttgatttcaagagagatccatggcctaaggtttctgataatgcaaaggatcttgtaaagaagatgcttgacccggatccaactcgacgactcacagctcagcaggttcttgagcacacctggttacaaaatataaagaaagcaccaaatgtctcattgggtgagactgtgaaagcaaggcttaaacaattttcagtaatgaacaagctcaagaaaagagctctaacgattatggccgagtttttatcagcggaagaagtggctggaatgaaggacgcatttgatatgatggatacaggaaagaaaggcaagattaaccttggagaacttaaaaatggtctgcaaaagcttggccatcagatccctgatgttgatcttcagattcttatggaagctgcggatgttgatggagatggaagcttaaattatggggagtttgttgctgtatctgttcatctcagaaaaatggcaaatgatgagcacctgcacaaagcattttcagtttttgacagagatcagagtggttacatagaaatcgaggagctgcgcagtgccttgagtgatgaggatggtggcaacagtgaggaagtcatcaatgccattatgcatgatgttgacactgacaagcttcaaagttcatcagttacattgtctataaccatgcaggatggccgcattagttacgaggaatttgctgcaatgatgaaggctggcacagattggagaaaagcatcgagacagtattctcgtgaaagattcaacagtctcagcttaaaattgatgagagatggctcgatacaagtcggaaaggaagaaggtagatga

SEQ ID NO: 51 - DNA, 1641 bp, Solanum lycopersicum; identical to SEQ ID NO: 39
  source 1..1641: mol_type = other DNA

SEQ ID NO: 52 - DNA, 1677 bp, Solanum lycopersicum
  source 1..1677: mol_type = other DNA
atggggaattgctgtgggacacctggtaattcttctgagaataagaagaagaagaacaaaccaaacccttttgctcttgattatggtgcaactcaagcatctggaggtgatggaaacaagcttgttgtgttgaaagatccaacaggacacaatattcaagaaaaatatgatcttggttgtgagctaggaagaggagaatttggggttacatatttatgtactgatgttgatacaggggacaaatatgcttgcaaatcgatatcaaagaagaaacttaggactgctgtagatatagatgatgttaggagagaagttgagatcatgaagcatttgcctaaacatcctaatattgtgaccttgaaggacacttatgaggatgataatgcagtgcatattgtgatggaactttgtgaggggggtgagttgtttgataggattgttgccaggggacattatacagagagagcagctgcggttattatgaagactatagtagaagttgttcagttgcattatgtttcctcaagaaatggctgttcttctttcaattttcaacttacggagtttcaattgacattgcagatgtgtcatatgcatggagtaatgcatcgtgatctcaaacctgagaactttctgtttggtaacaagaaagaaactgctcctttgaaggctattgactttggattatcagtgttctttaaacccggggaacgctttaatgagattgtgggaagtccttattacatggctccagaggtcctaaaacgcaattatggcccggaggttgatgtctggagtgctggagttatcctttatattcttctttgtggtgttccacctttctgggcagagactgaacaaggagtagcccaagcaattattcggtctgtggttgatttcaagagagatccatggcctaaggtttctgataatgcaaaggatcttgtaaagaagatgcttgacccggatccaactcgacgactcacagctcagcaggttcttgagcacacctggttacaaaatataaagaaagcaccaaatgtctcattgggtgagactgtgaaagcaaggcttaaacaattttcagtaatgaacaagctcaagaaaagagctctaacgattatggccgagtttttatcagcggaagaagtggctggaatgaaggacgcatttgatatgatggatacaggaaagaaaggcaagattaaccttggagaacttaaaaatggtctgcaaaagcttggccatcagatccctgatgttgatcttcagattcttatggaagctgcggatgttgatggagatggaagcttaaattatggggagtttgttgctgtatctgttcatctcagaaaaatggcaaatgatgagcacctgcacaaagcattttcagtttttgacagagatcagagtggttacatagaaatcgaggagctgcgcagtgccttgagtgatgaggatggtggcaacagtgaggaagtcatcaatgccattatgcatgatgttgacactgacaaggatggccgcattagttacgaggaatttgctgcaatgatgaaggctggcacagattggagaaaagcatcgagacagtattctcgtgaaagattcaacagtctcagcttaaaattgatgagagatggctcgatacaagtcggaaaggaagaaggtagatga

SEQ ID NO: 53 - DNA, 1677 bp, Solanum lycopersicum; identical to SEQ ID NO: 52
  source 1..1677: mol_type = other DNA

SEQ ID NO: 54 - DNA, 1674 bp, Solanum lycopersicum
  source 1..1674: mol_type = other DNA
atggggaattgctgtgggacacctggtaattcttctgagaataagaagaagaacaaaccaaacccgtttgctcttgattatggtgcaactcaagcatctggaggtgatggaaacaagcttgttgtgttgaaagatccaacaggacacaatattcaagaaaaatatgatcttggttgtgagctaggaagaggagaatttggggttacatatttatgtactgatgttgatacaggggacaaatatgcttgcaaatcgatatcgaagaagaaacttaggactgctgtagatatagatgatgttaggagagaagttgagatcatgaagcatttgcctaaacatcctaatattgtgaccttgaaggacacttatgaggatgataatgcagtgcatattgtgatggaactttgtgaggggggtgagttgtttgataggattgttgccaggggacattatacagagagagcagctgcggttattatgaagactatagtagaagttgttcagttgcattatgtttcctcaagaaatggctgttcttctttcaattttcaacttacggagtttcaattgacattgcagatgtgtcatatgcatggagtaatgcatcgtgatctcaaacctgagaactttctgtttggtaacaagaaagaaattgctcctttgaaggctattgactttggattatcagtgttctttaaacccggggaacggtttaatgagattgtgggaagtccttattacatggctccagaggtcctaaaacgcaattatggcccggaggttgatgtctggagtgctggagttatcctttatattcttctttgtggtgttccacctttctgggcagagactgaacaaggagtagcccaagcaattattcggtctgtggttgatttcaagagagatccatggcctaaggtttctgataatgcaaaggatcttgtaaagaagatgcttgacccggatccaactcgacgactcacagctcagcaggttcttgagcacacctggttacaaaatataaagaaagcaccaaatgtctcattgggtgagactgtgaaagcaaggcttaaacaattttcagtaatgaacaagctcaagaaaagagctctaacgattatggccgagtttttatcagcggaagaagtggctggaatgaaggacgcatttgatatgatggatacaggaaagaaaggcaagattaaccttggagaacttaaaaatggtctgcaaaagcttggccatcagatccctgatgttgatcttcagattcttatggaagctgcggatgttgatggagatggaagcttaaattatggggagtttgttgctgtatctgttcatctcagaaaaatggcaaatgatgagcacctgcacaaagcattttcagttttcgacagagatcagagtggttacatagaaatcgaggagctgcgcagtgccttgagtgatgaggatggtggcaacagtgaggaagtcatcaatgccattatgcatgatgttgacactgacaaggatggccgcattagttacgaggaatttgctgcaatgatgaaggctggcacagattggagaaaagcatcgagacagtattctcgtgaaagattcaacagtctcagcttaaaattgatgagagatggctcgatacaagtcggaaaggaagaaggtagatga

SEQ ID NO: 55 - DNA, 1677 bp, Solanum lycopersicum; identical to SEQ ID NO: 52
  source 1..1677: mol_type = other DNA

SEQ ID NO: 56 - DNA, 1713 bp, Solanum lycopersicum; identical to SEQ ID NO: 42
  source 1..1713: mol_type = other DNA

SEQ ID NO: 57 - DNA, 1641 bp, Solanum lycopersicum
  source 1..1641: mol_type = other DNA
atggggaattgctgtgggacacctggtaattcttctgagaataagaagaagaagaacaaaccaaacccttttgctcttgattatggtgcaactcaagcatctggaggtgatggaaacaagcttgttgtgttgaaagatccaacaggacacaatattcaagaaaaatatgatcttggttgtgagctaggaagaggagaatttggggttacatatttatgtactgatgttgatacaggggacaaatatgcttgcaaatcgatatcaaagaagaaacttaggactgctgtagatatagatgatgttaggagagaagttgagatcatgaagcatttgcctaaacatcctaatattgtgaccttgaaggacacttatgaggatgataatgcagtgcatattgtgatggaactttgtgaggggggtgagttgtttgataggattgttgccaggggacattatacagagagagcagctgcggttattatgaagactatagtagaagttgttcagatgtgtcatatgcatggagtaatgcatcgtgatctcaaacctgagaactttctgtttggtaacaagaaagaaactgctcctttgaaggctattgactttggattatcagtgttctttaaacccggggaacgctttaatgagattgtgggaagtccttattacatggctccagaggtcctaaaacgcaattatggcccggaggttgatgtctggagtgctggagttatcctttatattcttctttgtggtgttccacctttctgggcagagactgaacaaggagtagcccaagcaattattcggtctgtggttgatttcaagagagatccatggcctaaggtttctgataatgcaaaggatcttgtaaagaagatgcttgacccggatccaactcgacgactcacagctcagcaggttcttgagcacacctggttacaaaatataaagaaagcaccaaatgtctcattgggtgagactgtgaaagcaaggcttaaacaattttcagtaatgaacaagctcaagaaaagagctctaacgattatggccgagtttttatcagcggaagaagtggctggaatgaaggacgcatttgatatgatggatacaggaaagaaaggcaagattaaccttggagaacttaaaaatggtctgcaaaagcttggccatcagatccctgatgttgatcttcagattcttatggaagctgcggatgttgatggagatggaagcttaaattatggggagtttgttgctgtatctgttcatctcagaaaaatggcaaatgatgagcacctgcacaaagcattttcagtttttgacagagatcagagtggttacatagaaatcgaggagctgcgcagtgccttgagtgatgaggatggtggcaacagtgcggaagtcatcaatgccattatgcatgatgttgacactgacaagcttcaaagttcatcagttacattgtctataaccatgcaggatggccgcattagttacgaggaatttgctgcaatgatgaaggctggcacagattggagaaaagcatcgagacagtattctcgtgaaagattcaacagtctcagcttaaaattgatgagagatggctcgatacaagtcggaaaggaagaaggtagatga

SEQ ID NO: 58 - DNA, 1677 bp, Solanum lycopersicum; identical to SEQ ID NO: 52
  source 1..1677: mol_type = other DNA

SEQ ID NO: 59 - DNA, 1602 bp, Solanum lycopersicum
  source 1..1602: mol_type = other DNA
atggggaattgctgtgggacacctggtaattcttctgagaataagaagaagaagaacaaaccaaacccttttgctcttgattatggtgcaactcaagcatctggaggtgatggaaacaagcttgttgtgttgaaagatccaacaggacacaatattcaagaaaaatatgatcttggttgtgagctaggaagaggagaatttggggttacatatttatgtactgatgttgatacaggggacaaatatgcttgcaaatcgatatcaaagaagaaacttaggactgctgtagatatagatgatgttaggagagaagttgagatcatgaagcatttgcctaaacatcctaatattgtgaccttgaaggacacttatgaggatgataatgcagtgcatattgtgatggaactttgtgaggggggtgagttgtttgataggattgttgccaggggacattatacagagagagcagctgcggttattatgaagactatagtagaagttgttcagatgtgtcatatgcatggagtaatgcatcgtgatctcaaacctgagaactttctgtttggtaacaagaaagaaactgctcctttgaaggctattgactttggattatcagtgttctttaaacccggggaacgctttaatgagattgtgggaagtccttattacatggctccagaggtcctaaaacgcaattatggcccggaggttgatgtctggagtgctggagttatcctttatattcttctttgtggtgttccacctttctgggcagagactgaacaaggagtagcccaagcaattattcggtctgtggttgatttcaagagagatccatggcctaaggtttctgataatgcaaaggatcttgtaaagaagatgcttgacccggatccaactcgacgactcacagctcagcaggttcttgagcacacctggttacaaaatataaagaaagcaccaaatgtctcattgggtgagactgtgaaagcaaggcttaaacaattttcagtaatgaacaagctcaagaaaagagctctaacgattatggccgagtttttatcagcggaagaagtggctggaatgaaggacgcatttgatatgatggatacaggaaagaaaggcaagattaaccttggagaacttaaaaatggtctgcaaaagcttggccatcagatccctgatgttgatcttcagattcttatggaagctgcggatgttgatggagatggaagcttaaattatggggagtttgttgctgtatctgttcatctcagaaaaatggcaaatgatgagcacctgcacaaagcattttcagtttttgacagagatcagagtggttacatagaaatcgaggagctgcgcagtgccttgagtgatgaggatggtggcaacagtgcggaagtcatcaatgccattatgcatgatgttgacactgacaaggatggccgcattagttacgaggaatttgctgcaatgatgaaggctggcacagattggagaaaagcatcgagacagtattctcgtgaaagattcaacagtctcagcttaaaattgatgagagatggctcgatacaagtcggaaaggaagaaggtagatga

SEQ ID NO: 60 - DNA, 1713 bp, Solanum lycopersicum; identical to SEQ ID NO: 42
  source 1..1713: mol_type = other DNA

SEQ ID NO: 61 - DNA, 1641 bp, Solanum lycopersicum; identical to SEQ ID NO: 39
  source 1..1641: mol_type = other DNA

SEQ ID NO: 62 - DNA, 1713 bp, Solanum lycopersicum; identical to SEQ ID NO: 42
  source 1..1713: mol_type = other DNA

SEQ ID NO: 63 - DNA, 1677 bp, Solanum lycopersicum; identical to SEQ ID NO: 52
  source 1..1677: mol_type = other DNA

SEQ ID NO: 64 - DNA, 1713 bp, Solanum lycopersicum; identical to SEQ ID NO: 42
  source 1..1713: mol_type = other DNA

SEQ ID NO: 65 - DNA, 1677 bp, Solanum lycopersicum; identical to SEQ ID NO: 52
  source 1..1677: mol_type = other DNA

SEQ ID NO: 66 - protein, 545 aa, Solanum lycopersicum
MGNCCGTPGNSSENKKKNKPNPFALDYGATQASGGDGNKLVVLKDPTGHNIQEKYDLGCELGRGEFGVTYLCTDVDTGDKYACKSISKKKLRTAVDIDDVRREVEIMKHLPKHPNIVTLKDTYEDDNAVHIVMELCEGGELFDRIVARGHYTERAAAVVMKTIVEVVQMCHMHGVMHRDLKPENFLFGNKKEIAPLKAIDFGLSVFFKPGERFNEIVGSPYYMAPEVLKRNYGPEVDVWSAGVILYILLCGVPPFWAETEQGVAQAIIRSVVDFKRDPWPKVSDNAKDLVKKMLDPDPTRRLTAQQVLEHTWLQNIKKAPNVSLGETVKARLKQFSVMNKLKKRALTIMAEFLSAEEVAGMKDAFDMMDTGKKGKINLGELKNGLQKLGHQIPDVDLQILMEAADVDGDGSLNYGEFVAVSVHLRKMANDEHLHKAFSVFDRDQSGYIEIEELRSALSDEDGGNSEEVINAIMHDVDTDKLQSSSVTLSITMQDGRISYEEFAAMMKAGTDWRKASRQYSRERFNSLSLKLMRDGSIQVGKEEGR

SEQ ID NO: 67 - protein, 571 aa, Solanum lycopersicum
MGNCCGTPGNSSENKKKKNKPNPFALDYGATQASGGDGNKLVVLKDPTGHNIQEKYDLGCELGRGEFGVTYLCTDVDTGDKYACKSISKKKLRTAVDIDDVRREVEIMKHLPKHPNIVTLKDTYEDDNAVHIVMELCEGGELFDRIVARGHYTERAAAVIMKTIVEVVQLHYVSSRNGCSSFNFQLTEFQLTLQMCHMHGVMHRDLKPENFLFGNKKETAPLKAIDFGLSVFFKPGERFNEIVGSPYYMAPEVLKRNYGPEVDVWSAGVILYILLCGVPPFWAETEQGVAQAIIRSVVDFKRDPWPKVSDNAKDLVKKMLDPDPTRRLTAQQVLEHTWLQNIKKAPNVSLGETVKARLKQFSVMNKLKKRALTIMAEFLSAEEVAGMKDAFDMMDTGKKGKINLGELKNGLQKLGHQIPDVDLQILMEAADVDGDGSLNYGEFVAVSVHLRKMANDEHLHKAFSVFDRDQSGYIEIEELRSALSDEDGGNSEEVINAIMHDVDTDKLQSSSVTLSITMQDGRISYEEFAAMMKAGTDWRKASRQYSRERFNSLSLKLMRDGSIQVGKEEGR

SEQ ID NO: 68 - protein, 571 aa, Solanum lycopersicum; identical to SEQ ID NO: 67

SEQ ID NO: 69 - protein, 533 aa, Solanum lycopersicum; identical to SEQ ID NO: 2

SEQ ID NO: 70 - protein, 570 aa, Solanum lycopersicum
MGNCCGTPGNSSENKKKNKPNPFALDYGATQASGGDGNKLVVLKDPTGHNIQEKYDLGCELGRGEFGVTYLCTDVDTGDKYACKSISKKKLRTAVDIDDVRREVEIMKHLPKHPNIVTLKDTYEDDNAVHIVMELCEGGELFDRIVARGHYTERAAAVIMKTIVEVVQLHYVSSRNGCSSFNFQLTEFQLTLQMCHMHGVMHRDLKPENFLFGNKKEIAPLKAIDFGLSVFFKPGERFNEIVGSPYYMAPEVLKRNYGPEVDVWSAGVILYILLCGVPPFWAETEQGVAQAIIRSVVDFKRDPWPKVSDNAKDLVKKMLDPDPTRRLTAQQVLEHTWLQNIKKAPNVSLGETVKARLKQFSVMNKLKKRALTIMAEFLSAEEVAGMKDAFDMMDTGKKGKINLGELKNGLQKLGHQIPDVDLQILMEAADVDGDGSLNYGEFVAVSVHLRKMANDEHLHKAFSVFDRDQSGYIEIEELRSALSDEDGGNSEEVINAIMHDVDTDKLQSSSVTLSITMQDGRISYEEFAAMMKAGTDWRKASRQYSRERFNSLSLKLMRDGSIQVGKEEGR

SEQ ID NO: 71 - protein, 546 aa, Solanum lycopersicum
MGNCCGTPGNSSENKKKKNKPNPFALDYGATQASGGDGNKLVVLKDPTGHNIQEKYDLGCELGRGEFGVTYLCTDVDTGDKYACKSISKKKLRTAVDIDDVRREVEIMKHLPKHPNIVTLKDTYEDDNAVHIVMELCEGGELFDRIVARGHYTERAAAVIMKTIVEVVQMCHMHGVMHRDLKPENFLFGNKKETAPLKAIDFGLSVFFKPGERFNEIVGSPYYMAPEVLKRNYGPEVDVWSAGVILYILLCGVPPFWAETEQGVAQAIIRSVVDFKRDPWPKVSDNAKDLVKKMLDPDPTRRLTAQQVLEHTWLQNIKKAPNVSLGETVKARLKQFSVMNKLKKRALTIMAEFLSAEEVAGMKDAFDMMDTGKKGKINLGELKNGLQKLGHQIPDVDLQILMEAADVDGDGSLNYGEFVAVSVHLRKMANDEHLHKAFSVFDRDQSGYIEIEELRSALSDEDGGNSEEVINAIMHDVDTDKLQSSSVTLSITMQDGRISYEEFAAMMKAGTDWRKASRQYSRERFNSLSLKLMRDGSIQVGKEEGR

SEQ ID NO: 72 - protein, 571 aa, Solanum lycopersicum; identical to SEQ ID NO: 67

SEQ ID NO: 73 - protein, 533 aa, Solanum lycopersicum; identical to SEQ ID NO: 2

SEQ ID NO: 74 - protein, 532 aa, Solanum lycopersicum
MGNCCGTPGNSSENKKKNKPNPFALDYGATQASGGDGNKLVVLKDPTGHNIQEKYDLGCELGRGEFGVTYLCTDVDTGDKYACKSISKKKLRTAVDIDDVRREVEIMKHLPKHPNIVTLKDTYEDDNAVHIVMELCEGGELFDRIVARGHYTERAAAVIMKTIVEVVQMCHMHGVMHRDLKPENFLFGNKKEIAPLKAIDFGLSVFFKPGERFNEIVGSPYYMAPEVLKRNYGPEVDVWSAGVILYILLCGVPPFWAETEQGVAQAIIRSVVDFKRDPWPKVSDNAKDLVKKMLDPDPTRRLTAQQVLEHTWLQNIKKAPNVSLGETVKARLKQFSVMNKLKKRALTIMAEFLSAEEVAGMKDAFDMMDTGKKGKINLGELKNGLQKLGHQIPDVDLQILMEAADVDGDGSLNYGEFVAVSVHLRKMANDEHLHKAFSVFDRDQSGYIEIEELRSALSDEDGGNSEEVINAIMHDVDTDKDGRISYEEFAAMMKAGTDWRKASRQYSRERFNSLSLKLMRDGSIQVGKEEGR

SEQ ID NO: 75 - protein, 571 aa, Solanum lycopersicum; identical to SEQ ID NO: 67

SEQ ID NO: 76 - protein, 532 aa, Solanum lycopersicum; identical to SEQ ID NO: 74

SEQ ID NO: 77 - protein, 570 aa, Solanum lycopersicum; identical to SEQ ID NO: 70

SEQ ID NO: 78 - protein, 558 aa, Solanum lycopersicum
MGNCCGTPGNSSENKKKKNKPNPFALDYGATQASGGDGNKLVVLKDPTGHNIQEKYDLGCELGRGEFGVTYLCTDVDTGDKYACKSISKKKLRTAVDIDDVRREVEIMKHLPKHPNIVTLKDTYEDDNAVHIVMELCEGGELFDRIVARGHYTERAAAVIMKTIVEVVQLHYVSSRNGCSSFNFQLTEFQLTLQMCHMHGVMHRDLKPENFLFGNKKETAPLKAIDFGLSVFFKPGERFNEIVGSPYYMAPEVLKRNYGPEVDVWSAGVILYILLCGVPPFWAETEQGVAQAIIRSVVDFKRDPWPKVSDNAKDLVKKMLDPDPTRRLTAQQVLEHTWLQNIKKAPNVSLGETVKARLKQFSVMNKLKKRALTIMAEFLSAEEVAGMKDAFDMMDTGKKGKINLGELKNGLQKLGHQIPDVDLQILMEAADVDGDGSLNYGEFVAVSVHLRKMANDEHLHKAFSVFDRDQSGYIEIEELRSALSDEDGGNSAEVINAIMHDVDTDKDGRISYEEFAAMMKAGTDWRKASRQYSRERFNSLSLKLMRDGSIQVGKEEGR

SEQ ID NO: 79 - protein, 571 aa, Solanum lycopersicum; identical to SEQ ID NO: 67

SEQ ID NO: 80 - protein, 546 aa, Solanum lycopersicum; identical to SEQ ID NO: 71

SEQ ID NO: 81 - protein, 558 aa, Solanum lycopersicum
MGNCCGTPGNSSENKKKKNKPNPFALDYGATQASGGDGNKLVVLKDPTGHNIQEKYDLGCELGRGEFGVTYLCTDVDTGDKYACKSISKKKLRTAVDIDDVRREVEIMKHLPKHPNIVTLKDTYEDDNAVHIVMELCEGGELFDRIVARGHYTERAAAVIMKTIVEVVQLHYVSSRNGCSSFNFQLTEFQLTLQMCHMHGVMHRDLKPENFLFGNKKETAPLKAIDFGLSVFFKPGERFNEIVGSPYYMAPEVLKRNYGPEVDVWSAGVILYILLCGVPPFWAETEQGVAQAIIRSVVDFKRDPWPKVSDNAKDLVKKMLDPDPTRRLTAQQVLEHTWLQNIKKAPNVSLGETVKARLKQFSVMNKLKKRALTIMAEFLSAEEVAGMKDAFDMMDTGKKGKINLGELKNGLQKLGHQIPDVDLQILMEAADVDGDGSLNYGEFVAVSVHLRKMANDEHLHKAFSVFDRDQSGYIEIEELRSALSDEDGGNSEEVINAIMHDVDTDKDGRISYEEFAAMMKAGTDWRKASRQYSRERFNSLSLKLMRDGSIQVGKEEGR

SEQ ID NO: 82 - protein, 558 aa, Solanum lycopersicum; identical to SEQ ID NO: 81

SEQ ID NO: 83 - protein, 557 aa, Solanum lycopersicum
MGNCCGTPGNSSENKKKNKPNPFALDYGATQASGGDGNKLVVLKDPTGHNIQEKYDLGCELGRGEFGVTYLCTDVDTGDKYACKSISKKKLRTAVDIDDVRREVEIMKHLPKHPNIVTLKDTYEDDNAVHIVMELCEGGELFDRIVARGHYTERAAAVIMKTIVEVVQLHYVSSRNGCSSFNFQLTEFQLTLQMCHMHGVMHRDLKPENFLFGNKKEIAPLKAIDFGLSVFFKPGERFNEIVGSPYYMAPEVLKRNYGPEVDVWSAGVILYILLCGVPPFWAETEQGVAQAIIRSVVDFKRDPWPKVSDNAKDLVKKMLDPDPTRRLTAQQVLEHTWLQNIKKAPNVSLGETVKARLKQFSVMNKLKKRALTIMAEFLSAEEVAGMKDAFDMMDTGKKGKINLGELKNGLQKLGHQIPDVDLQILMEAADVDGDGSLNYGEFVAVSVHLRKMANDEHLHKAFSVFDRDQSGYIEIEELRSALSDEDGGNSEEVINAIMHDVDTDKDGRISYEEFAAMMKAGTDWRKASRQYSRERFNSLSLKLMRDGSIQVGKEEGR

SEQ ID NO: 84 - protein, 558 aa, Solanum lycopersicum; identical to SEQ ID NO: 81

SEQ ID NO: 85 - protein, 570 aa, Solanum lycopersicum; identical to SEQ ID NO: 70

SEQ ID NO: 86 - protein, 546 aa, Solanum lycopersicum
MGNCCGTPGNSSENKKKKNKPNPFALDYGATQASGGDGNKLVVLKDPTGHNIQEKYDLGCELGRGEFGVTYLCTDVDTGDKYACKSISKKKLRTAVDIDDVRREVEIMKHLPKHPNIVTLKDTYEDDNAVHIVMELCEGGELFDRIVARGHYTERAAAVIMKTIVEVVQMCHMHGVMHRDLKPENFLFGNKKETAPLKAIDFGLSVFFKPGERFNEIVGSPYYMAPEVLKRNYGPEVDVWSAGVILYILLCGVPPFWAETEQGVAQAIIRSVVDFKRDPWPKVSDNAKDLVKKMLDPDPTRRLTAQQVLEHTWLQNIKKAPNVSLGETVKARLKQFSVMNKLKKRALTIMAEFLSAEEVAGMKDAFDMMDTGKKGKINLGELKNGLQKLGHQIPDVDLQILMEAADVDGDGSLNYGEFVAVSVHLRKMANDEHLHKAFSVFDRDQSGYIEIEELRSALSDEDGGNSAEVINAIMHDVDTDKLQSSSVTLSITMQDGRISYEEFAAMMKAGTDWRKASRQYSRERFNSLSLKLMRDGSIQVGKEEGR

SEQ ID NO: 87 - protein, 558 aa, Solanum lycopersicum; identical to SEQ ID NO: 81

SEQ ID NO: 88 - protein, 533 aa, Solanum lycopersicum
MGNCCGTPGNSSENKKKKNKPNPFALDYGATQASGGDGNKLVVLKDPTGHNIQEKYDLGCELGRGEFGVTYLCTDVDTGDKYACKSISKKKLRTAVDIDDVRREVEIMKHLPKHPNIVTLKDTYEDDNAVHIVMELCEGGELFDRIVARGHYTERAAAVIMKTIVEVVQMCHMHGVMHRDLKPENFLFGNKKETAPLKAIDFGLSVFFKPGERFNEIVGSPYYMAPEVLKRNYGPEVDVWSAGVILYILLCGVPPFWAETEQGVAQAIIRSVVDFKRDPWPKVSDNAKDLVKKMLDPDPTRRLTAQQVLEHTWLQNIKKAPNVSLGETVKARLKQFSVMNKLKKRALTIMAEFLSAEEVAGMKDAFDMMDTGKKGKINLGELKNGLQKLGHQIPDVDLQILMEAADVDGDGSLNYGEFVAVSVHLRKMANDEHLHKAFSVFDRDQSGYIEIEELRSALSDEDGGNSAEVINAIMHDVDTDKDGRISYEEFAAMMKAGTDWRKASRQYSRERFNSLSLKLMRDGSIQVGKEEGR

SEQ ID NO: 89 - protein, 570 aa, Solanum lycopersicum; identical to SEQ ID NO: 70

SEQ ID NO: 90 - protein, 546 aa, Solanum lycopersicum; identical to SEQ ID NO: 71

SEQ ID NO: 91 - protein, 570 aa, Solanum lycopersicum; identical to SEQ ID NO: 70

SEQ ID NO: 92 - protein, 558 aa, Solanum lycopersicum; identical to SEQ ID NO: 81

SEQ ID NO: 93 - protein, 570 aa, Solanum lycopersicum; identical to SEQ ID NO: 70

SEQ ID NO: 94 - protein, 558 aa, Solanum lycopersicum; identical to SEQ ID NO: 81

SEQ ID NO: 95 - DNA, 5520 bp, Solanum lycopersicum
  source 1..5520: mol_type = genomic DNA
atgggtaattgctgtgtgaaaccgggtaaatctgccgaaaaaaagaataaaaagaacaacagcaaacctaaccctttttcaattgattatggggggactaaacatgcctctgggagtggaaacaagctagttgtattaaaagaaccaacagggcaaaatatacatgataagtatgatttggggcgtgagctcggaagaggagaatttggggttacttatctatgtactgacttggaaggaggagaaaaatatgcttgcaaatcgatatctaaaaagaagctaaggactgcagtggatattgatgatgttaggagagaggttgagatcatgaaacatttgcctgtgcatccgaatattgtgaccttgaaggatacttatgaggatgataatgcagtgcacattgtgatggaattgtgtgagggtggggagttgtttgatcgaatcgttgctagaggccactatacagagagagcagctgctggaattttgaagactgtcgtggaagtcgttcaggtatagtttttatcagcttcttagttctcagttacctactgcttttattaccttttgcttaggttatcttattatatccattattttcagcatagcttcttcattactgtatttccttttcatattgtttttatatatgtcttacttaggctgagggtccattggaaatagcctctctaccttcacaaggtaggagtaaggctgcgtacacactacccttcccacaccccacttgtgggactatactaagtatgttgttgttttagttctcaattgatgctttttggtttttatgtagtaacttgtggtgtttcttttactgagttcttcaaagcttttgtatgggttttatatcatgacggatgtatcctgtattgttgtttcgggtttttattaaagaagtctggcaatttcaagttaaaaagaaaatcatatcttaaaagagaagcctaatcttgagcaaatcttgagcagatagcaatttcagggtgaaatgtgaatattcttggtgaagttgcatatgaactggtaaccattattcaattcatttctagtgttgatctttgcaatcaatggtttcattctagtgtacgttcatgctgtagcatttaccttgatatcctcatggaatttcctttaccgccaaaattataatgagaagtggttatcttttttaataatggtaaagtatgagaagaggttttcttatgttctcagtctttgctagttctatttctttactcgttttacttaacttttttagtttcttgtgaactgtagtattgctctatatcttctcactcaaattcatgttctaaatcttaaccattctagtgatataaatgaagttaattggtgatataggatatccccctccaaaatctaacaatctttcaactcatcatagtcttgggcagatagctagttagaaccgtaacaaatatttaggaaagtagatcattcgaaatagttatccttgtgaaatattattctttatcttcattattgaccattggttttcaaactctagtactcttaagtggaagattcacttcttgtttctgtggagtattaactatagcggcctacaacagaatttgattgttgcactcaaagttaaacagagttctacagtttagggaaatgataatggaatttaaatttagtttgtatactgaagtaaatatggttgacactatcagaaacaagtgctttttacttcaaatattgatctttatcctcattgcgaaccattgatgtccaaactgttttagatggaagagcaatttgttgttcatttgagtggaatagtcaccaacaacagctaattaactacgtatagcttagagagatgcgaaccaatggtaaatttaagttgtctcctgaagtagttactgattgttcatgataaaggtcattaaagttgaattctctatttagtcagtgtccttttctgcatcgactatatagtggcctgaatgacattacaaaatatttatgagttggtaggaatctttttttcatatgtgaatcatgaatgtgttcacaaatgatcaatcagagagtgattattgtattatgtggtgttgataacttttgaacttttcttcatttggtttgtgtttaactgttatctgaaaggcttggttggtggtactaaagctattggattagcagaaaactttatacatgtttatggtcatgtttcgctctccagtccccgtttttatttgtcaaaggtcagttcatatatttccaatggttttgcagatgtgtcacaggcaaggggtaatgcatcgtgatctcaaacctgagaattttctttttggtaacaagaaagaaacagctccactgaaggctattgactttgggttgtctgttttctttaaacctggtaatggaattggaaaaaaaacagtgagtttaagacttttatcatgctaaacaaaggtttaacatgttgattattttaacaggggaacgctttaatgagatagtgggaagtccttattacatggctcctgaggtcctaaagcgcaattatggaccagaggtcgatgtctggagtgctggagttatactttacattcttctatgcggtgttccacctttctgggcaggtctgcttattttatttcttcgttttttataaccatggaacgaacctcaatgcagatattttcatgtgcaatttttggaacttgataattgattaactaagattgtgaatatgaagtagaacttgattcatgttagaatatgtcgttgaaatattagatgatgaggcaagtgaggtgaaagactgtccctgctttaatcaatgtagatcatgttcaattattttggtttctcttaatggttcttatgggttggactttgctaaataacttgcataaatatgttaacatattcttgatacttcccttaagttcctctgaatatttgcagagactgaacaaggagtagcccaagcgattattcgttctgtgattgatttcaagagggatccatggcctaaagtttctgataatgcaaaggatcttgtaaagaaaatgcttgatccagatccaactcgacggctcacagctcatcaagttcttggtaatgtttgtggaatattgagatattgtactttattcattcgttgttttactctctctctctctctctctctatctatctctgataagtatttttttccggggctttgactcttgtggtgcagagcatccctggttacataatataaagaaagcaccaaatgtctcattgggtgagactgttaaagcaagactcaagcagttttcagtaatgaacaagctcaagaaaaaagctctgacggtaagcacacacttagtctgcaatcatatttataagctctggattcttcactgtccactaaagatgaattcatatgcttttcctcatagatcgaaatgaaggagagaagattgtgtcttaattatttactgcactgccttgtgctatttaataaaaacttaattctcatcgtaaaaaatgagaggaggttctcaaaattttgatcaagtttcgtttttttatcttgatatatgtactttcttgtattccaaacaggttatagctgagtttttgtctgcggaggaagtcgctggaatgaaggaagcatttgaaatgatggataccggaaagaagggtaagataaacctgaatgaacttaaagatggcttgcagaagcttggccatcaaatccctgatgctgatcttcatattctcatggaagcggtaagcggtctcatgccctgcttcttggctcgatcagatttcttatagctctaccgggggtaacataatatttgaaagttagctgctaaacttttctgcctcaaagagaaaacaggtgcctgagatgatatggccatgtcttacgtagaactgtaaattacatcaatggacattattttaaaatgaccgaaaactacatggaatccatgtgaacttagtaaagaaaatattcaatggaagtaaaggataccaagtagttggattaaggctagattgttggtggtacactgacattagtgtctcaatgtttactaagagtctcagtttgattagagatttgcacgtagatgcagggataaccgtgagattaagaaaattttaagaaattcacggagatgaaaaagatctgtaatactcatatagcttagggccaagcccaactagtttgggatcaaatcgtagttgttgttgataagaatttagcattagacttttgtctgtcaccctactgtcaaaaaattgattgattacaaaatatattttgtcaatataagttgtaacatttttctaccatttcaatgtagaaaaaaggaaaatctgtagcaaaattagcttgacatttcgcttgtcttagcatccctggttcaatgcttattattatccagaaaggaaaaaaaaaacatttctcttgatccttttgcatcttcgacctgaaggatgcttatcttttttattattttatttccttgaacttttgttttatgtttttcttattctgtatcggttttacaggctgacgttgatggagatggaagtttaaattatccagagtttgttgctgtatctattcatcttagaaagatggccaatgatgaacacctgcacaaagcattttcatttttcgacaaaaatcagagtggtttcatagaaatcgaagagcttcgtagtgctttgagggatgaagacgacagcaacagcgaggaagtcaccaatgccattatgcatgacgttgatacagacaaggtcagtatgtccatttatgtgcacgtacaccatttagtaacttttcgttctttggttcatacttcatagtgcaaatattatgcattgttgctaatgtttacatcttaatgagttctcattttgaagttctcttctgaaccctcgtttgagtttagagctcaaatactccacctagttgtgacttattgtatctctaaagtccgtcatattatataaacgtattatactttgatggcatgcacactttctagcacatatgtgttgctaacgaaactctagtgctgtgacaaatgaaatacatgtatacattgatggcatctgttcttcccatcacatatgtactaccggtcattactctctagtgctgtgacattatgctctccctgttcgcttcatgagttacacggttggttaacctgctgctcgttacatgtctgctacagaattcaagttttgttagctgttttccatctcatctctaacaacatccccactcatttgtattagcttcttatctggagttttgtgagctcagtcttgtatcgtcttgtgtcaaaacgtgtgcaggatggtcggattagttatgaggaatttgctgcgatgatgaaggctggtacggactggagaaaagcatcgagacagtattctcgtgaacgttttaacagtctaagcttaaagttgatgagggaaggctcattacaagttgaaaacaaagtctag

SEQ ID NO: 96 - DNA, 5526 bp, Solanum lycopersicum
  source 1..5526: mol_type = genomic DNA
atgggtaattgctgtgtgaaaccgggtaaatctgccgaaaaaaagaataaaaagaacaacagcaaacctaaccctttttcaattgattatggggggactaaacatgcctctgggagtggaaacaagctagttgtattaaaagaaccaacagggcaaaatatacatgataagtatgatttggggcatgagctcggaagaggagaatttggggttacttatctatgtactgacttggaaggaggagaaaaatatgcttgcaaatcgatatctaaaaagaagctaaggactgcagtggatattgatgatgttaggagagaggttgagatcatgaaacatttgcctgtgcatccgaatattgtgaccttgaaggatacttatgaggatgataatgcagtgcacattgtgatggaattgtgtgagggtggggagttgtttgatcgaatcgttgctagaggccactatacagagagagcagctgctggaattttgaagactgtcgtggaagtcgttcaggtatagtttttatcaacttcttagttctcagttacctactgcttttattaccttttgcttaggttatcttattatatccattattttcagcatagcttcttcattactgtatttccttttcatattgtttttatatatgtcttacttaggctgagggtccattggaaatagcctctctaccttcacaaggtaggagtaaggctgcgtacacactacccttcccacaccccacttgtgggactatactaagtatgttgttgttttagttctcaattgatgctttttggtttttatgtagtaacttgtggtgtttcttttactgagttcttcaaagcttttgtatgggttttatatcatgacggatgtatcctgtattgttgtttcgggtttttattaaagaagtctggcaatttcaagttaaaaagaaaatcatatcttaaaagagaagcctaatcttgagcaaatcttgagcagatagcaatttcagggtgaaatgtgaatattcttggtgaagttgcatatgaactggtaaccattattcaattcatttctagtgttgatctttgcaatcaatggtttcattctagtgtacgttcatgctgtagcatttaccttgatatcctcatggaatttcctttactgccaaaattataatgagaagtggttatcttttttaataatggtaaagtatgagaagaggttttcttatgttctcagtctttgctagttctatttctttactcgttttacttaacttttttagtttcttgtgaactgtagtattgctctatatcttctcactcaaattcatgttctaaatcttaaccattctagtgatataaatgaagttaattggtgatataggatatccccctccaaaatctaacaatctttcaactcatcatagtcttgggcagatagctagttagaaccgtaacaaatatttaggaaagtagatcattcgaaatagttatccttgtgaaatattattctttatcttcattattgaccattggttttcaaactctagtactcttaagtggaagactcacttcttgtttctgtggagtattagctatagcggcctacaacagaatttgattgttgcactcaaagttaaacagagttctacagtttagggaaatgataatggaatttaaatttagtttgtatactgaagtaaatatggttgacactatcagaaacaagtgctttttacttcaaatattgatctttatcctcattgcgaaccattgatgtccaaactgttttagatggaagagcaatttgttgttcatttgagtggaatagtcaccaacaacagctaattaactacgtatagcttagagagatgcgaaccaatggtaaatttaagttgtctcctgaagtagttactgattgttcatgataaaggtcattaaagttgaattctctatttagtcagtgtccttttctgcatcaactatatagtggcctgaatgacattacaaaatatttatgagttggtaggaatctttttttcatatgtgaatcatgaatgtgttcacaaatgatcaatcagagagtgattattgtattatgtggtgttgataacttttgaacttttcttcatttggtttgtgtttaactgttatctgaaaggcttggttggtggtactaaagctattggattagcagaaaactttatacatgtttatggtcatgtttcgctctccagtccccgtttttatttgtcaaaggtcagttcatatatttccaatggttttgcagatgtgtcacaggcaaggggtaatgcatcgtgatctcaaacctgagaattttctttttggtaacaagaaagaaacagctccactgaaggctattgactttgggttgtctgttttctttaaacctggtaatggaattggaaaaaaaacagtgagtttaagacttttatcatgctaaacaaaggtttaacatgttgattattttaacaggggaacgctttaatgagatagtgggaagtccttattacatggctcctgaggtcctaaagcgcaattatggaccagaggtcgatgtctggagtgctggagttatactttacattcttctatgcggtgttccacctttctgggcaggtctgcttattttatttcttcgttttttataaccatggaacgaacctcaatgcagatattttcatgtgcaatttttggaacttgataattgattaactaagattgtgaatatgaagtagaacttgattcatgttagaatatgttgttgaaatattagatgatgaggcaagtgaggtgaaagactgtccctgctttaatcaatgtagatcatgttcaattattttggtttctcttaatggttcttatgggttggactttgctaaataacttgcataaatatgttaacatattcttgatacttcccttaagttcctctgaatatttgcagagactgaacaaggagtagcccaagcgattattcgttctgtgattgatttcaagagggatccatggcctaaagtttctgataatgcaaaggatcttgtaaagaaaatgcttgatccagatccaactcgacggctcacagctcatcaagttcttggtaatgtttgtggaatattgagatattgtactttattcattcgttgttttactctctctctctctctctctctctctctatctatctctgataagtatttttttccggggctttgactcttgtggtgcagagcatccctggttacataatataaagaaagcaccaaacgtctcattgggtgagactgttaaagcaagactcaagcagttttcagtaatgaacaagctcaagaaaaaagctctgacggtaagcacacacttagtctgcaatcatatttataagctctggattcttcactgtccactaaagatgaattcatatgcttttcctcatagatcgaaatgaaggagagaaggttgtgtcttaattatttactgcactgccttgtgctatttaataaaaacttaattctcatcgtaaaaaatgagaggcggttctcaaaattttgatcaagtttcgtttttttatcttgatatatgtactttcttgtattccaaacaggttatagctgagtttttgtctgcggaggaagtcgctggaatgaaggaagcatttgaaatgatggataccggaaagaagggcaagataaacctgaatgaacttaaagatggcttgcagaagcttggccatcaaatccctgatgctgatcttcatattctcatggaagcggtaagcggtctcatgccctgcttcttggctcgatcagatttcttatagctctaccgggggtaacataatatttgaaagttagctgctaaacttttctgcctcaaagagaaaacaggtgcctgagatgatatggccatgtcttacgtagaactgtaaattacatcaatggacattattttaaaatgaccgaaaactacatggaatccatgtgaacttagtaaagaaaatattcaatggaagtaaaggataccaagtagttggattaaggctagattgttggtggtacactgacattagtgtctcaatgtttactaagagtctcagtttgattagagatttgcacgtagatgcagggataaccgtgagattaagaaaattttaagaaattcacggagatgaaaaagatctgtaatactcatatagcttagggccaagcccaactagtttgggatcaaatcgtagttgttgttgataagaatttagcattagacttttgtctgtcaccctactgtcaaaaaattgattgattacaaaatatattttgtcaatataagttgtaacatttttctaccatttcaatgtagaaaaaaggaaaatctgtagcaaaattagcttgacatttcgcttgtcttatcatccctggttcaatgcttattattatccagaaaggaaaaaaaaaacatttctcttgatccttttgcatcttcgacctgaaggatgcttatcttttttattattttatttccttgaacttttgttttatgtttttcttattctgtatcggttttacaggctgacgttgatggagatggaagtttaaattatccagagtttgttgctgtatctattcatcttagaaagatggccaatgatgaacacctgcacaaagcattttcatttttcgacaaaaatcagagtggtttcatagaaatcgaagagcttcgtagtgctttgagggatgaagacgacagcaacagcgaggaagtcaccaatgccattatgcatgacgttgatacagacaaggtcagtatgtccatttatgtgcacgtacaccatttagtaacttttcgttctttggttcatacttcatagtgcaaatattatgcattgttgctaatgtttacatcttaatgagttctcattttgaagttctcttctgaaccctcgtttgagtttagagctcaaatactccacctagttgtgacttattgtatctctaaagtccgtcatattatataaacgtattatactttgatggcatgcacactttctagcacatatgtgttgctaacgaaactctagtgctgtgacaaatgaaatacatgtatacattgatggcatctgttcttcccatcacatatgtactaccggtcattactctctagtgctgtgacattatgctctccctgttcgcttcatgagttacacggttggttaacctgctgctcgttacatgtctgctacagaattcaagttttgttagctgttttccatctcatctctaacaacatccccactcatttgtattagcttcttatctggagttttgtgagctcagtcttgtatcgtcttgtgtcaaaacgtgtgcaggatggtcggattagttatgaggaatttgctgcgatgatgaaggctggtacggactggagaaaagcatcgagacagtattctcgtgaacgttttaacagtctaagcttaaagttgatgagggaaggctcattacaagttgaaaacaaagtctag

SEQ ID NO: 97 - DNA, 5520 bp, Solanum lycopersicum
  source 1..5520: mol_type = genomic DNA
atgggtaattgctgtgtgaaaccgggtaaatctgccgaaaaaaagaataaaaagaacaacagcaaacctaaccctttttcaattgattatggggggactaaacatgcctctgggagtggaaacaagctagttgtattaaaagaaccaacagggcaaaatatacatgataagtatgatttggggcgtgagctcggaagaggagaatttggggttacttatctatgtactgacttggaaggaggagaaaaatatgcttgcaaatcgatatctaaaaagaagctaaggactgcagtggatattgatgatgttaggagagaggttgagatcatgaaacatttgcctgtgcatccgaatattgtgaccttgaaggatacttatgaggatgataatgcagtgcacattgtgatggaattgtgtgagggtggggagttgtttgatcgaatcgttgctagaggccactatacagagagagcagctgctggaattttgaagactgtcgtggaagtcgttcaggtatagtttttatcagcttcttagttctcagttacctactgcttttattaccttttgcttaggttatcttattatatccattattttcagcatagcttcttcattactgtatttccttttcatattgtttttatatatgtcttacttaggctgagggtccattggaaatagcctctctaccttcacaaggtaggagtaaggctgcgtacacactacccttcccacaccccacttgtgggactatactaagtatgttgttgttttagttcacaattgatgctttttggtttttatgtagtaacttctggtgtttcttttactgagttcttcaaagcttttgtatgggttttatatcatgacggatgtatcctgtattgttgtttcgggtttttattaaagaagtctggcaatttcaagttaaaaagaaaatcatatcttaaaagagaagcctaatcttgagcagatagcaatttcagggtgaaatgtgaatattcttggtgaagttgcatatgaacatatgaactggctaaccattattcaattcatttctagtgttgatctttgcaatcaatggtttcattctagtgtacgttcatgctgtagcatttaccttgatatcctcatggaatttcctttaccgccaaaattataatgagaagtggttatcttttttaataatggtaaagtatgagaagaggttttcttatgttctcagtctttgctagttctatttctttactcgttttacttaacttttttagtttcttgtgaactgtagtattgctctatatcttctcactcaaattcatgttctaaatcttaaccattctagtgatataaatgaagttaattggtgatataggatatccccctccaaaatctaacaatctttcaactcatcatagtcttgggcagatagctagttagaaccgtaacaaatatttaggaaagtagatcattcgaaatagttatccttgtgaaatattattctttatcttcattattgaccattggttttcaaactctagtactcttaagtggaagactcacttcttgtttctgtggagtattagctatagcggcctacaacagaatttgattgttgcactcaaagttaaacagagttctacagtttagggaaatgataatggaatttaaatttagtttgtatactgaagtaaatatggttgacactatcagaaacaagtgctttttacttcaaatattgatctttatcctcattgcgaaccattgatgtccaaactgttttagatggaagagcaatttgttgttcatttgagtggaatagtcaccaacaacagctaattaactacgtatagcttagagagatgcgaaccaatggtaaatttaagttgtctcctgaagtagttactgattgttcatgataaaggtcattaaagttgaattctctatttagtcagcgtccttttctgcatcgactatatagtggcctgaatgacattacaaaatatttatgagttggtaggaatctttttttcatatgtgaatcatgaatgtgttcacaaatgatcaatcagagagtgattattgtattatgtggtgttgataacttttgaacttttcttcatttggtttgtgtttaactgttatctgaaaggcttggttggtggtactaaagctattggattagcagaaaactttatacatgtttatggtcatgtttcgctctccagtctccgtttttatttgtcaaaggtcagttcatatatttccaatggttttgcagatgtgtcacaggcaaggggtaatgcatcgtgatctcaaacctgagaattttctttttggtaacaagaaagaaacagctccactgaaggctattgactttgggttgtctgttttctttaaacctggtaatggaattggaaaagaaacagtgagtttaagacttttatcatgctaaacaaaggtttaacattttgattattttaacaggggaacgctttaatgagatagtgggaagtccttattacatggctcctgaggtcctaaagcgcaattatggaccagaggtcgatgtctggagtgctggagttatactttacattcttctatgcggtgttccacctttctgggcaggtctgcttattttatttcttcgttttttataaccatggaacgaacctcaatgcagatattttcatgtgcaatttttggaacttgataattgattaactaagattgtgaatatgaagtagaacttgattcatgttagaatatgtcgttgaaatattagatgatgaggcaagtgaggtgaaagactgtccctgctttaatcaatgtagatcatgttcaattattttggtttctcttaatggttcttatgggttggactttgctaaataacttgcataaatatgttaacatattcttgatacttcccttaagttcctctgaatatttgcagagactgaacaaggagtagcccaagcgattattcgttctgtgattgatttcaagagggatccatggcctaaagtttctgataatgcaaaggatcttgtaaagaaaatgcttgatccagatccaactcgacggctcacagctcatcaagttcttggtaatgtttgtggaatattgagatattgtactttattcattcgttgttttactctctctctctctctctctctctatctatctctgataagtattttttttccggggctttgactcttgtggtgcagagcatccctggttacataatataaagaaagcaccaaacgtctcattgggtgagactgttaaagcaagactcaagcagttttcagtaatgaacaagctcaagaaaaaagctctgacggtaagcacacacttagtctgcaatcatatttataagctctggtttcttcactgtccactaaagatgaattcatatgcttttcctcatagatcgaaatgaaggagagaaggttgtgtcttaattatttactgcactgccttgtgctatttaataaaaacttaattctcatcgtaaaaaatgagaggcggttctcaaaattttgatcaagtttcgtttttttatcttgatatatgtactttcttgtattccaaacaggttatagctgagtttttgtctgcggaggaagtcgctggaatgaaggaagcatttgaaatgatggataccggaaagaagggcaagataaacctgaatgaacttaaagatggcttgcagaagcttggccatcaaatccctgatgctgatcttcatattctcatggaagcggtaagcggtctcatgccctgcttcttggctcgatcagatttcttatagctctaccgggggtaacataatatttgaaagttagctgctaaacttttctgcctcaaagagaaaacaggtgcctgagatgatatggccatgtcttacgtagaactgtaaattacatcaatggacattattttaaaatgaccgaaaactacatggaatccatgtgaacttagtaaagaaaatattcaatggaagtaaaggataccaagtagttggattaaggctagattgttggtggtacactgacattagtgtctcaatgtttactaagagtctcagtttgattagagatttgcacgtagatgcagggataaccgtgagattaagaaaattttaagaaattcacggagatgaaaaagatctgtaatactcatatagcttagggccaagcccaactagtttgggatcaaatcgtagttgttgttgataagaatttagcattagacttttgtctgtcaccctactgtcaaaaaattgattgattacaaaatatattttgtcaatataagttgtaacatttttctaccatttcaatgtagaaaaaaggaaaatctgtagcaaaattagcttgacatttcgcttgtcttagcatccctggttcaatgcttattattatccagaaaggaaaaaaaaacatttctcttgatccttttgcatcttcgacctgaaggatgcttatcttttttattattttatttccttgaacttttgttttatgtttttcttattctgtatcggttttacaggctgacgttgatggagatggaagtttaaattatccagagtttgttgctgtatctattcatcttagaaagatggccaatgatgaacacctgcacaaagcattttcatttttcgacaaaaatcagagtggtttcatagaaatcgaagagcttcgtagtgctttgagggatgaagacgacagcaacagcgaggaagtcaccaatgccattatgcatgacgttgatacagacaaggtcagtatgtccatttatgtgcacgtacaccatttagtaacttttcgttctttggttcatacttcatagtgcaaatattatgcatcgatgctaatgtttacatcttaatgagttctcattttgaagttcccttctgaaccctcgtttgagtttagagctcaaatactccacctagttgtgacttattgtatctctaaagtccgtcatgttatataaacgtattatactttgatggcatgcacactttctagcacatatgtgttgctaacgaaactctagtgctgtgacaaatgaaatacatgtatacattgatggcatctgttcttcccatcacatatgtactaccggtcattactctctagtgctgtgacattatgctctccctgttcgcttcatgatttacacggttggttaacctgctgctcgttacatgtctgctacagaattcaagttttgttagctgttttccatctcatctctaacaacatccccactcatttgtattagcttcttatctggagttttgtgagctcagtcttgtatcgtcttgtgtcaaaacgtgtgcaggatggtcggattagttatgaggaatttgctgcgatgatgaaggctggtacggactggagaaaagcatcgagacagtattctcgtgaacgttttaacagtctaagcttaaagttgatgagggaaggctcattacaagttgaaaacaaagtctag

SEQ ID NO: 98 - DNA, 5517 bp, Solanum lycopersicum
  source 1..5517: mol_type = genomic DNA
atgggtaattgctgtgtaaaaccgggtaaatctgccgaaaaaaagaataaaaagaacaacagcaaacctaaccctttttcaattgattatggggggactaaacatgcctctgggagtggaaacaagctagttgtattaaaagaaccaacagggcaaaatatacatgataagtatgatttggggcgtgagctcggaagaggagaatttggggttacttatctatgtactgacttggaaggaggagaaaaatatgcttgcaaatcgatatctaaaaagaagctaaggactgcagtggatattgatgatgttaggagagaggttgagatcatgaaacatttgcctgtgcatccgaatattgtgaccttgaaggatacttatgaggatgataatgcagtgcacattgtgatggaattgtgtgagggtggggagttgtttgatcgaatcgttgctagaggccactatacagagagagcagctgctggaattttgaagactgtcgtggaagtcgttcaggtatagtttttatcagcttcttagttctcagttacctactgcttttattaccttttgcttaggttatcttattatatccattattttcagcatagcttcttcattactgtatttccttttcatattgtttttatatatgtcttacttaggctgagggtccattggaaatagcctctctaccttcacaaggtaggagtaaggctgcgtacacactacccttcccacaccccacttgtgggactatactaagtatgttgttgttttagttcacaattgatgctttttggtttttatgtagtaacttctggtgtttcttttactgagttcttcaaagcttttgtatgggttttatatcatgacggatgtatcctgtattgttgtttcgggtttttattaaagaagtctggcaatttcaagttaaaaagaaaatcatatcttaaaagagaagcctaatcttgagcagatagcaatttcagggtgaaatgtgaatattcttggtgaagttgcatatgaacatatgaactggctaaccattattcaattcatttctagtgttgatctttgcaatcaatggtttcattctagtgtacgttcatgctgtagcatttaccttgatatcctcatggaatttcctttaccgccaaaattataatgagaagtggttatcttttttaataatggtaaagtatgagaagaggttttcttatgttctcagtctttgctagttctatttctttactcgttttacttaacttttttagtttcttgtgaactgtagtattgctctatatcttctcactcaaattcatgttctaaatcttaaccattctagtgatataaatgaagttaattggtgatataggatatccccctccaaaatctaacaatctttcaactcatcatagtcttgggcagatagctagttagaaccgtaacaaatatttaggaaagtagatcattcgaaatagttatccttgtgaaatattattctttatcttcattattgaccattggttttcaaactctagtactcttaagtggaagactcacttcttgtttctgtggagtattagctatagcggcctacaacagaatttgattgttgcactcaaagttaaacagagttctacagtttagggaaatgataatggaatttaaatttagtttgtatactgaagtaaatatggttgacactatcagaaacaagtgctttttacttcaaatattgatctttatcctcattgcgaaccattgatgtccaaactgttttagatggaagagcaatttgttgttcatttgagtggaatagtcaccaacaacagctaattaactacgtatagcttagagagatgcgaaccaatggtaaatttaagttgtctcctgaagtagttactgattgttcatgataaaggtcattaaagttgaattctctatttagtcagcgtccttttctgcatcgactatatagtggcctgaatgacattacaaaatatttatgagttggtaggaatctttttttcatatgtgaatcatgaatgtgttcacaaatgatcaatcagagagtgattattgtattatgtggtgttgataacttttgaacttttcttcatttggtttgtgtttaactgttatctgaaaggcttggttggtggtactaaagctattggattagcagaaaactttatacatgtttatggtcatgtttcgctctccagtctccgtttttatttgtcaaaggtcagttcatatatttccaatggttttgcagatgtgtcacaggcaaggggtaatgcatcgtgatctcaaacctgagaattttctttttggtaacaagaaagaaacagctccactgaaggctattgactttgggttgtctgttttctttaaacctggtaatggaattggaaaagaaacagtgagtttaagacttttatcatgctaaacaaaggtttaacattttgattattttaacaggggaacgctttaatgagatagtgggaagtccttattacatggctcctgaggtcctaaagcgcaattatggaccagaggtcgatgtctggagtgctggagttatactttacattcttctatgcggtgttccacctttctgggcaggtctgcttattttatttcttcgttttttataaccatggaacgaacctcaatgcagatattttcatgtgcaatttttggaacttgataattgattaactaagattgtgaatatgaagtagaacttgattcatgttagaatatgtcgttgaaatattagatgatgaggcaagtgaggtgaaagactgtccctgctttaatcaatgtagatcatgttcaattattttggtttctcttaatggttcttatgggttggactttgctaaataacttgcataaatatgttaacatattcttgatacttcccttaagttcctctgaatatttgcagagactgaacaaggagtagcccaagcgattattcgttctgtgattgatttcaagagggatccatggcctaaagtttctgataatgcaaaggatcttgtaaagaaaatgcttgatccagatccaactcgacggctcacagctcatcaagttcttggtaatgtttgtggaatattgagatattgtactttattcattcgttgttttactctctctctctctctctatctatctatctctgataagtatttttttccggggctttgactcttgtggtgcagagcatccctggttacataatataaagaaagcaccaaacgtctcattgggtgagactgttaaagcaagactcaagcagttttcagtaatgaacaagctcaagaaaaaagctctgacggtaagcacacacttagtctgcaatcatatttataagctctggtttcttcactgtccactaaagatgaattcatatgcttttcctcatagatcgaaatgaaggagagaaggttgtgtcttaattatttactgcactgccttgtgctatttaataaaaacttaattctcatcgtaaaaaatgagaggcggttctcaaaattttgatcaagtttcgtttttttatcttgatatatgtactttcttgtattccaaacaggttatagctgagtttttgtctgcggaggaagtcgctggaatgaaggaagcatttgaaatgatggataccggaaagaagggcaagataaacctgaatgaacttaaagatggcttgcagaagcttggccatcaaatccctgatgctgatcttcatattctcatggaagcggtaagcggtctcatgccctgcttcttggctcgatcagatttcttatagctctaccgggggtaacataatatttgaaagttagctgctaaacttttctgcctcaaagagaaaacaggtgcctgagatgatatggccatgtcttacgtagaactgtaaattacatcaatggacattattttaaaatgaccgaaaactacatggaatccatgtgaacttagtaaagaaaatattcaatggaagtaaaggataccaagtagttggattaaggctagattgttggtggtacactgacattagtgtctcaatgtttactaagagtctcagtttgattagagatttgcacgtagatgcagggataaccgtgagattaagaaaattttaagaaattcacggagatgaaaaagatctgtaatactcatatagcttagggccaagcccaactagtttgggatcaaatcgtagttgttgttgataagaatttagcattagacttttgtctgtcaccctactgtcaaaaaattgattgattacaaaatatattttgtcaatataagttgtaacatttttctaccatttcaatgtagaaaaaaggaaaatctgtagcaaaattagcttgacatttcgcttgtcttagcatccctggttcaatgcttattattatccagaaaggaaaaaaaaacatttctcttgatccttttgcatcttcgacctgaaggatgcttatcttttttattattttatttccttgaacttttgttttatgtttttcttattctgtatcggttttacaggctgacgttgatggagatggaagtttaaattatccagagtttgttgctgtatctattcatcttagaaagatggccaatgatgaacacctgcacaaagcattttcatttttcgacaaaaatcagagtggtttcatagaaatcgaagagcttcgtagtgctttgagggatgaagacgacagcaacagcgaggaagtcaccaatgccattatgcatgacgttgatacagacaaggtcagtatgtccatttatgtgcacgtacaccatttagtaacttttcgttctttggttcatacttcatagtgcaaatattatgcatcgatgctaatgtttacatcttaatgagttctcattttgaagttcccttctgaaccctcgtttgagtttagagctcaaatactccacctagttgtgacttattgtatctctaaagtccgtcatgttatataaacgtattatactttgatggcatgcacactttctagcacatatgtgttgctaacgaaactctagtgctgtgacaaatgaaatacatgtatacattgatggcatctgttcttcccatcacatatgtactaccggtcattactctctagtgctgtgacattatgctctccctgttcgcttcatgatttacacggttggttaacctgctgctcgttacatgtctgctacagaattcaagttttgttagctgttttccatctcatctctaacaacatccccactcatttgtattagcttcttatctggagttttgtgagctcagtcttgtatcgtcttgtgtcaaaacgtgtgcaggatggtcggattagttatgaggaatttgctgcgatgatgaaggctggtacggactggagaaaagcatcgagacagtattctcgtgaacgttttaacagtctaagcttaaagttgatgagggaaggctcattacaagttgaaaacaaagtctag

SEQ ID NO: 99 - DNA, 5525 bp, Solanum lycopersicum
  source 1..5525: mol_type = genomic DNA
atgggtaattgctgtgtgaaaccgggtaaatctgccgaaaaaaagaataaaaagaacaacagcaaacctaaccctttttcaattgattatggggggactaaacatgcctctgggagtggaaacaagctagttgtattaaaagaaccaacagggcaaaatatacatgataagtatgatttggggcatgagctcggaagaggagaatttggggttacttatctatgtactgacttggaaggaggagaaaaatatgcttgcaaatcgatatctaaaaagaagctaaggactgcagtggatattgatgatgttaggagagaggttgagatcatgaaacatttgcctgtgcatccgaatattgtgaccttgaaggatacttatgaggatgataatgcagtgcacattgtgatggaattgtgtgagggtggggagttgtttgatcgaatcgttgctagaggccactatacagagagagcagctgctggaattttgaagactgtcgtggaagtcgttcaggtatagtttttatcaacttcttagttctcagttacctactgcttttattaccttttgcttaggttatcttattatatccattattttcagcatagcttcttcattactgtatttccttttcatattgtttttatatatgtcttacttaggctgagggtccattggaaatagcctctctaccttcacaaggtaggagtaaggctgcgtacacactacccttcccacaccccacttgtgggactatactaagtatgttgttgttttagttctcaattgatgctttttggtttttatgtagtaacttgtggtgtttcttttactgagttcttcaaagcttttgtatgggttttatatcatgacggatgtatcctgtattgttgtttcgggtttttattaaagaagtctggcaatttcaagttaaaaagaaaatcatatcttaaaagagaagcctaatcttgagcaaatcttgagcagatagcaatttcagggtgaaatgtgaatattcttggtgaagttgcatatgaactggtaaccattattcaattcatttctagtgttgatctttgcaatcaatggtttcattctagtgtacgttcatgctgtagcatttaccttgatatcctcatggaatttcctttactgccaaaattataatgagaagtggttatcttttttaataatggtaaagtatgagaagaggttttcttatgttctcagtctttgctagttctatttctttactcgttttacttaacttttttagtttcttgtgaactgtagtattgctctatatcttctcactcaaattcatgttctaaatcttaaccattctagtgatataaatgaagttaattggtgatataggatatccccctccaaaatctaacaatctttcaactcatcatagtcttgggcagatagctagttagaaccgtaacaaatatttaggaaagtagatcattcgaaatagttatccttgtgaaatattattctttatcttcattattgaccattggttttcaaactctagtactcttaagtggaagactcacttcttgtttctgtggagtattagctatagcggcctacaacagaatttgattgttgcactcaaagttaaacagagttctacagtttagggaaatgataatggaatttaaatttagtttgtatactgaagtaaatatggttgacactatcagaaacaagtgctttttacttcaaatattgatctttatcctcattgcgaaccattgatgtccaaactgttttagatggaagagcaatttgttgttcatttgagtggaatagtcaccaacaacagctaattaactacgtatagcttagagagatgcgaaccaatggtaaatttaagttgtctcctgaagtagttactgattgttcatgataaaggtcattaaagttgaattctctatttagtcagtgtccttttctgcatcgactatatagtggcctgaatgacattacaaaatatttatgagttggtaggaatctttttttcatatgtgaatcatgaatgtgttcacaaatgatcaatcagagagtgattattgtattatgtggtgttgataacttttgaacttttcttcatttggtttgtgtttaactgttatctgaaaggcttggttggtggtactaaagctattggattagcagaaaactttatacatgtttatggtcatgtttcgctctccagtccccgtttttatttgtcaaaggtcagttcatatatttccaatggttttgcagatgtgtcacaggcaaggggtaatgcatcgtgatctcaaacctgagaattttctttttggtaacaagaaagaaacagctccactgaaggctattgactttgggttgtctgttttctttaaacctggtaatggaattggaaaaaaaacagtgagtttaagacttttatcatgctaaacaaaggtttaacatgttgattattttaacaggggaacgctttaatgagatagtgggaagtccttattacatggctcctgaggtcctaaagcgcaattatggaccagaggtcgatgtctggagtgctggagttatactttacattcttctatgcggtgttccacctttctgggcaggtctgcttattttatttcttcgttttttataaccatggaacgaacctcaatgcagatattttcatgtgcaatttttggaacttgataattgattaactaagattgtgaatatgaagtagaacttgattcatgttagaatatgttgttgaaatattagatgatgaggcaagtgaggtgaaagactgtccctgctttaatcaatgtagatcatgttcaattattttggtttctcttaatggttcttatgggttggactttgctaaataacttgcataaatatgttaacatattcttgatacttcccttaagttcctctgaatatttgcagagactgaacaaggagtagcccaagcgattattcgttctgtgattgatttcaagagggatccatggcctaaagtttctgataatgcaaaggatcttgtaaagaaaatgcttgatccagatccaactcgacggctcacagctcatcaagttcttggtaatgtttgtggaatattgagatattgtactttattcattcgttgttttactctctctctctctctctctctctctctatctatctctgataagtatttttttccggggctttgactcttgtggtgcagagcatccctggttacataatataaagaaagcaccaaacgtctcattgggtgagactgttaaagcaagactcaagcagttttcagtaatgaacaagctcaagaaaaaagctctgacggtaagcacacacttagtctgcaatcatatttataagctctggattcttcactgtccactaaagatgaattcatatgcttttcctcatagatcgaaatgaaggagagaaggttgtgtcttaattatttactgcactgccttgtgctatttaataaaaacttaattctcatcgtaaaaaatgagaggcggttctcaaaattttgatcaagtttcgtttttttatcttgatatatgtactttcttgtattccaaacaggttatagctgagtttttgtctgcggaggaagtcgctggaatgaaggaagcatttgaaatgatggataccggaaagaagggcaagataaacctgaatgaacttaaagatggcttgcagaagcttggccatcaaatccctgatgctgatcttcatattctcatggaagcggtaagcggtctcatgccctgcttcttggctcgatcagatttcttatagctctaccgggggtaacataatatttgaaagttagctgctaaacttttctgcctcaaagagaaaacaggtgcctgagatgatatggccatgtcttacgtagaactgtaaattacatcaatggacattattttaaaatgaccgaaaactacatggaatccatgtgaacttagtaaagaaaatattcaatggaagtaaaggataccaagtagttggattaaggctagattgttggtggtacactgacattagtgtctcaatgtttactaagagtctcagtttgattagagatttgcacgtagatgcagggataaccgtgagattaagaaaattttaagaaattcacggagatgaaaaagatctgtaatactcatatagcttagggccaagcccaactagtttgggatcaaatcgtagttgttgttgataagaatttagcattagacttttgtctgtcaccctactgtcaaaaaattgattgattacaaaatatattttgtcaatataagttgtaacatttttctaccatttcaatgtagaaaaaaggaaaatctgtagcaaaattagcttgacatttcgcttgtcttagcatccctggttcaatgcttattattatccagaaaggaaaaaaaaacatttctcttgatccttttgcatcttcgacctgaaggatgcttatcttttttattattttatttccttgaacttttgttttatgtttttcttattctgtatcggttttacaggctgacgttgatggagatggaagtttaaattatccagagtttgttgctgtatctattcatcttagaaagatggccaatgatgaacacctgcacaaagcattttcatttttcgacaaaaatcagagtggtttcatagaaatcgaagagcttcgtagtgctttgagggatgaagacgacagcaacagcgaggaagtcaccaatgccattatgcatgacgttgatacagacaaggtcagtatgtccatttatgtgcacgtacaccatttagtaacttttcgttctttggttcatacttcatagtgcaaatattatgcattgttgctaatgtttacatcttaatgagttctcattttgaagttctcttctgaaccctcgtttgagtttagagctcaaatactccacctagttgtgacttattgtatctctaaagtccgtcatattatataaacgtattatactttgatggcatgcacactttctagcacatatgtgttgctaacgaaactctagtgctgtgacaaatgaaatacatgtatacattgatggcatctgttcttcccatcacatatgtactaccggtcattactctctagtgctgtgacattatgctctccctgttcgcttcatgagttacacggttggttaacctgctgctcgttacatgtctgctacagaattcaagttttgttagctgttttccatctcatctctaacaacatccccactcatttgtattagcttcttatctggagttttgtgagctcagtcttgtatcgtcttgtgtcaaaacgtgtgcaggatggtcggattagttatgaggaatttgctgcgatgatgaaggctggtacggactggagaaaagcatcgagacagtattctcgtgaacgttttaacagtctaagcttaaagttgatgagggaaggctcattacaagttgaaaacaaagtctag

SEQ ID NO: 100 - DNA, 5517 bp, Solanum lycopersicum; identical to SEQ ID NO: 98
  source 1..5517: mol_type = genomic DNA

SEQ ID NO: 101 - DNA, 5516 bp, Solanum lycopersicum
  source 1..5516: mol_type = genomic DNA
atgggtaattgctgtgtgaaaccgggtaaatctgccgaaaaaaagaataaaaagaacaacagcaaacctaaccctttttcaattgattatggggggactaaacatgcctctgggagtggaaacaagctagttgtattaaaagaaccaacagggcaaaatatacatgataagtatgatttggggcgtgagctcggaagaggagaatttggggttacttatctatgtactgacttggaaggaggagaaaaatatgcttgcaaatcgatatctaaaaagaagctaaggactgcagtggatattgatgatgttaggagagaggttgagatcatgaaacatttgcctgtgcatccgaatattgtgaccttgaaggatacttatgaggatgataatgcagtgcacattgtgatggaattgtgtgagggtggggagttgtttgatcgaatcgttgctagaggccactatacagagagagcagctgctggaattttgaagactgtcgtggaagtcgttcaggtatagtttttatcagcttcttagttctcagttacctactgcttttattaccttttgcttaggttatcttattatatccattattttcagcatagcttcttcattactgtatttccttttcatattgtttttatatatgtcttacttaggctgagggtccattggaaatagcctctctaccttcacaaggtaggagtaaggctgcgtacacactacccttcccacaccccacttgtgggactatactaagtatgttgttgttttagttctcaattgatgctttttggtttttatgtagtaacttgtggtgtttcttttactgagttcttcaaagcttttgtatgggttttatatcatgacggatgtatcctgtattgttgtttcgggtttttattaaagaagtctggcaatttcaagttaaaaagaaaatcatatcttaaaagagaagcctaatcttgagcaaatcttgagcagatagcaatttcagggtgaaatgtgaatattcttggtgaagttgcatatgaactggtaaccattattcaattcatttctagtgttgatctttgcaatcaatggtttcattctagtgtacgttcatgctgtagcatttaccttgatatcctcatggaatttcctttaccgccaaaattataatgagaagtggttatcttttttaataatggtaaagtatgagaagaggttttcttatgttctcagtctttgctagttctatttctttactcgttttacttaacttttttagtttcttgtgaactgtagtattgctctatatcttctcactcaaattcatgttctaaatcttaaccattctagtgatataaatgaagttaattggtgatataggatatccccctccaaaatctaacaatctttcaactcatcatagtcttgggcagatagctagttagaaccgtaacaaatatttaggaaagtagatcattcgaaatagttatccttgtgaaatattattctttatcttcattattgaccattggttttcaaactctagtactcttaagtggaagattcacttcttgtttctgtggagtattaactatagcggcctacaacagaatttgattgttgcactcaaagttaaacagagttctacagtttagggaaatgataatggaatttaaatttagtttgtatactgaagtaaatatggttgacactatcagaaacaagtgctttttacttcaaatattgatctttatcctcattgcgaaccattgatgtccaaactgttttagatggaagagcaatttgttgttcatttgagtggaatagtcaccaacaacagctaattaactacgtatagcttagagagatgcgaaccaatggtaaatttaagttgtctcctgaagtagttactgattgttcatgataaaggtcattaaagttgaattctctatttagtcagtgtccttttctgcatcgactatatagtggcctgaatgacattacaaaatatttatgagttggtaggaatctttttttcatatgtgaatcatgaatgtgttcacaaatgatcaatcagagagtgattattgtattatgtggtgttgataacttttgaacttttcttcatttggtttgtgtttaactgttatctgaaaggcttggttggtggtactaaagctattggattagcagaaaactttatacatgtttatggtcatgtttcgctctccagtccccgtttttatttgtcaaaggtcagttcatatatttccaatggttttgcagatgtgtcacaggcaaggggtaatgcatcgtgatctcaaacctgagaattttctttttggtaacaagaaagaaacagctccactgaaggctattgactttgggttgtctgttttctttaaacctggtaatggaattggaaaaaaaacagtgagtttaagacttttatcatgctaaacaaaggtttaacatgttgattattttaacaggggaacgctttaatgagatagtgggaagtccttattacatggctcctgaggtcctaaagcgcaattatggaccagaggtcgatgtctggagtgctggagttatactttacattcttctatgcggtgttccacctttctgggcaggtctgcttattttatttcttcgttttttataaccatggaacgaacctcaatgcagatattttcatgtgcaatttttggaacttgataattgattaactaagattgtgaatatgaagtagaacttgattcatgttagaatatgtcgttgaaatattagatgatgaggcaagtgaggtgaaagactgtccctgctttaatcaatgtagatcatgttcaattattttggtttctcttaatggttcttatgggttggactttgctaaataacttgcataaatatgttaacatattcttgatacttcccttaagttcctctgaatatttgcagagactgaacaaggagtagcccaagcgattattcgttctgtgattgatttcaagagggatccatggcctaaagtttctgataatgcaaaggatcttgtaaagaaaatgcttgatccagatccaactcgacggctcacagctcatcaagttcttggtaatgtttgtggaatattgagatattgtactttattcattcgttgttttactctctctctctctctctatctatctctgataagtatttttttccggggctttgactcttgtggtgcagagcatccctggttacataatataaagaaagcaccaaatgtctcattgggtgagactgttaaagcaagactcaagcagttttcagtaatgaacaagctcaagaaaaaagctctgacggtaagcacacacttagtctgcaatcatatttataagctctggattcttcactgtccactaaagatgaattcatatgcttttcctcatagatcgaaatgaaggagagaagattgtgtcttaattatttactgcactgccttgtgctatttaataaaaacttaattctcatcgtaaaaaatgagaggaggttctcaaaattttgatcaagtttcgtttttttatcttgatatatgtactttcttgtattccaaacaggttatagctgagtttttgtctgcggaggaagtcgctggaatgaaggaagcatttgaaatgatggataccggaaagaagggtaagataaacctgaatgaacttaaagatggcttgcagaagcttggccatcaaatccctgatgctgatcttcatattctcatggaagcggtaagcggtctcatgccctgcttcttggctcgatcagatttcttatagctctaccgggggtaacataatatttgaaagttagctgctaaacttttctgcctcaaagagaaaacaggtgcctgagatgatatggccatgtcttacgtagaactgtaaattacatcaatggacattattttaaaatgaccgaaaactacatggaatccatgtgaacttagtaaagaaaatattcaatggaagtaaaggataccaagtagttggattaaggctagattgttggtggtacactgacattagtgtctcaatgtttactaagagtctcagtttgattagagatttgcacgtagatgcagggataaccgtgagattaagaaaattttaagaaattcacggagatgaaaaagatctgtaatactcatatagcttagggccaagcccaactagtttgggatcaaatcgtagttgttgttgataagaatttagcattagacttttgtctgtcaccctactgtcaaaaaattgattgattacaaaatatattttgtcaatataagttgtaacatttttctaccatttcaatgtagaaaaaaggaaaatctgtagcaaaattagcttgacatttcgcttgtcttagcatccctggttcaatgcttattattatccagaaaggaaaaaaaaaacatttctcttgatccttttgcatcttcgacctgaaggatgcttatcttttttattattttatttccttgaacttttgttttatgtttttcttattctgtatcggttttacaggctgacgttgatggagatggaagtttaaattatccagagtttgttgctgtatctattcatcttagaaagatggccaatgatgaacacctgcacaaagcattttcatttttcgacaaaaatcagagtggtttcatagaaatcgaagagcttcgtagtgctttgagggatgaagacgacagcaacagcgaggaagtcaccaatgccattatgcatgacgttgatacagacaaggtcagtatgtccatttatgtgcacgtacaccatttagtaacttttcgttctttggttcatacttcatagtgcaaatattatgcattgttgctaatgtttacatcttaatgagttctcattttgaagttctcttctgaaccctcgtttgagtttagagctcaaatactccacctagttgtgacttattgtatctctaaagtccgtcatattatataaacgtattatactttgatggcatgcacactttctagcacatatgtgttgctaacgaaactctagtgctgtgacaaatgaaatacatgtatacattgatggcatctgttcttcccatcacatatgtactaccggtcattactctctagtgctgtgacattatgctctccctgttcgcttcatgagttacacggttggttaacctgctgctcgttacatgtctgctacagaattcaagttttgttagctgttttccatctcatctctaacaacatccccactcatttgtattagcttcttatctggagttttgtgagctcagtcttgtatcgtcttgtgtcaaaacgtgtgcaggatggtcggattagttatgaggaatttgctgcgatgatgaaggctggtacggactggagaaaagcatcgagacagtattctcgtgaacgttttaacagtctaagcttaaagttgatgagggaaggctcattacaagttgaaaacaaagtctag

SEQ ID NO: 102 - DNA, 5501 bp, Solanum lycopersicum
  source 1..5501: mol_type = genomic DNA
atgggtaattgctgtgtgaaaccgggtaaatctgccgaaaaaaagaataaaaagaacaacagcaaacctaaccctttttcaattgattatggggggactaaacatgcctctgggagtggaaacaagctagttgtattaaaagaaccaacagggcaaaatatacatgataagtatgatttggggcgtgagctcggaagaggagaatttggggttacttatctatgtactgacttggaaggaggagaaaaatatgcttgcaaatcgatatctaaaaagaagctaaggactgcagtggatattgatgatgttaggagagaggttgagatcatgaaacatttgcctgtgcatccgaatattgtgaccttgaaggatacttatgaggatgataatgcagtgcacattgtgatggaattgtgtgagggtggggagttgtttgatcgaatcgttgctagaggccactatacagagagggcagctgctggaattttgaagactgtcgtggaagttgttcaggtatagtttttatcagcttcttagttcacagttactactgtttttattaccttttgcttaggttatcttattatatccattattttcagcatagcttcttcattactgtatttccttttcatattgtttttatatatgtcttacttaggctgagggtccattggaaatagcctctctaccttcacaaggtaggagtaaggctgcgtacacactacccttcccacaccccacttgtgggactatactaagtatgttgttgttttagttcacaattgatgctttttgttttttatgtagtaacttgtggtgtttcttttactgagttcttcaaagcttttgtatgggttttatatcatgacggatgtatcctgtattgttgtttcgggtttttattaaagaagtctggcaatttcaagttaaaaagaaaatcatatcttaaaagagaagcctaatcttgagcagatagcaatttcagggtgaaatgtgaatattcttggtgaagttgcatatgaactggctaaccattattcaattcatttctagtgttgatctttgcaatcaatggtttcattctagtgtacgttcatgctgtagcatttaccttgatatcctcatggaatttcctttaccgccaaaattataatgagaagtggttatcttttttaataatggtaaagtatgagaagaggttttcttatgttctcagtctttgctagttctatttctttactcgttttacttaacttttttagtttcttgtgaactgtagtattgctctatatcttctcactcaaattcatgttctaaatcttaaccattctagtgatataaatgaagttaattggtgatataggatatccccctccaaaatctaacaatctttcaactcatcatagtcttgggcagatagctagttagaaccgtaacaaatatttaggaaagtagatcattcgaaatagttatccttgtgaaatattattctttatcttcattattgaccattggttttcaaactctagtactcttaagtggaagactcacttcttgtttctgtggagtattagctatagcggcctacaacagaatttgattgttgcactcaaagttaaacagagttctacagtttagggaaatgataatggaatttaaatttagtttgtatactgaagtaaatatggttgacactatcagaaacaagtgctttttacttcaaatattgatctttatcctcattgcgaaccattgatgtccaaactgttttagatggaagagcaatttgttgttcatttgagtggaatagtcaccaacaacagctaattaactacgtatagcttagagagatgcgaaccaatggtaaatttaagttgtctcctgaagtagttactgattgttcacgataaaggtcattaaagttgaattctctatttagtcagcgtccttttctgcatcgactatatagtggcctgaatgacattacaaaatatttatgagttggtaggaatctttttttcatatgtgaatcatgaatgtgttcacaaatgatcaatcagagagtgattattgtattatgtggtgttgataacttttgaacttttcttcatttggtttgtgtttaactgttatctgaaaggcttggttggtggtactaaagctattggattagcagaaaactttatacatgtttatggtcatgtttcgctctccagtctccgtttttatttgtcaaaggtcagttcatatatttccaatggttttgcagatgtgtcacaggcaaggggtaatgcatcgtgatctcaaacctgagaattttctttttggtaacaagaaagaaacagctccactgaaggctattgactttgggttgtctgttttctttaaacctggtaatggaattggaaaaaaaacagtgagtttaagacttttatcatgctaaacaaaggtttaacattttgattattttaacaggggaacgctttaatgagatagtgggaagtccttattacatggctcctgaggtcctaaagcgcaattatggaccagaggtcgatgtctggagtgctggagttatactttacattcttctatgcggtgttccacctttctgggcaggtctgcttattttatttcttcgttttttataaccatggaacgaacctcaatgcagatattttcatgtgcaatttttggaacttgataattgattaactaagattgtgaatatgaagtagaacttgattcatgttagaatatgtcgttgaaatattagatgatgaggcaagtgaggtgaaagactgtccctgctttaatcaatgtagatcatgttcaattattttggtttctcttaatggttcttatgggttggactttgctaaataacttgcataaatatgttaacatattcttgatacttcccttaagttcctctgaatatttgcagagactgaacaaggagtagcccaagcgattattcgttctgtgattgatttcaagagggatccatggcctaaagtttctgataatgcaaaggatcttgtaaagaaaatgcttgatccagatccaactcgacggctcacagctcatcaagttcttggtaatgtttgtggaatattgagatattgtacttcattcattcgttgttttactctctctctctctctctctatctatgataagtatttttttccggggctttgactcttgtggtgcagagcatccctggttacataatataaagaaagcaccaaacgtctcattgggtgagactgttaaagcaagactcaagcagttttcagtaatgaacaagctcaagaaaaaagctctgacggtaagcacacacttagtctgcaatcatatttataagctctggattcttcactgtccactaaagatgaattcatatgcttttcctcatagattgaaatgaaggagagaaggttgtgtcttaattatttactgcactgccttgtgctatttaataaaaacttaattctcatcgtaaaaaatgagagacggttctcaaaattttgatcaggtttcgtttttttatcttgatatatgtactttcttgtattccaaacaggttatagctgagtttttgtctgcggaggaagtcgctggaatgaaggaagcatttgaaatgatggataccggaaagaagggcaagataaacctgaatgaacttaaagatggcttgcagaagcttggccatcaaatccctgatgctgatcttcagattctcatggaagcggtaagcggtctcatgccctgcttcttggctcgatcagatttcttatagctctaccgggggtaacataatatttgaaagttagctgctaaacttttctgcctcaaagagaaaacaggtgcctgagatgatatggccatgtcttacgtagaactgtaaattacatcaatggacattattttaaaatgaccgaaaactacatggaatccatgtgaacttagtaaagaaaatactcaatggaaggaagtaaaggataccaagtagttggattaaggctagattgttggtggtacactgacattagtgactcaatgtttactaagactctcagtttgattagagatttgcacgtagatgcagggataaccgtgagattaagaaaattttaagaaattcgcggagatgaaatagatctgtaatactcatatagcttagggccaagcccaactagtttgggatcaaatcgtagttgttgttgatgagaatttagcattagacttttgtctgtcaccctactgtcaaaaaattgattgattacaaaatatattttgtcaatataagttgtaacatttttctaccatttcaatgtagaaaaaaggaaaatgtagcaaaattagcttgacatttcgcttgtcttagcatccctggttcaatgcttattattatccagaaaggaaaaaaaaaacatttctcttgatccttttgcatcttcgacctgaaggatgcttatcttttttattattttatttccttgaacttttgttttatgtttttcttattctgtatcggttttacaggctgacgttgatggagatggaagtttaaattatccagagtttgttgctgtatctattcatcttagaaagatggccaatgatgaacacctgcacaaagcattttcattttttgacaaaaaccaaagtggtttcatagaaatcgaagagcttcgtagtgctttgagggatgaagacgacagcaacagcaaggaagtcaccgatgccattatgcatgacgttgatacagacaaggtcagtatgtccatttatgtgcacgtacaccatttagtaacttttcgttctttggttcatacttcatagtgcaaatattatgcatcgatgctaatgtttacatcttaatgagttctcattttgaagttcccttctgaaccctcgtttgagtttagagctcaaatactccacctagttgtgacttattgtatctctaaagtccgtcatgttatataaattatactttgatggcatgcacactttctagcacatatgtgttgctaacgaaactctagtgctgtgacaaatgaaatacatgtatacattgatggcatctgttcttcccatcacatatgtactaccggtcattactctctagtgctgtgacattatgctctccctgttcgcttcatgatttacacggttggttaacctgctgctcgttacatgtctgctacagaattcaagttttgttagctgttttccatctcatctctaacaacatccccactcatttgtattagcttcttatctggagttttgtgagctcagtcttgtatcgtcttgtgtcaaaacgtgtgcaggatggtcggattagttatgaggaatttgctgcgatgatgaaggctggtacggactggagaaaagcatcgagacagtattctcgtgaacgttttaacagtctaagcttaaagttgatgagggaaggctcattacaagttgaaaacaaagtctag

SEQ ID NO: 103 - DNA, 5526 bp, Solanum lycopersicum; identical to SEQ ID NO: 11
  source 1..5526: mol_type = genomic DNA

SEQ ID NO: 104 - DNA, 5517 bp, Solanum lycopersicum; identical to SEQ ID NO: 98
  source 1..5517: mol_type = genomic DNA

SEQ ID NO: 105 - DNA, 5501 bp, Solanum lycopersicum; identical to SEQ ID NO: 102
  source 1..5501: mol_type = genomic DNA

SEQ ID NO: 106 - DNA, 5517 bp, Solanum lycopersicum
  source 1..5517: mol_type = genomic DNA
atgggtaattgctgtgtgaaaccgggtaaatctgccgaaaaaaagaataaaaagaacaacagcaaacctaaccctttttcaattgattatggggggactaaacatgcctctgggagtggaaacaagctagttgtattaaaagaaccaacagggcaaaatatacatgataagtatgatttggggcgtgagctcggaagaggagaatttggggttacttatctatgtactgacttggaaggaggagaaaaatatgcttgcaaatcgatatctaaaaagaagctaaggactgcagtggatattgatgatgttaggagagaggttgagatcatgaaacatttgcctgtgcatccgaatattgtgaccttgaaggatacttatgaggatgataatgcagtgcacattgtgatggaattgtgtgagggtggggagttgtttgatcgaatcgttgctagaggccactatacagagagagcagctgctggaattttgaagactgtcgtggaagtcgttcaggtatagtttttatcagcttcttagttctcagttacctactgcttttattaccttttgcttaggttatcttattatatccattattttcagcatagcttcttcattactgtatttccttttcatattgtttttatatatgtcttacttaggctgagggtccattggaaatagcctctctaccttcacaaggtaggagtaaggctgcgtacacactacccttcccacaccccacttgtgggactatactaagtatgttgttgttttagttcacaattgatgctttttggtttttatgtagtaacttctggtgtttcttttactgagttcttcaaagcttttgtatgggttttatatcatgacggatgtatcctgtattgttgtttcgggtttttattaaagaagtctggcaatttcaagttaaaaagaaaatcatatcttaaaagagaagcctaatcttgagcagatagcaatttcagggtgaaatgtgaatattcttggtgaagttgcatatgaacatatgaactggctaaccattattcaattcatttctagtgttgatctttgcaatcaatggtttcattctagtgtacgttcatgctgtagcatttaccttgatatcctcatggaatttcctttaccgccaaaattataatgagaagtggttatcttttttaataatggtaaagtatgagaagaggttttcttatgttctcagtctttgctagttctatttctttactcgttttacttaacttttttagtttcttgtgaactgtagtattgctctatatcttctcactcaaattcatgttctaaatcttaaccattctagtgatataaatgaagttaattggtgatataggatatccccctccaaaatctaacaatctttcaactcatcatagtcttgggcagatagctagttagaaccgtaacaaatatttaggaaagtagatcattcgaaatagttatccttgtgaaatattattctttatcttcattattgaccattggttttcaaactctagtactcttaagtggaagactcacttcttgtttctgtggagtattagctatagcggcctacaacagaatttgattgttgcactcaaagttaaacagagttctacagtttagggaaatgataatggaatttaaatttagtttgtatactgaagtaaatatggttgacactatcagaaacaagtgctttttacttcaaatattgatctttatcctcattgcgaaccattgatgtccaaactgttttagatggaagagcaatttgttgttcatttgagtggaatagtcaccaacaacagctaattaactacgtatagcttagagagatgcgaaccaatggtaaatttaagttgtctcctgaagtagttactgattgttcatgataaaggtcattaaagttgaattctctatttagtcagcgtccttttctgcatcgactatatagtggcctgaatgacattacaaaatatttatgagttggtaggaatctttttttcatatgtgaatcatgaatgtgttcacaaatgatcaatcagagagtgattattgtattatgtggtgttgataacttttgaacttttcttcatttggtttgtgtttaactgttatctgaaaggcttggttggtggtactaaagctattggattagcagaaaactttatacatgtttatggtcatgtttcgctctccagtctccgtttttatttgtcaaaggtcagttcatatatttccaatggttttgcagatgtgtcacaggcaaggggtaatgcatcgtgatctcaaacctgagaattttctttttggtaacaagaaagaaacagctccactgaaggctattgactttgggttgtctgttttctttaaacctggtaatggaattggaaaagaaacagtgagtttaagacttttatcatgctaaacaaaggtttaacattttgattattttaacaggggaacgctttaatgagatagtgggaagtccttattacatggctcctgaggtcctaaagcgcaattatggaccagaggtcgatgtctggagtgctggagttatactttacattcttctatgcggtgttccacctttctgggcaggtctgcttattttatttcttcgttttttataaccatggaacgaacctcaatgcagatattttcatgtgcaatttttggaacttgataattgattaactaagattgtgaatatgaagtagaacttgattcatgttagaatatgtcgttgaaatattagatgatgaggcaagtgaggtgaaagactgtccctgctttaatcaatgtagatcatgttcaattattttggtttctcttaatggttcttatgggttggactttgctaaataacttgcataaatatgttaacatattcttgatacttcccttaagttcctctgaatatttgcagagactgaacaaggagtagcccaagcgattattcgttctgtgattgatttcaagagggatccatggcctaaagtttctgataatgcaaaggatcttgtaaagaaaatgcttgatccagatccaactcgacggctcacagctcatcaagttcttggtaatgtttgtggaatattgagatattgtactttattcattcgttgttttactctctctctctctctctatctatctatctctgataagtatttttctccggggctttgactcttgtggtgcagagcatccctggttacataatataaagaaagcaccaaacgtctcattgggtgagactgttaaagcaagactcaagcagttttcagtaatgaacaagctcaagaaaaaagctctgacggtaagcacacacttagtctgcaatcatatttataagctctggtttcttcactgtccactaaagatgaattcatatgcttttcctcatagatcgaaatgaaggagagaaggttgtgtcttaattatttactgcactgccttgtgctatttaataaaaacttaattctcatcgtaaaaaatgagaggcggttctcaaaattttgatcaagtttcgtttttttatcttgatatatgtactttcttgtattccaaacaggttatagctgagtttttgtctgcggaggaagtcgctggaatgaaggaagcatttgaaatgatggataccggaaagaagggcaagataaacctgaatgaacttaaagatggcttgcagaagcttggccatcaaatccctgatgctgatcttcatattctcatggaagcggtaagcggtctcatgccctgcttcttggctcgatcagatttcttatagctctaccgggggtaacataatatttgaaagttagctgctaaacttttctgcctcaaagagaaaacaggtgcctgagatgatatggccatgtcttacgtagaactgtaaattacatcaatggacattattttaaaatgaccgaaaactacatggaatccatgtgaacttagtaaagaaaatattcaatggaagtaaaggataccaagtagttggattaaggctagattgttggtggtacactgacattagtgtctcaatgtttactaagagtctcagtttgattagagatttgcacgtagatgcagggataaccgtgagattaagaaaattttaagaaattcacggagatgaaaaagatctgtaatactcatatagcttagggccaagcccaactagtttgggatcaaatcgtagttgttgttgataagaatttagcattagacttttgtctgtcaccctactgtcaaaaaattgattgattacaaaatatattttgtcaatataagttgtaacatttttctaccatttcaatgtagaaaaaaggaaaatctgtagcaaaattagcttgacatttcgcttgtcttagcatccctggttcaatgcttattattatccagaaaggaaaaaaaaacatttctcttgatccttttgcatcttcgacctgaaggatgcttatcttttttattattttatttccttgaacttttgttttatgtttttcttattctgtatcggttttacaggctgacgttgatggagatggaagtttaaattatccagagtttgttgctgtatctattcatcttagaaagatggccaatgatgaacacctgcacaaagcattttcatttttcgacaaaaatcagagtggtttcatagaaatcgaagagcttcgtagtgctttgagggatgaagacgacagcaacagcgaggaagtcaccaatgccattatgcatgacgttgatacagacaaggtcagtatgtccatttatgtgcacgtacaccatttagtaacttttcgttctttggttcatacttcatagtgcaaatattatgcatcgatgctaatgtttacatcttaatgagttctcattttgaagttcccttctgaaccctcgtttgagtttagagctcaaatactccacctagttgtgacttattgtatctctaaagtccgtcatgttatataaacgtattatactttgatggcatgcacactttctagcacatatgtgttgctaacgaaactctagtgctgtgacaaatgaaatacatgtatacattgatggcatctgttcttcccatcacatatgtactaccggtcattactctctagtgctgtgacattatgctctccctgttcgcttcatgatttacacggttggttaacctgctgctcgttacatgtctgctacagaattcaagttttgttagctgttttccatctcatctctaacaacatccccactcatttgtattagcttcttatctggagttttgtgagctcagtcttgtatcgtcttgtgtcaaaacgtgtgcaggatggtcggattagttatgaggaatttgctgcgatgatgaaggctggtacggactggagaaaagcatcgagacagtattctcgtgaacgttttaacagtctaagcttaaagttgatgagggaaggctcattacaagttgaaaacaaagtctag

SEQ ID NO: 107 - DNA, 5517 bp, Solanum lycopersicum; identical to SEQ ID NO: 106
  source 1..5517: mol_type = genomic DNA

SEQ ID NO: 108 - DNA, 5501 bp, Solanum lycopersicum; identical to SEQ ID NO: 102
  source 1..5501: mol_type = genomic DNA

SEQ ID NO: 109 - DNA, 1602 bp, Solanum lycopersicum; identical to SEQ ID NO: 9
  source 1..1602: mol_type = other DNA

SEQ ID NO: 110 - DNA, 1644 bp, Solanum lycopersicum
  source 1..1644: mol_type = other DNA
atgggtaattgctgtgtgaaaccgggtaaatctgccgaaaaaaagaataaaaagaacaacagcaaacctaaccctttttcaattgattatggggggactaaacatgcctctgggagtggaaacaagctagttgtattaaaagaaccaacagggcaaaatatacatgataagtatgatttggggcgtgagctcggaagaggagaatttggggttacttatctatgtactgacttggaaggaggagaaaaatatgcttgcaaatcgatatctaaaaagaagctaaggactgcagtggatattgatgatgttaggagagaggttgagatcatgaaacatttgcctgtgcatccgaatattgtgaccttgaaggatacttatgaggatgataatgcagtgcacattgtgatggaattgtgtgagggtggggagttgtttgatcgaatcgttgctagaggccactatacagagagagcagctgctggaattttgaagactgtcgtggaagtcgttcagatgtgtcacaggcaaggggtaatgcatcgtgatctcaaacctgagaattttctttttggtaacaagaaagaaacagctccactgaaggctattgactttgggttgtctgttttctttaaacctggggaacgctttaatgagatagtgggaagtccttattacatggctcctgaggtcctaaagcgcaattatggaccagaggtcgatgtctggagtgctggagttatactttacattcttctatgcggtgttccacctttctgggcagagactgaacaaggagtagcccaagcgattattcgttctgtgattgatttcaagagggatccatggcctaaagtttctgataatgcaaaggatcttgtaaagaaaatgcttgatccagatccaactcgacggctcacagctcatcaagttcttggtaatgtttgtggaatattgagatattgtactttattcattcagcatccctggttacataatataaagaaagcaccaaatgtctcattgggtgagactgttaaagcaagactcaagcagttttcagtaatgaacaagctcaagaaaaaagctctgacggttatagctgagtttttgtctgcggaggaagtcgctggaatgaaggaagcatttgaaatgatggataccggaaagaagggtaagataaacctgaatgaacttaaagatggcttgcagaagcttggccatcaaatccctgatgctgatcttcatattctcatggaagcggctgacgttgatggagatggaagtttaaattatccagagtttgttgctgtatctattcatcttagaaagatggccaatgatgaacacctgcacaaagcattttcatttttcgacaaaaatcagagtggtttcatagaaatcgaagagcttcgtagtgctttgagggatgaagacgacagcaacagcgaggaagtcaccaatgccattatgcatgacgttgatacagacaaggatggtcggattagttatgaggaatttgctgcgatgatgaaggctggtacggactggagaaaagcatcgagacagtattctcgtgaacgttttaacagtctaagcttaaagttgatgagggaaggctcattacaagttgaaaacaaagtctag

SEQ ID NO: 111 - DNA, 1602 bp, Solanum lycopersicum; identical to SEQ ID NO: 9
  source 1..1602: mol_type = other DNA

SEQ ID NO: 112 - DNA, 1602 bp, Solanum lycopersicum; identical to SEQ ID NO: 9
  source 1..1602: mol_type = other DNA

SEQ ID NO: 113 - DNA, 1602 bp, Solanum lycopersicum; identical to SEQ ID NO: 9
  source 1..1602: mol_type = other DNA

SEQ ID NO: 114 - DNA, 1602 bp, Solanum lycopersicum; identical to SEQ ID NO: 9
  source 1..1602: mol_type = other DNA

SEQ ID NO: 115 - DNA, 1602 bp, Solanum lycopersicum; identical to SEQ ID NO: 9
  source 1..1602: mol_type = other DNA

SEQ ID NO: 116 - DNA, 1602 bp, Solanum lycopersicum; identical to SEQ ID NO: 9
  source 1..1602: mol_type = other DNA

SEQ ID NO: 117 - DNA, 1602 bp, Solanum lycopersicum; identical to SEQ ID NO: 9
  source 1..1602: mol_type = other DNA

SEQ ID NO: 118 - DNA, 1635 bp, Solanum lycopersicum
  source 1..1635: mol_type = other DNA
atgggtaattgctgtgtgaaaccgggtaaatctgccgaaaaaaagaataaaaagaacaacagcaaacctaaccctttttcaattgattatggggggactaaacatgcctctgggagtggaaacaagctagttgtattaaaagaaccaacagggcaaaatatacatgataagtatgatttggggcgtgagctcggaagaggagaatttggggttacttatctatgtactgacttggaaggaggagaaaaatatgcttgcaaatcgatatctaaaaagaagctaaggactgcagtggatattgatgatgttaggagagaggttgagatcatgaaacatttgcctgtgcatccgaatattgtgaccttgaaggatacttatgaggatgataatgcagtgcacattgtgatggaattgtgtgagggtggggagttgtttgatcgaatcgttgctagaggccactatacagagagagcagctgctggaattttgaagactgtcgtggaaatgtgtcacaggcaaggggtaatgcatcgtgatctcaaacctgagaattttctttttggtaacaagaaagaaacagctccactgaaggctattgactttgggttgtctgttttctttaaacctggggaacgctttaatgagatagtgggaagtccttattacatggctcctgaggtcctaaagcgcaattatggaccagaggtcgatgtctggagtgctggagttatactttacattcttctatgcggtgttccacctttctgggcagagactgaacaaggagtagcccaagcgattattcgttctgtgattgatttcaagagggatccatggcctaaagtttctgataatgcaaaggatcttgtaaagaaaatgcttgatccagatccaactcgacggctcacagctcatcaagttcttggtaatgtttgtggaatattgagatattgtactttattcattcagcatccctggttacataatataaagaaagcaccaaacgtctcattgggtgagactgttaaagcaagactcaagcagttttcagtaatgaacaagctcaagaaaaaagctctgacggttatagctgagtttttgtctgcggaggaagtcgctggaatgaaggaagcatttgaaatgatggataccggaaagaagggcaagataaacctgaatgaacttaaagatggcttgcagaagcttggccatcaaatccctgatgctgatcttcatattctcatggaagcggctgacgttgatggagatggaagtttaaattatccagagtttgttgctgtatctattcatcttagaaagatggccaatgatgaacacctgcacaaagcattttcatttttcgacaaaaatcagagtggtttcatagaaatcgaagagcttcgtagtgctttgagggatgaagacgacagcaacagcgaggaagtcaccaatgccattatgcatgacgttgatacagacaaggatggtcggattagttatgaggaatttgctgcgatgatgaaggctggtacggactggagaaaagcatcgagacagtattctcgtgaacgttttaacagtctaagcttaaagttgatgagggaaggctcattacaagttgaaaacaaagtctag

SEQ ID NO: 119 - DNA, 1602 bp, Solanum lycopersicum; identical to SEQ ID NO: 9
  source 1..1602: mol_type = other DNA

SEQ ID NO: 120 - DNA, 1602 bp, Solanum lycopersicum; identical to SEQ ID NO: 9
  source 1..1602: mol_type = other DNA

SEQ ID NO: 121 - DNA, 1626 bp, Solanum lycopersicum
  source 1..1626: mol_type = other DNA
atgggtaattgctgtgtaaaaccgggtaaatctgccgaaaaaaagaataaaaagaacaacagcaaacctaaccctttttcaattgattatggggggactaaacatgcctctgggagtggaaacaagctagttgtattaaaagaaccaacagggcaaaatatacatgataagtatgatttggggcgtgagctcggaagaggagaatttggggttacttatctatgtactgacttggaaggaggagaaaaatatgcttgcaaatcgatatctaaaaagaagctaaggactgcagtggatattgatgatgttaggagagaggttgagatcatgaaacatttgcctgtgcatccgaatattgtgaccttgaaggatacttatgaggatgataatgcagtgcacattgtgatggaattgtgtgagggtggggagttgtttgatcgaatcgttgctagaggccactatacagagagagcagctgctggaattttgaagactatgtgtcacaggcaaggggtaatgcatcgtgatctcaaacctgagaattttctttttggtaacaagaaagaaacagctccactgaaggctattgactttgggttgtctgttttctttaaacctggggaacgctttaatgagatagtgggaagtccttattacatggctcctgaggtcctaaagcgcaattatggaccagaggtcgatgtctggagtgctggagttatactttacattcttctatgcggtgttccacctttctgggcagagactgaacaaggagtagcccaagcgattattcgttctgtgattgatttcaagagggatccatggcctaaagtttctgataatgcaaaggatcttgtaaagaaaatgcttgatccagatccaactcgacggctcacagctcatcaagttcttggtaatgtttgtggaatattgagatattgtactttattcattcagcatccctggttacataatataaagaaagcaccaaacgtctcattgggtgagactgttaaagcaagactcaagcagttttcagtaatgaacaagctcaagaaaaaagctctgacggttatagctgagtttttgtctgcggaggaagtcgctggaatgaaggaagcatttgaaatgatggataccggaaagaagggcaagataaacctgaatgaacttaaagatggcttgcagaagcttggccatcaaatccctgatgctgatcttcatattctcatggaagcggctgacgttgatggagatggaagtttaaattatccagagtttgttgctgtatctattcatcttagaaagatggccaatgatgaacacctgcacaaagcattttcatttttcgacaaaaatcagagtggtttcatagaaatcgaagagcttcgtagtgctttgagggatgaagacgacagcaacagcgaggaagtcaccaatgccattatgcatgacgttgatacagacaaggatggtcggattagttatgaggaatttgctgcgatgatgaaggctggtacggactggagaaaagcatcgagacagtattctcgtgaacgttttaacagtctaagcttaaagttgatgagggaaggctcattacaagttgaaaacaaagtctag

SEQ ID NO: 122 - DNA, 1602 bp, Solanum lycopersicum; identical to SEQ ID NO: 9
  source 1..1602: mol_type = other DNA

SEQ ID NO: 123 - DNA, 1602 bp, Solanum lycopersicum; identical to SEQ ID NO: 9
  source 1..1602: mol_type = other DNA

SEQ ID NO: 124 - DNA, 1587 bp, Solanum lycopersicum
  source 1..1587: mol_type = other DNA
atgggtaattgctgtgtaaaaccgggtaaatctgccgaaaaaaagaataaaaagaacaacagcaaacctaaccctttttcaattgattatggggggactaaacatgcctctgggagtggaaacaagctagttgtattaaaagaaccaacagggcaaaatatacatgataagtatgatttggggcgtgagctcggaagaggagaatttggggttacttatctatgtactgacttggaaggaggagaaaaatatgcttgcaaatcgatatctaaaaagaagctaaggactgcagtggatattgatgatgttaggagagaggttgagatcatgaaacatttgcctgtgcatccgaatattgtgaccttgaaggatacttatgaggatgataatgcagtgcacattgtgatggaattgtgtgagggtggggagttgtttgatcgaatcgttgctagaggccactatacagagagagcagctgctggaattttgaagactgtcatgtgtcacaggcaaggggtaatgcatcgtgatctcaaacctgagaattttctttttggtaacaagaaagaaacagctccactgaaggctattgactttgggttgtctgttttctttaaacctggggaacgctttaatgagatagtgggaagtccttattacatggctcctgaggtcctaaagcgcaattatggaccagaggtcgatgtctggagtgctggagttatactttacattcttctatgcggtgttccacctttctgggcagagactgaacaaggagtagcccaagcgattattcgttctgtgattgatttcaagagggatccatggcctaaagtttctgataatgcaaaggatcttgtaaagaaaatgcttgatccagatccaactcgacggctcacagctcatcaagttcttgagcatccctggttacataatataaagaaagcaccaaacgtctcattgggtgagactgttaaagcaagactcaagcagttttcagtaatgaacaagctcaagaaaaaagctctgacggttatagctgagtttttgtctgcggaggaagtcgctggaatgaaggaagcatttgaaatgatggataccggaaagaagggcaagataaacctgaatgaacttaaagatggcttgcagaagcttggccatcaaatccctgatgctgatcttcatattctcatggaagcggctgacgttgatggagatggaagtttaaattatccagagtttgttgctgtatctattcatcttagaaagatggccaatgatgaacacctgcacaaagcattttcatttttcgacaaaaatcagagtggtttcatagaaatcgaagagcttcgtagtgctttgagggatgaagacgacagcaacagcgaggaagtcaccaatgccattatgcatgacgttgatacagacaaggatggtcggattagttatgaggaatttgctgcgatgatgaaggctggtacggactggagaaaagcatcgagacagtattctcgtgaacgttttaacagtctaagcttaaagttgatgagggaaggctcattacaagttgaaaacaaagtctag

SEQ ID NO: 125 - DNA, 1602 bp, Solanum lycopersicum; identical to SEQ ID NO: 9
  source 1..1602: mol_type = other DNA

SEQ ID NO: 126 - DNA, 1788 bp, Solanum lycopersicum
  source 1..1788: mol_type = other DNA
atgaatttcttttgtggacaaagtgctcttattggattgttcaatgaagtttcgacactgaggttaggtataaagtctaattatggtgtttcaatattgggaggaatgcttcgcttttactatactcattatcaatggcagatggacggatctttcttttttctcttcttttttaccccttttttggtctataattggaaaaaaatcaacaattttcaggagttggttgatcttataaagtatcatggcaaacctaaccctttttcaattgattatggggggactaaacatgcctctgggagtggaaacaagctagttgtattaaaagaaccaacagggcaaaatatacatgataagtatgatttggggcgtgagctcggaagaggagaatttggggttacttatctatgtactgacttggaaggaggagaaaaatatgcttgcaaatcgatatctaaaaagaagctaaggactgcagtggatattgatgatgttaggagagaggttgagatcatgaaacatttgcctgtgcatccgaatattgtgaccttgaaggatacttatgaggatgataatgcagtgcacattgtgatggaattgtgtgagggtggggagttgtttgatcgaatcgttgctagaggccactatacagagagagcagctgctggaattttgaagactgtcgtggaagtcgttcagatgtgtcacaggcaaggggtaatgcatcgtgatctcaaacctgagaattttctttttggtaacaagaaagaaacagctccactgaaggctattgactttgggttgtctgttttctttaaacctggggaacgctttaatgagatagtgggaagtccttattacatggctcctgaggtcctaaagcgcaattatggaccagaggtcgatgtctggagtgctggagttatactttacattcttctatgcggtgttccacctttctgggcagagactgaacaaggagtagcccaagcgattattcgttctgtgattgatttcaagagggatccatggcctaaagtttctgataatgcaaaggatcttgtaaagaaaatgcttgatccagatccaactcgacggctcacagctcatcaagttcttgagcatccctggttacataatataaagaaagcaccaaatgtctcattgggtgagactgttaaagcaagactcaagcagttttcagtaatgaacaagctcaagaaaaaagctctgacggttatagctgagtttttgtctgcggaggaagtcgctggaatgaaggaagcatttgaaatgatggataccggaaagaagggtaagataaacctgaatgaacttaaagatggcttgcagaagcttggccatcaaatccctgatgctgatcttcatattctcatggaagcggctgacgttgatggagatggaagtttaaattatccagagtttgttgctgtatctattcatcttagaaagatggccaatgatgaacacctgcacaaagcattttcatttttcgacaaaaatcagagtggtttcatagaaatcgaagagcttcgtagtgctttgagggatgaagacgacagcaacagcgaggaagtcaccaatgccattatgcatgacgttgatacagacaaggatggtcggattagttatgaggaatttgctgcgatgatgaaggctggtacggactggagaaaagcatcgagacagtattctcgtgaacgttttaacagtctaagcttaaagttgatgagggaaggctcattacaagttgaaaacaaagtctag

SEQ ID NO: 127 - DNA, 1602 bp, Solanum lycopersicum; identical to SEQ ID NO: 9
  source 1..1602: mol_type = other DNA

SEQ ID NO: 128 - DNA, 1584 bp, Solanum lycopersicum
  source 1..1584: mol_type = other DNA
atgggtaattgctgtgtgaaaccgggtaaatctgccgaaaaaaagaataaaaagaacaacagcaaacctaaccctttttcaattgattatggggggactaaacatgcctctgggagtggaaacaagctagttgtattaaaagaaccaacagggcaaaatatacatgataagtatgatttggggcatgagctcggaagaggagaatttggggttacttatctatgtactgacttggaaggaggagaaaaatatgcttgcaaatcgatatctaaaaagaagctaaggactgcagtggatattgatgatgttaggagagaggttgagatcatgaaacatttgcctgtgcatccgaatattgtgaccttgaaggatacttatgaggatgataatgcagtgcacattgtgatggaattgtgtgagggtggggagttgtttgatcgaatcgttgctagaggccactatacagagagagcagctgctggaattttgaagactatgtgtcacaggcaaggggtaatgcatcgtgatctcaaacctgagaattttctttttggtaacaagaaagaaacagctccactgaaggctattgactttgggttgtctgttttctttaaacctggggaacgctttaatgagatagtgggaagtccttattacatggctcctgaggtcctaaagcgcaattatggaccagaggtcgatgtctggagtgctggagttatactttacattcttctatgcggtgttccacctttctgggcagagactgaacaaggagtagcccaagcgattattcgttctgtgattgatttcaagagggatccatggcctaaagtttctgataatgcaaaggatcttgtaaagaaaatgcttgatccagatccaactcgacggctcacagctcatcaagttcttgagcatccctggttacataatataaagaaagcaccaaacgtctcattgggtgagactgttaaagcaagactcaagcagttttcagtaatgaacaagctcaagaaaaaagctctgacggttatagctgagtttttgtctgcggaggaagtcgctggaatgaaggaagcatttgaaatgatggataccggaaagaagggcaagataaacctgaatgaacttaaagatggcttgcagaagcttggccatcaaatccctgatgctgatcttcatattctcatggaagcggctgacgttgatggagatggaagtttaaattatccagagtttgttgctgtatctattcatcttagaaagatggccaatgatgaacacctgcacaaagcattttcatttttcgacaaaaatcagagtggtttcatagaaatcgaagagcttcgtagtgctttgagggatgaagacgacagcaacagcgaggaagtcaccaatgccattatgcatgacgttgatacagacaaggatggtcggattagttatgaggaatttgctgcgatgatgaaggctggtacggactggagaaaagcatcgagacagtattctcgtgaacgttttaacagtctaagcttaaagttgatgagggaaggctcattacaagttgaaaacaaagtctag

SEQ ID NO: 129 - DNA, 1602 bp, Solanum lycopersicum; identical to SEQ ID NO: 9
  source 1..1602: mol_type = other DNA

SEQ ID NO: 130 - DNA, 1602 bp, Solanum lycopersicum; identical to SEQ ID NO: 9
  source 1..1602: mol_type = other DNA

SEQ ID NO: 131 - DNA, 1602 bp, Solanum lycopersicum; identical to SEQ ID NO: 9
  source 1..1602: mol_type = other DNA

SEQ ID NO: 132 - DNA, 1602 bp, Solanum lycopersicum; identical to SEQ ID NO: 9
  source 1..1602: mol_type = other DNA

SEQ ID NO: 133 - DNA, 1587 bp, Solanum lycopersicum
  source 1..1587: mol_type = other DNA
atgggtaattgctgtgtgaaaccgggtaaatctgccgaaaaaaagaataaaaagaacaacagcaaacctaaccctttttcaattgattatggggggactaaacatgcctctgggagtggaaacaagctagttgtattaaaagaaccaacagggcaaaatatacatgataagtatgatttggggcatgagctcggaagaggagaatttggggttacttatctatgtactgacttggaaggaggagaaaaatatgcttgcaaatcgatatctaaaaagaagctaaggactgcagtggatattgatgatgttaggagagaggttgagatcatgaaacatttgcctgtgcatccgaatattgtgaccttgaaggatacttatgaggatgataatgcagtgcacattgtgatggaattgtgtgagggtggggagttgtttgatcgaatcgttgctagaggccactatacagagagagcagctgctggaattttgaagactgtcatgtgtcacaggcaaggggtaatgcatcgtgatctcaaacctgagaattttctttttggtaacaagaaagaaacagctccactgaaggctattgactttgggttgtctgttttctttaaacctggggaacgctttaatgagatagtgggaagtccttattacatggctcctgaggtcctaaagcgcaattatggaccagaggtcgatgtctggagtgctggagttatactttacattcttctatgcggtgttccacctttctgggcagagactgaacaaggagtagcccaagcgattattcgttctgtgattgatttcaagagggatccatggcctaaagtttctgataatgcaaaggatcttgtaaagaaaatgcttgatccagatccaactcgacggctcacagctcatcaagttcttgagcatccctggttacataatataaagaaagcaccaaacgtctcattgggtgagactgttaaagcaagactcaagcagttttcagtaatgaacaagctcaagaaaaaagctctgacggttatagctgagtttttgtctgcggaggaagtcgctggaatgaaggaagcatttgaaatgatggataccggaaagaagggcaagataaacctgaatgaacttaaagatggcttgcagaagcttggccatcaaatccctgatgctgatcttcatattctcatggaagcggctgacgttgatggagatggaagtttaaattatccagagtttgttgctgtatctattcatcttagaaagatggccaatgatgaacacctgcacaaagcattttcatttttcgacaaaaatcagagtggtttcatagaaatcgaagagcttcgtagtgctttgagggatgaagacgacagcaacagcgaggaagtcaccaatgccattatgcatgacgttgatacagacaaggatggtcggattagttatgaggaatttgctgcgatgatgaaggctggtacggactggagaaaagcatcgagacagtattctcgtgaacgttttaacagtctaagcttaaagttgatgagggaaggctcattacaagttgaaaacaaagtctag

SEQ ID NO: 134 - DNA, 1602 bp, Solanum lycopersicum; identical to SEQ ID NO: 9
  source 1..1602: mol_type = other DNA

SEQ ID NO: 135 - DNA, 1602 bp, Solanum lycopersicum; identical to SEQ ID NO: 9
  source 1..1602: mol_type = other DNA

SEQ ID NO: 136 - DNA, 1602 bp, Solanum lycopersicum; identical to SEQ ID NO: 9
  source 1..1602: mol_type = other DNA

SEQ ID NO: 137 - DNA, 1614 bp, Solanum lycopersicum
  source 1..1614: mol_type = other DNA
atggcggatttttcttttttctcttcttttttaccccttttttggtctataattggaaaaaaatcaacaattttcagtatcatgggtaattgctgtgtgaaaccgggtaaatctgccgaaaaaaagaataaaaagaacaacagcaaacctaaccctttttcaattgattatggggggactaaacatgcctctgggagtggaaacaagctagttgtattaaaagaaccaacagggcaaaatatacatgataagtatgatttggggcgtgagctcggaagaggagaatttggggttacttatctatgtactgacttggaaggaggagaaaaatatgcttgcaaatcgatatctaaaaagaagctaaggactgcagtggatattgatgatgttaggagagaggttgagatcatgaaacatttgcctgtgcatccgaatattgtgaccttgaaggatacttatgaggatgataatgcagtgcacattgtgatggaattgtgtgagggtggggagttgtttgatcgaatcatgtgtcacaggcaaggggtaatgcatcgtgatctcaaacctgagaattttctttttggtaacaagaaagaaacagctccactgaaggctattgactttgggttgtctgttttctttaaacctggggaacgctttaatgagatagtgggaagtccttattacatggctcctgaggtcctaaagcgcaattatggaccagaggtcgatgtctggagtgctggagttatactttacattcttctatgcggtgttccacctttctgggcagagactgaacaaggagtagcccaagcgattattcgttctgtgattgatttcaagagggatccatggcctaaagtttctgataatgcaaaggatcttgtaaagaaaatgcttgatccagatccaactcgacggctcacagctcatcaagttcttgagcatccctggttacataatataaagaaagcaccaaacgtctcattgggtgagactgttaaagcaagactcaagcagttttcagtaatgaacaagctcaagaaaaaagctctgacggttatagctgagtttttgtctgcggaggaagtcgctggaatgaaggaagcatttgaaatgatggataccggaaagaagggcaagataaacctgaatgaacttaaagatggcttgcagaagcttggccatcaaatccctgatgctgatcttcagattctcatggaagcggctgacgttgatggagatggaagtttaaattatccagagtttgttgctgtatctattcatcttagaaagatggccaatgatgaacacctgcacaaagcattttcattttttgacaaaaaccaaagtggtttcatagaaatcgaagagcttcgtagtgctttgagggatgaagacgacagcaacagcaaggaagtcaccgatgccattatgcatgacgttgatacagacaaggatggtcggattagttatgaggaatttgctgcgatgatgaaggctggtacggactggagaaaagcatcgagacagtattctcgtgaacgttttaacagtctaagcttaaagttgatgagggaaggctcattacaagttgaaaacaaagtctag

SEQ ID NO: 138 - DNA, 1602 bp, Solanum lycopersicum; identical to SEQ ID NO: 9
  source 1..1602: mol_type = other DNA

SEQ ID NO: 139 - DNA, 1602 bp, Solanum lycopersicum; identical to SEQ ID NO: 9
  source 1..1602: mol_type = other DNA

SEQ ID NO: 140 - DNA, 1602 bp, Solanum lycopersicum; identical to SEQ ID NO: 9
  source 1..1602: mol_type = other DNA

SEQ ID NO: 141 - DNA, 1584 bp, Solanum lycopersicum
  source 1..1584: mol_type = other DNA
atgggtaattgctgtgtaaaaccgggtaaatctgccgaaaaaaagaataaaaagaacaacagcaaacctaaccctttttcaattgattatggggggactaaacatgcctctgggagtggaaacaagctagttgtattaaaagaaccaacagggcaaaatatacatgataagtatgatttggggcgtgagctcggaagaggagaatttggggttacttatctatgtactgacttggaaggaggagaaaaatatgcttgcaaatcgatatctaaaaagaagctaaggactgcagtggatattgatgatgttaggagagaggttgagatcatgaaacatttgcctgtgcatccgaatattgtgaccttgaaggatacttatgaggatgataatgcagtgcacattgtgatggaattgtgtgagggtggggagttgtttgatcgaatcgttgctagaggccactatacagagagagcagctgctggaattttgaagactatgtgtcacaggcaaggggtaatgcatcgtgatctcaaacctgagaattttctttttggtaacaagaaagaaacagctccactgaaggctattgactttgggttgtctgttttctttaaacctggggaacgctttaatgagatagtgggaagtccttattacatggctcctgaggtcctaaagcgcaattatggaccagaggtcgatgtctggagtgctggagttatactttacattcttctatgcggtgttccacctttctgggcagagactgaacaaggagtagcccaagcgattattcgttctgtgattgatttcaagagggatccatggcctaaagtttctgataatgcaaaggatcttgtaaagaaaatgcttgatccagatccaactcgacggctcacagctcatcaagttcttgagcatccctggttacataatataaagaaagcaccaaacgtctcattgggtgagactgttaaagcaagactcaagcagttttcagtaatgaacaagctcaagaaaaaagctctgacggttatagctgagtttttgtctgcggaggaagtcgctggaatgaaggaagcatttgaaatgatggataccggaaagaagggcaagataaacctgaatgaacttaaagatggcttgcagaagcttggccatcaaatccctgatgctgatcttcatattctcatggaagcggctgacgttgatggagatggaagtttaaattatccagagtttgttgctgtatctattcatcttagaaagatggccaatgatgaacacctgcacaaagcattttcatttttcgacaaaaatcagagtggtttcatagaaatcgaagagcttcgtagtgctttgagggatgaagacgacagcaacagcgaggaagtcaccaatgccattatgcatgacgttgatacagacaaggatggtcggattagttatgaggaatttgctgcgatgatgaaggctggtacggactggagaaaagcatcgagacagtattctcgtgaacgttttaacagtctaagcttaaagttgatgagggaaggctcattacaagttgaaaacaaagtctag

SEQ ID NO: 142 - DNA, 1602 bp, Solanum lycopersicum; identical to SEQ ID NO: 9
  source 1..1602: mol_type = other DNA

SEQ ID NO: 143 - DNA, 1587 bp, Solanum lycopersicum; identical to SEQ ID NO: 124
  source 1..1587: mol_type = other DNA

SEQ ID NO: 144 - DNA, 1479 bp, Solanum lycopersicum
  source 1..1479: mol_type = other DNA
atgggtaattgctgtgtgaaaccgggtaaatctgccgaaaaaaagaataaaaagaacaacagcaaacctaaccctttttcaattgattatggggggactaaacatgcctctgggagtggaaacaagctagttgtattaaaagaaccaacagggcaaaatatacatgataagtatgatttggggcgaggagaaaaatatgcttgcaaatcgatatctaaaaagaagctaaggactgcagtggatattgatgatgttaggagagaggttgagatcatgaaacatttgcctgtgcatccgaatattgtgaccttgaaggatacttatgaggatgataatgcagtgcacattgtgatggaattgtgtgagggtggggagttgtttgatcgaatcatgtgtcacaggcaaggggtaatgcatcgtgatctcaaacctgagaattttctttttggtaacaagaaagaaacagctccactgaaggctattgactttgggttgtctgttttctttaaacctggggaacgctttaatgagatagtgggaagtccttattacatggctcctgaggtcctaaagcgcaattatggaccagaggtcgatgtctggagtgctggagttatactttacattcttctatgcggtgttccacctttctgggcagagactgaacaaggagtagcccaagcgattattcgttctgtgattgatttcaagagggatccatggcctaaagtttctgataatgcaaaggatcttgtaaagaaaatgcttgatccagatccaactcgacggctcacagctcatcaagttcttgagcatccctggttacataatataaagaaagcaccaaacgtctcattgggtgagactgttaaagcaagactcaagcagttttcagtaatgaacaagctcaagaaaaaagctctgacggttatagctgagtttttgtctgcggaggaagtcgctggaatgaaggaagcatttgaaatgatggataccggaaagaagggcaagataaacctgaatgaacttaaagatggcttgcagaagcttggccatcaaatccctgatgctgatcttcagattctcatggaagcggctgacgttgatggagatggaagtttaaattatccagagtttgttgctgtatctattcatcttagaaagatggccaatgatgaacacctgcacaaagcattttcattttttgacaaaaaccaaagtggtttcatagaaatcgaagagcttcgtagtgctttgagggatgaagacgacagcaacagcaaggaagtcaccgatgccattatgcatgacgttgatacagacaaggatggtcggattagttatgaggaatttgctgcgatgatgaaggctggtacggactggagaaaagcatcgagacagtattctcgtgaacgttttaacagtctaagcttaaagttgatgagggaaggctcattacaagttgaaaacaaagtctag

SEQ ID NO: 145 - DNA, 1602 bp, Solanum lycopersicum; identical to SEQ ID NO: 9
  source 1..1602: mol_type = other DNA

SEQ ID NO: 146 - DNA, 1647 bp, Solanum lycopersicum
  source 1..1647: mol_type = other DNA
atggcggatttttcttttttctcttcttttttaccccttttttggtctataattggaaaaaaatcaacaattttcagtatcatgggtaattgctgtgtgaaaccgggtaaatctgccgaaaaaaagaataaaaagaacaacagcaaacctaaccctttttcaattgattatggggggactaaacatgcctctgggagtggaaacaagctagttgtattaaaagaaccaacagggcaaaatatacatgataagtatgatttggggcgtgagctcggaagaggagaatttggggttacttatctatgtactgacttggaaggaggagaaaaatatgcttgcaaatcgatatctaaaaagaagctaaggactgcagtggatattgatgatgttaggagagaggttgagatcatgaaacatttgcctgtgcatccgaatattgtgaccttgaaggatacttatgaggatgataatgcagtgcacattgtgatggaattgtgtgagggtggggagttgtttgatcgaatcgttgctagaggccactatacagagagagcagctgctggaattttgaagactgtcatgtgtcacaggcaaggggtaatgcatcgtgatctcaaacctgagaattttctttttggtaacaagaaagaaacagctccactgaaggctattgactttgggttgtctgttttctttaaacctggggaacgctttaatgagatagtgggaagtccttattacatggctcctgaggtcctaaagcgcaattatggaccagaggtcgatgtctggagtgctggagttatactttacattcttctatgcggtgttccacctttctgggcagagactgaacaaggagtagcccaagcgattattcgttctgtgattgatttcaagagggatccatggcctaaagtttctgataatgcaaaggatcttgtaaagaaaatgcttgatccagatccaactcgacggctcacagctcatcaagttcttggtaataaagcaccaaacgtctcattgggtgagactgttaaagcaagactcaagcagttttcagtaatgaacaagctcaagaaaaaagctctgacggttatagctgagtttttgtctgcggaggaagtcgctggaatgaaggaagcatttgaaatgatggataccggaaagaagggcaagataaacctgaatgaacttaaagatggcttgcagaagcttggccatcaaatccctgatgctgatcttcatattctcatggaagcggctgacgttgatggagatggaagtttaaattatccagagtttgttgctgtatctattcatcttagaaagatggccaatgatgaacacctgcacaaagcattttcatttttcgacaaaaatcagagtggtttcatagaaatcgaagagcttcgtagtgctttgagggatgaagacgacagcaacagcgaggaagtcaccaatgccattatgcatgacgttgatacagacaaggatggtcggattagttatgaggaatttgctgcgatgatgaaggctggtacggactggagaaaagcatcgagacagtattctcgtgaacgttttaacagtctaagcttaaagttgatgagggaaggctcattacaagttgaaaacaaagtctag

SEQ ID NO: 147 - DNA, 1602 bp, Solanum lycopersicum; identical to SEQ ID NO: 9
  source 1..1602: mol_type = other DNA

SEQ ID NO: 148 - DNA, 1587 bp, Solanum lycopersicum
  source 1..1587: mol_type = other DNA
atgggtaattgctgtgtgaaaccgggtaaatctgccgaaaaaaagaataaaaagaacaacagcaaacctaaccctttttcaattgattatggggggactaaacatgcctctgggagtggaaacaagctagttgtattaaaagaaccaacagggcaaaatatacatgataagtatgatttggggcgtgagctcggaagaggagaatttggggttacttatctatgtactgacttggaaggaggagaaaaatatgcttgcaaatcgatatctaaaaagaagctaaggactgcagtggatattgatgatgttaggagagaggttgagatcatgaaacatttgcctgtgcatccgaatattgtgaccttgaaggatacttatgaggatgataatgcagtgcacattgtgatggaattgtgtgagggtggggagttgtttgatcgaatcgttgctagaggccactatacagagagagcagctgctggaattttgaagactgtcatgtgtcacaggcaaggggtaatgcatcgtgatctcaaacctgagaattttctttttggtaacaagaaagaaacagctccactgaaggctattgactttgggttgtctgttttctttaaacctggggaacgctttaatgagatagtgggaagtccttattacatggctcctgaggtcctaaagcgcaattatggaccagaggtcgatgtctggagtgctggagttatactttacattcttctatgcggtgttccacctttctgggcagagactgaacaaggagtagcccaagcgattattcgttctgtgattgatttcaagagggatccatggcctaaagtttctgataatgcaaaggatcttgtaaagaaaatgcttgatccagatccaactcgacggctcacagctcatcaagttcttgagcatccctggttacataatataaagaaagcaccaaacgtctcattgggtgagactgttaaagcaagactcaagcagttttcagtaatgaacaagctcaagaaaaaagctctgacggttatagctgagtttttgtctgcggaggaagtcgctggaatgaaggaagcatttgaaatgatggataccggaaagaagggcaagataaacctgaatgaacttaaagatggcttgcagaagcttggccatcaaatccctgatgctgatcttcatattctcatggaagcggctgacgttgatggagatggaagtttaaattatccagagtttgttgctgtatctattcatcttagaaagatggccaatgatgaacacctgcacaaagcattttcatttttcgacaaaaatcagagtggtttcatagaaatcgaagagcttcgtagtgctttgagggatgaagacgacagcaacagcgaggaagtcaccaatgccattatgcatgacgttgatacagacaaggatggtcggattagttatgaggaatttgctgcgatgatgaaggctggtacggactggagaaaagcatcgagacagtattctcgtgaacgttttaacagtctaagcttaaagttgatgagggaaggctcattacaagttgaaaacaaagtctag

SEQ ID NO: 149 - DNA, 1602 bp, Solanum lycopersicum; identical to SEQ ID NO: 9
  source 1..1602: mol_type = other DNA

SEQ ID NO: 150 - DNA, 1602 bp, Solanum lycopersicum; identical to SEQ ID NO: 9
  source 1..1602: mol_type = other DNA

SEQ ID NO: 151 - DNA, 1602 bp, Solanum lycopersicum
  source 1..1602: mol_type = other DNA
atgggtaattgctgtgtgaaaccgggtaaatctgccgaaaaaaagaataaaaagaacaacagcaaacctaaccctttttcaattgattatggggggactaaacatgcctctgggagtggaaacaagctagttgtattaaaagaaccaacagggcaaaatatacatgataagtatgatttggggcgtgagctcggaagaggagaatttggggttacttatctatgtactgacttggaaggaggagaaaaatatgcttgcaaatcgatatctaaaaagaagctaaggactgcagtggatattgatgatgttaggagagaggttgagatcatgaaacatttgcctgtgcatccgaatattgtgaccttgaaggatacttatgaggatgataatgcagtgcacattgtgatggaattgtgtgagggtggggagttgtttgatcgaatcgttgctagaggccactatacagagagggcagctgctggaattttgaagactgtcgtggaagttgttcagatgtgtcacaggcaaggggtaatgcatcgtgatctcaaacctgagaattttctttttggtaacaagaaagaaacagctccactgaaggctattgactttgggttgtctgttttctttaaacctggggaacgctttaatgagatagtgggaagtccttattacatggctcctgaggtcctaaagcgcaattatggaccagaggtcgatgtctggagtgctggagttatactttacattcttctatgcggtgttccacctttctgggcagagactgaacaaggagtagcccaagcgattattcgttctgtgattgatttcaagagggatccatggcctaaagtttctgataatgcaaaggatcttgtaaagaaaatgcttgatccagatccaactcgacggctcacagctcatcaagttcttgagcatccctggttacataatataaagaaagcaccaaacgtctcattgggtgagactgttaaagcaagactcaagcagttttcagtaatgaacaagctcaagaaaaaagctctgacggttatagctgagtttttgtctgcggaggaagtcgctggaatgaaggaagcatttgaaatgatggataccggaaagaagggcaagataaacctgaatgaacttaaagatggcttgcagaagcttggccatcaaatccctgatgctgatcttcagattctcatggaagcggctgacgttgatggagatggaagtttaaattatccagagtttgttgctgtatctattcatcttagaaagatggccaatgatgaacacctgcacaaagcattttcattttttgacaaaaaccaaagtggtttcatagaaatcgaagagcttcgtagtgctttgagggatgaagacgacagcaacagcaaggaagtcaccgatgccattatgcatgacgttgatacagacaaggatggtcggattagttatgaggaatttgctgcgatgatgaaggctggtacggactggagaaaagcatcgagacagtattctcgtgaacgttttaacagtctaagcttaaagttgatgagggaaggctcattacaagttgaaaacaaagtctag

SEQ ID NO: 152 - DNA, 1626 bp, Solanum lycopersicum
  source 1..1626: mol_type = other DNA
atgggtaattgctgtgtgaaaccgggtaaatctgccgaaaaaaagaataaaaagaacaacagcaaacctaaccctttttcaattgattatggggggactaaacatgcctctgggagtggaaacaagctagttgtattaaaagaaccaacagggcaaaatatacatgataagtatgatttggggcatgagctcggaagaggagaatttggggttacttatctatgtactgacttggaaggaggagaaaaatatgcttgcaaatcgatatctaaaaagaagctaaggactgcagtggatattgatgatgttaggagagaggttgagatcatgaaacatttgcctgtgcatccgaatattgtgaccttgaaggatacttatgaggatgataatgcagtgcacattgtgatggaattgtgtgagggtggggagttgtttgatcgaatcgttgctagaggccactatacagagagagcagctgctggaattttgaagactatgtgtcacaggcaaggggtaatgcatcgtgatctcaaacctgagaattttctttttggtaacaagaaagaaacagctccactgaaggctattgactttgggttgtctgttttctttaaacctggggaacgctttaatgagatagtgggaagtccttattacatggctcctgaggtcctaaagcgcaattatggaccagaggtcgatgtctggagtgctggagttatactttacattcttctatgcggtgttccacctttctgggcagagactgaacaaggagtagcccaagcgattattcgttctgtgattgatttcaagagggatccatggcctaaagtttctgataatgcaaaggatcttgtaaagaaaatgcttgatccagatccaactcgacggctcacagctcatcaagttcttggtaatgtttgtggaatattgagatattgtactttattcattcagcatccctggttacataatataaagaaagcaccaaacgtctcattgggtgagactgttaaagcaagactcaagcagttttcagtaatgaacaagctcaagaaaaaagctctgacggttatagctgagtttttgtctgcggaggaagtcgctggaatgaaggaagcatttgaaatgatggataccggaaagaagggcaagataaacctgaatgaacttaaagatggcttgcagaagcttggccatcaaatccctgatgctgatcttcatattctcatggaagcggctgacgttgatggagatggaagtttaaattatccagagtttgttgctgtatctattcatcttagaaagatggccaatgatgaacacctgcacaaagcattttcatttttcgacaaaaatcagagtggtttcatagaaatcgaagagcttcgtagtgctttgagggatgaagacgacagcaacagcgaggaagtcaccaatgccattatgcatgacgttgatacagacaaggatggtcggattagttatgaggaatttgctgcgatgatgaaggctggtacggactggagaaaagcatcgagacagtattctcgtgaacgttttaacagtctaagcttaaagttgatgagggaaggctcattacaagttgaaaacaaagtctag

SEQ ID NO: 153 - protein, 533 aa, Solanum lycopersicum; identical to SEQ ID NO: 10

SEQ ID NO: 154 - protein, 547 aa, Solanum lycopersicum
MGNCCVKPGKSAEKKNKKNNSKPNPFSIDYGGTKHASGSGNKLVVLKEPTGQNIHDKYDLGRELGRGEFGVTYLCTDLEGGEKYACKSISKKKLRTAVDIDDVRREVEIMKHLPVHPNIVTLKDTYEDDNAVHIVMELCEGGELFDRIVARGHYTERAAAGILKTVVEVVQMCHRQGVMHRDLKPENFLFGNKKETAPLKAIDFGLSVFFKPGERFNEIVGSPYYMAPEVLKRNYGPEVDVWSAGVILYILLCGVPPFWAETEQGVAQAIIRSVIDFKRDPWPKVSDNAKDLVKKMLDPDPTRRLTAHQVLGNVCGILRYCTLFIQHPWLHNIKKAPNVSLGETVKARLKQFSVMNKLKKKALTVIAEFLSAEEVAGMKEAFEMMDTGKKGKINLNELKDGLQKLGHQIPDADLHILMEAADVDGDGSLNYPEFVAVSIHLRKMANDEHLHKAFSFFDKNQSGFIEIEELRSALRDEDDSNSEEVTNAIMHDVDTDKDGRISYEEFAAMMKAGTDWRKASRQYSRERFNSLSLKLMREGSLQVENKV

SEQ ID NO: 155 - protein, 533 aa, Solanum lycopersicum; identical to SEQ ID NO: 10

SEQ ID NO: 156 - protein, 533 aa, Solanum lycopersicum; identical to SEQ ID NO: 10

SEQ ID NO: 157 - protein, 533 aa, Solanum lycopersicum; identical to SEQ ID NO: 10

SEQ ID NO: 158 - protein, 533 aa, Solanum lycopersicum; identical to SEQ ID NO: 10

SEQ ID NO: 159 - protein, 533 aa, Solanum lycopersicum; identical to SEQ ID NO: 10

SEQ ID NO: 160 - protein, 533 aa, Solanum lycopersicum; identical to SEQ ID NO: 10

SEQ ID NO: 161 - protein, 533 aa, Solanum lycopersicum; identical to SEQ ID NO: 10

SEQ ID NO: 162 - protein, 544 aa, Solanum lycopersicum
MGNCCVKPGKSAEKKNKKNNSKPNPFSIDYGGTKHASGSGNKLVVLKEPTGQNIHDKYDLGRELGRGEFGVTYLCTDLEGGEKYACKSISKKKLRTAVDIDDVRREVEIMKHLPVHPNIVTLKDTYEDDNAVHIVMELCEGGELFDRIVARGHYTERAAAGILKTVVEMCHRQGVMHRDLKPENFLFGNKKETAPLKAIDFGLSVFFKPGERFNEIVGSPYYMAPEVLKRNYGPEVDVWSAGVILYILLCGVPPFWAETEQGVAQAIIRSVIDFKRDPWPKVSDNAKDLVKKMLDPDPTRRLTAHQVLGNVCGILRYCTLFIQHPWLHNIKKAPNVSLGETVKARLKQFSVMNKLKKKALTVIAEFLSAEEVAGMKEAFEMMDTGKKGKINLNELKDGLQKLGHQIPDADLHILMEAADVDGDGSLNYPEFVAVSIHLRKMANDEHLHKAFSFFDKNQSGFIEIEELRSALRDEDDSNSEEVTNAIMHDVDTDKDGRISYEEFAAMMKAGTDWRKASRQYSRERFNSLSLKLMREGSLQVENKV

SEQ ID NO: 163 - protein, 533 aa, Solanum lycopersicum; identical to SEQ ID NO: 10

SEQ ID NO: 164 - protein, 533 aa, Solanum lycopersicum; identical to SEQ ID NO: 10

SEQ ID NO: 165 - protein, 541 aa, Solanum lycopersicum
MGNCCVKPGKSAEKKNKKNNSKPNPFSIDYGGTKHASGSGNKLVVLKEPTGQNIHDKYDLGRELGRGEFGVTYLCTDLEGGEKYACKSISKKKLRTAVDIDDVRREVEIMKHLPVHPNIVTLKDTYEDDNAVHIVMELCEGGELFDRIVARGHYTERAAAGILKTMCHRQGVMHRDLKPENFLFGNKKETAPLKAIDFGLSVFFKPGERFNEIVGSPYYMAPEVLKRNYGPEVDVWSAGVILYILLCGVPPFWAETEQGVAQAIIRSVIDFKRDPWPKVSDNAKDLVKKMLDPDPTRRLTAHQVLGNVCGILRYCTLFIQHPWLHNIKKAPNVSLGETVKARLKQFSVMNKLKKKALTVIAEFLSAEEVAGMKEAFEMMDTGKKGKINLNELKDGLQKLGHQIPDADLHILMEAADVDGDGSLNYPEFVAVSIHLRKMANDEHLHKAFSFFDKNQSGFIEIEELRSALRDEDDSNSEEVTNAIMHDVDTDKDGRISYEEFAAMMKAGTDWRKASRQYSRERFNSLSLKLMREGSLQVENKV

SEQ ID NO: 166 - protein, 533 aa, Solanum lycopersicum; identical to SEQ ID NO: 10

SEQ ID NO: 167 - protein, 533 aa, Solanum lycopersicum; identical to SEQ ID NO: 10

SEQ ID NO: 168 - protein, 528 aa, Solanum lycopersicum
MGNCCVKPGKSAEKKNKKNNSKPNPFSIDYGGTKHASGSGNKLVVLKEPTGQNIHDKYDLGRELGRGEFGVTYLCTDLEGGEKYACKSISKKKLRTAVDIDDVRREVEIMKHLPVHPNIVTLKDTYEDDNAVHIVMELCEGGELFDRIVARGHYTERAAAGILKTVMCHRQGVMHRDLKPENFLFGNKKETAPLKAIDFGLSVFFKPGERFNEIVGSPYYMAPEVLKRNYGPEVDVWSAGVILYILLCGVPPFWAETEQGVAQAIIRSVIDFKRDPWPKVSDNAKDLVKKMLDPDPTRRLTAHQVLEHPWLHNIKKAPNVSLGETVKARLKQFSVMNKLKKKALTVIAEFLSAEEVAGMKEAFEMMDTGKKGKINLNELKDGLQKLGHQIPDADLHILMEAADVDGDGSLNYPEFVAVSIHLRKMANDEHLHKAFSFFDKNQSGFIEIEELRSALRDEDDSNSEEVTNAIMHDVDTDKDGRISYEEFAAMMKAGTDWRKASRQYSRERFNSLSLKLMREGSLQVENKV

SEQ ID NO: 169 - protein, 533 aa, Solanum lycopersicum; identical to SEQ ID NO: 10

SEQ ID NO: 170 - protein, 595 aa, Solanum lycopersicum
MNFFCGQSALIGLFNEVSTLRLGIKSNYGVSILGGMLRFYYTHYQWQMDGSFFFLFFFTPFLVYNWKKINNFQELVDLIKYHGKPNPFSIDYGGTKHASGSGNKLVVLKEPTGQNIHDKYDLGRELGRGEFGVTYLCTDLEGGEKYACKSISKKKLRTAVDIDDVRREVEIMKHLPVHPNIVTLKDTYEDDNAVHIVMELCEGGELFDRIVARGHYTERAAAGILKTVVEVVQMCHRQGVMHRDLKPENFLFGNKKETAPLKAIDFGLSVFFKPGERFNEIVGSPYYMAPEVLKRNYGPEVDVWSAGVILYILLCGVPPFWAETEQGVAQAIIRSVIDFKRDPWPKVSDNAKDLVKKMLDPDPTRRLTAHQVLEHPWLHNIKKAPNVSLGETVKARLKQFSVMNKLKKKALTVIAEFLSAEEVAGMKEAFEMMDTGKKGKINLNELKDGLQKLGHQIPDADLHILMEAADVDGDGSLNYPEFVAVSIHLRKMANDEHLHKAFSFFDKNQSGFIEIEELRSALRDEDDSNSEEVTNAIMHDVDTDKDGRISYEEFAAMMKAGTDWRKASRQYSRERFNSLSLKLMREGSLQVENKV

SEQ ID NO: 171 - protein, 533 aa, Solanum lycopersicum; identical to SEQ ID NO: 10

SEQ ID NO: 172 - protein, 527 aa, Solanum lycopersicum
MGNCCVKPGKSAEKKNKKNNSKPNPFSIDYGGTKHASGSGNKLVVLKEPTGQNIHDKYDLGHELGRGEFGVTYLCTDLEGGEKYACKSISKKKLRTAVDIDDVRREVEIMKHLPVHPNIVTLKDTYEDDNAVHIVMELCEGGELFDRIVARGHYTERAAAGILKTMCHRQGVMHRDLKPENFLFGNKKETAPLKAIDFGLSVFFKPGERFNEIVGSPYYMAPEVLKRNYGPEVDVWSAGVILYILLCGVPPFWAETEQGVAQAIIRSVIDFKRDPWPKVSDNAKDLVKKMLDPDPTRRLTAHQVLEHPWLHNIKKAPNVSLGETVKARLKQFSVMNKLKKKALTVIAEFLSAEEVAGMKEAFEMMDTGKKGKINLNELKDGLQKLGHQIPDADLHILMEAADVDGDGSLNYPEFVAVSIHLRKMANDEHLHKAFSFFDKNQSGFIEIEELRSALRDEDDSNSEEVTNAIMHDVDTDKDGRISYEEFAAMMKAGTDWRKASRQYSRERFNSLSLKLMREGSLQVENKV

SEQ ID NO: 173 - protein, 533 aa, Solanum lycopersicum; identical to SEQ ID NO: 10

SEQ ID NO: 174 - protein, 533 aa, Solanum lycopersicum; identical to SEQ ID NO: 10

SEQ ID NO: 175 - protein, 533 aa, Solanum lycopersicum; identical to SEQ ID NO: 10

SEQ ID NO: 176 - protein, 533 aa, Solanum lycopersicum; identical to SEQ ID NO: 10

SEQ ID NO: 177 - protein, 528 aa, Solanum lycopersicum
MGNCCVKPGKSAEKKNKKNNSKPNPFSIDYGGTKHASGSGNKLVVLKEPTGQNIHDKYDLGHELGRGEFGVTYLCTDLEGGEKYACKSISKKKLRTAVDIDDVRREVEIMKHLPVHPNIVTLKDTYEDDNAVHIVMELCEGGELFDRIVARGHYTERAAAGILKTVMCHRQGVMHRDLKPENFLFGNKKETAPLKAIDFGLSVFFKPGERFNEIVGSPYYMAPEVLKRNYGPEVDVWSAGVILYILLCGVPPFWAETEQGVAQAIIRSVIDFKRDPWPKVSDNAKDLVKKMLDPDPTRRLTAHQVLEHPWLHNIKKAPNVSLGETVKARLKQFSVMNKLKKKALTVIAEFLSAEEVAGMKEAFEMMDTGKKGKINLNELKDGLQKLGHQIPDADLHILMEAADVDGDGSLNYPEFVAVSIHLRKMANDEHLHKAFSFFDKNQSGFIEIEELRSALRDEDDSNSEEVTNAIMHDVDTDKDGRISYEEFAAMMKAGTDWRKASRQYSRERFNSLSLKLMREGSLQVENKV

SEQ ID NO: 178 - protein, 533 aa, Solanum lycopersicum; identical to SEQ ID NO: 10

SEQ ID NO: 179 - protein, 533 aa, Solanum lycopersicum; identical to SEQ ID NO: 10

SEQ ID NO: 180 - protein, 533 aa, Solanum lycopersicum; identical to SEQ ID NO: 10

SEQ ID NO: 181 - protein, 537 aa, Solanum lycopersicum
MADFSFFSSFLPLFWSIIGKKSTIFSIMGNCCVKPGKSAEKKNKKNNSKPNPFSIDYGGTKHASGSGNKLVVLKEPTGQNIHDKYDLGRELGRGEFGVTYLCTDLEGGEKYACKSISKKKLRTAVDIDDVRREVEIMKHLPVHPNIVTLKDTYEDDNAVHIVMELCEGGELFDRIMCHRQGVMHRDLKPENFLFGNKKETAPLKAIDFGLSVFFKPGERFNEIVGSPYYMAPEVLKRNYGPEVDVWSAGVILYILLCGVPPFWAETEQGVAQAIIRSVIDFKRDPWPKVSDNAKDLVKKMLDPDPTRRLTAHQVLEHPWLHNIKKAPNVSLGETVKARLKQFSVMNKLKKKALTVIAEFLSAEEVAGMKEAFEMMDTGKKGKINLNELKDGLQKLGHQIPDADLQILMEAADVDGDGSLNYPEFVAVSIHLRKMANDEHLHKAFSFFDKNQSGFIEIEELRSALRDEDDSNSKEVTDAIMHDVDTDKDGRISYEEFAAMMKAGTDWRKASRQYSRERFNSLSLKLMREGSLQVENKV

SEQ ID NO: 182 - protein, 533 aa, Solanum lycopersicum; identical to SEQ ID NO: 10

SEQ ID NO: 183 - protein, 533 aa, Solanum lycopersicum; identical to SEQ ID NO: 10

SEQ ID NO: 184 - protein, 533 aa, Solanum lycopersicum; identical to SEQ ID NO: 10

SEQ ID NO: 185 - protein, 527 aa, Solanum lycopersicum
MGNCCVKPGKSAEKKNKKNNSKPNPFSIDYGGTKHASGSGNKLVVLKEPTGQNIHDKYDLGRELGRGEFGVTYLCTDLEGGEKYACKSISKKKLRTAVDIDDVRREVEIMKHLPVHPNIVTLKDTYEDDNAVHIVMELCEGGELFDRIVARGHYTERAAAGILKTMCHRQGVMHRDLKPENFLFGNKKETAPLKAIDFGLSVFFKPGERFNEIVGSPYYMAPEVLKRNYGPEVDVWSAGVILYILLCGVPPFWAETEQGVAQAIIRSVIDFKRDPWPKVSDNAKDLVKKMLDPDPTRRLTAHQVLEHPWLHNIKKAPNVSLGETVKARLKQFSVMNKLKKKALTVIAEFLSAEEVAGMKEAFEMMDTGKKGKINLNELKDGLQKLGHQIPDADLHILMEAADVDGDGSLNYPEFVAVSIHLRKMANDEHLHKAFSFFDKNQSGFIEIEELRSALRDEDDSNSEEVTNAIMHDVDTDKDGRISYEEFAAMMKAGTDWRKASRQYSRERFNSLSLKLMREGSLQVENKV

SEQ ID NO: 186 - protein, 533 aa, Solanum lycopersicum; identical to SEQ ID NO: 10

SEQ ID NO: 187 - protein, 528 aa, Solanum lycopersicum; identical to SEQ ID NO: 168

SEQ ID NO: 188 - protein, 492 aa, Solanum lycopersicum
MGNCCVKPGKSAEKKNKKNNSKPNPFSIDYGGTKHASGSGNKLVVLKEPTGQNIHDKYDLGRGEKYACKSISKKKLRTAVDIDDVRREVEIMKHLPVHPNIVTLKDTYEDDNAVHIVMELCEGGELFDRIMCHRQGVMHRDLKPENFLFGNKKETAPLKAIDFGLSVFFKPGERFNEIVGSPYYMAPEVLKRNYGPEVDVWSAGVILYILLCGVPPFWAETEQGVAQAIIRSVIDFKRDPWPKVSDNAKDLVKKMLDPDPTRRLTAHQVLEHPWLHNIKKAPNVSLGETVKARLKQFSVMNKLKKKALTVIAEFLSAEEVAGMKEAFEMMDTGKKGKINLNELKDGLQKLGHQIPDADLQILMEAADVDGDGSLNYPEFVAVSIHLRKMANDEHLHKAFSFFDKNQSGFIEIEELRSALRDEDDSNSKEVTDAIMHDVDTDKDGRISYEEFAAMMKAGTDWRKASRQYSRERFNSLSLKLMREGSLQVENKV

SEQ ID NO: 189 - protein, 533 aa, Solanum lycopersicum; identical to SEQ ID NO: 10

SEQ ID NO: 190 - protein, 548 aa, Solanum lycopersicum
MADFSFFSSFLPLFWSIIGKKSTIFSIMGNCCVKPGKSAEKKNKKNNSKPNPFSIDYGGTKHASGSGNKLVVLKEPTGQNIHDKYDLGRELGRGEFGVTYLCTDLEGGEKYACKSISKKKLRTAVDIDDVRREVEIMKHLPVHPNIVTLKDTYEDDNAVHIVMELCEGGELFDRIVARGHYTERAAAGILKTVMCHRQGVMHRDLKPENFLFGNKKETAPLKAIDFGLSVFFKPGERFNEIVGSPYYMAPEVLKRNYGPEVDVWSAGVILYILLCGVPPFWAETEQGVAQAIIRSVIDFKRDPWPKVSDNAKDLVKKMLDPDPTRRLTAHQVLGNKAPNVSLGETVKARLKQFSVMNKLKKKALTVIAEFLSAEEVAGMKEAFEMMDTGKKGKINLNELKDGLQKLGHQIPDADLHILMEAADVDGDGSLNYPEFVAVSIHLRKMANDEHLHKAFSFFDKNQSGFIEIEELRSALRDEDDSNSEEVTNAIMHDVDTDKDGRISYEEFAAMMKAGTDWRKASRQYSRERFNSLSLKLMREGSLQVENKV

SEQ ID NO: 191 - protein, 533 aa, Solanum lycopersicum; identical to SEQ ID NO: 10

SEQ ID NO: 192 - protein, 528 aa, Solanum lycopersicum; identical to SEQ ID NO: 168

SEQ ID NO: 193 - protein, 533 aa, Solanum lycopersicum; identical to SEQ ID NO: 10

SEQ ID NO: 194 - protein, 533 aa, Solanum lycopersicum; identical to SEQ ID NO: 10

SEQ ID NO: 195 - protein, 533 aa, Solanum lycopersicum
MGNCCVKPGKSAEKKNKKNNSKPNPFSIDYGGTKHASGSGNKLVVLKEPTGQNIHDKYDLGRELGRGEFGVTYLCTDLEGGEKYACKSISKKKLRTAVDIDDVRREVEIMKHLPVHPNIVTLKDTYEDDNAVHIVMELCEGGELFDRIVARGHYTERAAAGILKTVVEVVQMCHRQGVMHRDLKPENFLFGNKKETAPLKAIDFGLSVFFKPGERFNEIVGSPYYMAPEVLKRNYGPEVDVWSAGVILYILLCGVPPFWAETEQGVAQAIIRSVIDFKRDPWPKVSDNAKDLVKKMLDPDPTRRLTAHQVLEHPWLHNIKKAPNVSLGETVKARLKQFSVMNKLKKKALTVIAEFLSAEEVAGMKEAFEMMDTGKKGKINLNELKDGLQKLGHQIPDADLQILMEAADVDGDGSLNYPEFVAVSIHLRKMANDEHLHKAFSFFDKNQSGFIEIEELRSALRDEDDSNSKEVTDAIMHDVDTDKDGRISYEEFAAMMKAGTDWRKASRQYSRERFNSLSLKLMREGSLQVENKV

SEQ ID NO: 196 - protein, 541 aa, Solanum lycopersicum
MGNCCVKPGKSAEKKNKKNNSKPNPFSIDYGGTKHASGSGNKLVVLKEPTGQNIHDKYDLGHELGRGEFGVTYLCTDLEGGEKYACKSISKKKLRTAVDIDDVRREVEIMKHLPVHPNIVTLKDTYEDDNAVHIVMELCEGGELFDRIVARGHYTERAAAGILKTMCHRQGVMHRDLKPENFLFGNKKETAPLKAIDFGLSVFFKPGERFNEIVGSPYYMAPEVLKRNYGPEVDVWSAGVILYILLCGVPPFWAETEQGVAQAIIRSVIDFKRDPWPKVSDNAKDLVKKMLDPDPTRRLTAHQVLGNVCGILRYCTLFIQHPWLHNIKKAPNVSLGETVKARLKQFSVMNKLKKKALTVIAEFLSAEEVAGMKEAFEMMDTGKKGKINLNELKDGLQKLGHQIPDADLHILMEAADVDGDGSLNYPEFVAVSIHLRKMANDEHLHKAFSFFDKNQSGFIEIEELRSALRDEDDSNSEEVTNAIMHDVDTDKDGRISYEEFAAMMKAGTDWRKASRQYSRERFNSLSLKLMREGSLQVENKV